European Patent Application EP 4 141 032 A1, published March 1, 2023. Title: COMBINATION THERAPY OF T CELL ACTIVATING BISPECIFIC ANTIGEN BINDING MOLECULES AND PD-1 AXIS BINDING ANTAGONISTS. Applicant: F. Hoffmann-La Roche AG. The sequence listing filed with the application follows.

SEQUENCE LISTING (430 sequences)

SEQ ID NO: 1 - protein, 120 aa, synthetic construct
  REGION 1..120: note = source = /note="Description of Artificial Sequence: Syntheticpolypeptide"
QVQLVQSGAEVKKPGASVKVSCKASGYTFTSYYMHWVRQAPGQGLEWMGIINPSGGSTSYAQKFQGRVTMTRDTSTSTVYMELSSLRSEDTAVYYCARNYYAGVTPFDYWGQGTLVTVSS

SEQ ID NO: 2 - protein, 120 aa, synthetic construct
  REGION 1..120: note = source = /note="Description of Artificial Sequence: Syntheticpolypeptide"
QVQLVQSGAEVKKPGASVKVSCKASGYTFTSYYMHWVRQAPGQGLEWMGIINPSGGSTSYAQKFQGRVTMTRDTSTSTVYMELSSLRSEDTAVYYCARNYYTGGSSAFDYWGQGTLVTVS

SEQ ID NO: 3 - protein, 120 aa, synthetic construct
  REGION 1..120: note = source = /note="Description of Artificial Sequence: Syntheticpolypeptide"
QVQLVQSGAEVKKPGASVKVSCKASGYTFTSYYMHWVRQAPGQGLEWMGIINPSGGSTSYAQKFQGRVTMTRDTSTSTVYMELSSLRSEDTAVYYCARNYYLFSTSFDYWGQGTLVTVSS

SEQ ID NO: 4 - protein, 120 aa, synthetic construct
  REGION 1..120: note = source = /note="Description of Artificial Sequence: Syntheticpolypeptide"
QVQLVQSGAEVKKPGASVKVSCKASGYTFTSYYMHWVRQAPGQGLEWMGIINPSGGSTSYAQKFQGRVTMTRDTSTSTVYMELSSLRSEDTAVYYCARNYYIGIVPFDYWGQGTLVTVSS

SEQ ID NO: 5 - protein, 120 aa, synthetic construct
  REGION 1..120: note = source = /note="Description of Artificial Sequence: Syntheticpolypeptide"
QVQLVQSGAEVKKPGASVKVSCKASGYTFTSYYMHWVRQAPGQGLEWMGIINPSGGSTSYAQKFQGRVTMTRDTSTSTVYMELSSLRSEDTAVYYCARNYYVGVSPFDYWGQGTLVTVSS

SEQ ID NO: 6 - protein, 120 aa, synthetic construct
  REGION 1..120: note = source = /note="Description of Artificial Sequence: Syntheticpolypeptide"
QVQLVQSGAEVKKPGASVKVSCKASGYTFTSYYMHWVRQAPGQGLEWMGIINPSGGSTSYAQKFQGRVTMTRDTSTSTVYMELSSLRSEDTAVYYCARNFTVLRVPFDYWGQGTLVTVSS

SEQ ID NO: 7 - protein, 120 aa, synthetic construct
  REGION 1..120: note = source = /note="Description of Artificial Sequence: Syntheticpolypeptide"
QVQLVQSGAEVKKPGASVKVSCKASGYTFTSYYMHWVRQAPGQGLEWMGIINPSGGSTSYAQKFQGRVTMTRDTSTSTVYMELSSLRSEDTAVYYCARNYYIGVVTFDYWGQGTLVTVSS

SEQ ID NO: 8 - protein, 5 aa, synthetic construct
  REGION 1..5: note = source = /note="Description of Artificial Sequence: Syntheticpeptide"
SYYMH

SEQ ID NO: 9 - protein, 17 aa, synthetic construct
  REGION 1..17: note = source = /note="Description of Artificial Sequence: Syntheticpeptide"
IINPSGGSTSYAQKFQG

SEQ ID NO: 10 - protein, 11 aa, synthetic construct
  REGION 1..11: note = source = /note="Description of Artificial Sequence: Syntheticpeptide"
NYYIGVVTFDY

SEQ ID NO: 11 - protein, 120 aa, synthetic construct
  REGION 1..120: note = source = /note="Description of Artificial Sequence: Syntheticpolypeptide"
QVQLVQSGAEVKKPGASVKVSCKASGYTFTSYYMHWVRQAPGQGLEWMGIINPSGGSTSYAQKFQGRVTMTRDTSTSTVYMELSSLRSEDTAVYYCARGEWRRYTSFDYWGQGTLVTVSS

SEQ ID NO: 12 - protein, 11 aa, synthetic construct
  REGION 1..11: note = source = /note="Description of Artificial Sequence: Syntheticpeptide"
GEWRRYTSFDY

SEQ ID NO: 13 - protein, 120 aa, synthetic construct
  REGION 1..120: note = source = /note="Description of Artificial Sequence: Syntheticpolypeptide"
QVQLVQSGAEVKKPGASVKVSCKASGYTFTSYYMHWVRQAPGQGLEWMGIINPSGGSTSYAQKFQGRVTMTRDTSTSTVYMELSSLRSEDTAVYYCARGGWIRWEHFDYWGQGTLVTVSS

SEQ ID NO: 14 - protein, 11 aa, synthetic construct
  REGION 1..11: note = source = /note="Description of Artificial Sequence: Syntheticpeptide"
GGWIRWEHFDY

SEQ ID NO: 15 - protein, 120 aa, synthetic construct
  REGION 1..120: note = source = /note="Description of Artificial Sequence: Syntheticpolypeptide"
EVQLVESGGGLVKPGGSLRLSCAASGFTFSNAWMSWVRQAPGKGLEWVGRIKSKTDGGTTDYAAPVKGRFTISRDDSKNTLYLQMNSLKTEDTAVYYCTTPWEWSWYDYWGQGTLVTVSS

SEQ ID NO: 16 - protein, 5 aa, synthetic construct
  REGION 1..5: note = source = /note="Description of Artificial Sequence: Syntheticpeptide"
NAWMS

SEQ ID NO: 17 - protein, 19 aa, synthetic construct
  REGION 1..19: note = source = /note="Description of Artificial Sequence: Syntheticpeptide"
RIKSKTDGGTTDYAAPVKG

SEQ ID NO: 18 - protein, 9 aa, synthetic construct
  REGION 1..9: note = source = /note="Description of Artificial Sequence: Syntheticpeptide"
PWEWSWYDY

SEQ ID NO: 19 - protein, 120 aa, synthetic construct
  REGION 1..120: note = source = /note="Description of Artificial Sequence: Syntheticpolypeptide"
EVQLVESGGGLVKPGGSLRLSCAASGFTFSNAWMSWVRQAPGKGLEWVGRIKSKTDGGTTDYAAPVKGRFTISRDDSKNTLYLQMNSLKTEDTAVYYCTTPWEWSYFDYWGQGTLVTVSS

SEQ ID NO: 20 - protein, 9 aa, synthetic construct
  REGION 1..9: note = source = /note="Description of Artificial Sequence: Syntheticpeptide"
PWEWSYFDY

SEQ ID NO: 21 - protein, 120 aa, synthetic construct
  REGION 1..120: note = source = /note="Description of Artificial Sequence: Syntheticpolypeptide"
EVQLVESGGGLVKPGGSLRLSCAASGFTFSNAWMSWVRQAPGKGLEWVGRIKSKTDGGTTDYAAPVKGRFTISRDDSKNTLYLQMNSLKTEDTAVYYCTTPWEWAWFDYWGQGTLVTVSS

SEQ ID NO: 22 - protein, 9 aa, synthetic construct
  REGION 1..9: note = source = /note="Description of Artificial Sequence: Syntheticpeptide"
PWEWAWFDY

SEQ ID NO: 23 - protein, 120 aa, synthetic construct
  REGION 1..120: note = source = /note="Description of Artificial Sequence: Syntheticpolypeptide"
EVQLVESGGGLVKPGGSLRLSCAASGFTFSNAWMSWVRQAPGKGLEWVGRIKSKTDGGTTDYAAPVKGRFTISRDDSKNTLYLQMNSLKTEDTAVYYCTTPWEWAYFDYWGQGTLVTVSS

SEQ ID NO: 24 - protein, 9 aa, synthetic construct
  REGION 1..9: note = source = /note="Description of Artificial Sequence: Syntheticpeptide"
PWEWAYFDY

SEQ ID NO: 25 - protein, 120 aa, synthetic construct
  REGION 1..120: note = source = /note="Description of Artificial Sequence: Syntheticpolypeptide"
QVQLVQSGAEVKKPGASVKVSCKASGYTFTSYYMHWVRQAPGQGLEWMGIINPSGGSTSYAQKFQGRVTMTRDTSTSTVYMELSSLRSEDTAVYYCARTGWSRWGYMDYWGQGTLVTVSS

SEQ ID NO: 26 - protein, 11 aa, synthetic construct
  REGION 1..11: note = source = /note="Description of Artificial Sequence: Syntheticpeptide"
TGWSRWGYMDY

SEQ ID NO: 27 - protein, 120 aa, synthetic construct
  REGION 1..120: note = source = /note="Description of Artificial Sequence: Syntheticpolypeptide"
QVQLVQSGAEVKKPGASVKVSCKASGYTFTSYYMHWVRQAPGQGLEWMGIINPSGGSTSYAQKFQGRVTMTRDTSTSTVYMELSSLRSEDTAVYYCARGEWIRYYHFDYWGQGTLVTVSS

SEQ ID NO: 28 - protein, 11 aa, synthetic construct
  REGION 1..11: note = source = /note="Description of Artificial Sequence: Syntheticpeptide"
GEWIRYYHFDY

SEQ ID NO: 29 - protein, 120 aa, synthetic construct
  REGION 1..120: note = source = /note="Description of Artificial Sequence: Syntheticpolypeptide"
QVQLVQSGAEVKKPGASVKVSCKASGYTFTSYYMHWVRQAPGQGLEWMGIINPSGGSTSYAQKFQGRVTMTRDTSTSTVYMELSSLRSEDTAVYYCARVGWYRWGYMDYWGQGTLVTVSS

SEQ ID NO: 30 - protein, 11 aa, synthetic construct
  REGION 1..11: note = source = /note="Description of Artificial Sequence: Syntheticpeptide"
VGWYRWGYMDY

SEQ ID NO: 31 - protein, 109 aa, synthetic construct
  REGION 1..109: note = source = /note="Description of Artificial Sequence: Syntheticpolypeptide"
QAVVTQEPSLTVSPGGTVTLTCGSSTGAVTTSNYANWVQEKPGQAFRGLIGGTNKRAPGTPARFSGSLLGGKAALTLSGAQPEDEAEYYCALWYSNLWVFGGGTKLTVL

SEQ ID NO: 32 - protein, 14 aa, synthetic construct
  REGION 1..14: note = source = /note="Description of Artificial Sequence: Syntheticpeptide"
GSSTGAVTTSNYAN

SEQ ID NO: 33 - protein, 7 aa, synthetic construct
  REGION 1..7: note = source = /note="Description of Artificial Sequence: Syntheticpeptide"
GTNKRAP

SEQ ID NO: 34 - protein, 9 aa, synthetic construct
  REGION 1..9: note = source = /note="Description of Artificial Sequence: Syntheticpeptide"
ALWYSNLWV

SEQ ID NO: 35 - protein, 215 aa, synthetic construct
  REGION 1..215: note = source = /note="Description of Artificial Sequence: Syntheticpolypeptide"
QAVVTQEPSLTVSPGGTVTLTCGSSTGAVTTSNYANWVQEKPGQAFRGLIGGTNKRAPGTPARFSGSLLGGKAALTLSGAQPEDEAEYYCALWYSNLWVFGGGTKLTVLGQPKAAPSVTLFPPSSEELQANKATLVCLISDFYPGAVTVAWKADSSPVKAGVETTTPSKQSNNKYAASSYLSLTPEQWKSHRSYSCQVTHEGSTVEKTVAPTECS

SEQ ID NO: 36 - protein, 125 aa, synthetic construct
  REGION 1..125: note = source = /note="Description of Artificial Sequence: Syntheticpolypeptide"
EVQLLESGGGLVQPGGSLRLSCAASGFTFSTYAMNWVRQAPGKGLEWVSRIRSKYNNYATYYADSVKGRFTISRDDSKNTLYLQMNSLRAEDTAVYYCVRHGNFGNSYVSWFAYWGQGTLVTVSS

SEQ ID NO: 37 - protein, 5 aa, synthetic construct
  REGION 1..5: note = source = /note="Description of Artificial Sequence: Syntheticpeptide"
TYAMN

SEQ ID NO: 38 - protein, 19 aa, synthetic construct
  REGION 1..19: note = source = /note="Description of Artificial Sequence: Syntheticpeptide"
RIRSKYNNYATYYADSVKG

SEQ ID NO: 39 - protein, 14 aa, synthetic construct
  REGION 1..14: note = source = /note="Description of Artificial Sequence: Syntheticpeptide"
HGNFGNSYVSWFAY

SEQ ID NO: 40 - protein, 228 aa, synthetic construct
  REGION 1..228: note = source = /note="Description of Artificial Sequence: Syntheticpolypeptide"
EVQLLESGGGLVQPGGSLRLSCAASGFTFSTYAMNWVRQAPGKGLEWVSRIRSKYNNYATYYADSVKGRFTISRDDSKNTLYLQMNSLRAEDTAVYYCVRHGNFGNSYVSWFAYWGQGTLVTVSSASTKGPSVFPLAPSSKSTSGGTAALGCLVKDYFPEPVTVSWNSGALTSGVHTFPAVLQSSGLYSLSSVVTVPSSSLGTQTYICNVNHKPSNTKVDKKVEPKSC

SEQ ID NO: 41 - protein, 121 aa, synthetic construct
  REGION 1..121: note = source = /note="Description of Artificial Sequence: Syntheticpolypeptide"
QVQLVQSGAEVKKPGSSVKVSCKASGGTFSSYAISWVRQAPGQGLEWMGGIIPIFGTANYAQKFQGRVTITADKSTSTAYMELSSLRSEDTAVYYCARAVFYRAWYSFDYWGQGTTVTVSS

SEQ ID NO: 42 - protein, 5 aa, synthetic construct
  REGION 1..5: note = source = /note="Description of Artificial Sequence: Syntheticpeptide"
SYAIS

SEQ ID NO: 43 - protein, 17 aa, synthetic construct
  REGION 1..17: note = source = /note="Description of Artificial Sequence: Syntheticpeptide"
GIIPIFGTANYAQKFQG

SEQ ID NO: 44 - protein, 12 aa, synthetic construct
  REGION 1..12: note = source = /note="Description of Artificial Sequence: Syntheticpeptide"
AVFYRAWYSFDY

SEQ ID NO: 45 - protein, 107 aa, synthetic construct
  REGION 1..107: note = source = /note="Description of Artificial Sequence: Syntheticpolypeptide"
DIQMTQSPSTLSASVGDRVTITCRASQSISSWLAWYQQKPGKAPKLLIYDASSLESGVPSRFSGSGSGTEFTLTISSLQPDDFATYYCQQYTSPPPTFGQGTKVEIK

SEQ ID NO: 46 - protein, 11 aa, synthetic construct
  REGION 1..11: note = source = /note="Description of Artificial Sequence: Syntheticpeptide"
RASQSISSWLA

SEQ ID NO: 47 - protein, 7 aa, synthetic construct
  REGION 1..7: note = source = /note="Description of Artificial Sequence: Syntheticpeptide"
DASSLES

SEQ ID NO: 48 - protein, 9 aa, synthetic construct
  REGION 1..9: note = source = /note="Description of Artificial Sequence: Syntheticpeptide"
QQYTSPPPT

SEQ ID NO: 49 - protein, 119 aa, synthetic construct
  REGION 1..119: note = source = /note="Description of Artificial Sequence: Syntheticpolypeptide"
QVQLVQSGAEVKKPGASVKVSCKASGYTFTSYYMHWVRQAPGQGLEWMGIINPSGGSTSYAQKFQGRVTMTHDTSTSTVYMELSSLRSEDTAVYYCARSFFTGFHLDYWGQGTLVTVSS

SEQ ID NO: 50 - protein, 10 aa, synthetic construct
  REGION 1..10: note = source = /note="Description of Artificial Sequence: Syntheticpeptide"
SFFTGFHLDY

SEQ ID NO: 51 - protein, 109 aa, synthetic construct
  REGION 1..109: note = source = /note="Description of Artificial Sequence: Syntheticpolypeptide"
EIVLTQSPGTLSLSPGERATLSCRASQSVSSSYLAWYQQKPGQAPRLLIYGASSRATGIPDRFSGSGSGTDFTLTISRLEPEDFAVYYCQQYTNEHYYTFGQGTKVEIK

SEQ ID NO: 52 - protein, 12 aa, synthetic construct
  REGION 1..12: note = source = /note="Description of Artificial Sequence: Syntheticpeptide"
RASQSVSSSYLA

SEQ ID NO: 53 - protein, 7 aa, synthetic construct
  REGION 1..7: note = source = /note="Description of Artificial Sequence: Syntheticpeptide"
GASSRAT

SEQ ID NO: 54 - protein, 10 aa, synthetic construct
  REGION 1..10: note = source = /note="Description of Artificial Sequence: Syntheticpeptide"
QQYTNEHYYT

SEQ ID NO: 55 - protein, 117 aa, synthetic construct
  REGION 1..117: note = source = /note="Description of Artificial Sequence: Syntheticpolypeptide"
QVQLVQSGAEVKKPGASVKVSCKASGYTFTSYYMHWVRQAPGQGLEWMGIINPSGGPTSYAQKFQGRVTMTRDTSTSTVYMELSSLRSEDTAVYYCARGDFAWLDYWGQGTLVTVSS

SEQ ID NO: 56 - protein, 17 aa, synthetic construct
  REGION 1..17: note = source = /note="Description of Artificial Sequence: Syntheticpeptide"
IINPSGGPTSYAQKFQG

SEQ ID NO: 57 - protein, 8 aa, synthetic construct
  REGION 1..8: note = source = /note="Description of Artificial Sequence: Syntheticpeptide"
GDFAWLDY

SEQ ID NO: 58 - protein, 112 aa, synthetic construct
  REGION 1..112: note = source = /note="Description of Artificial Sequence: Syntheticpolypeptide"
DIVMTQSPLSLPVTPGEPASISCRSSQSLLHSNGYNYLDWYLQKPGQSPQLLIYLGSNRASGVPDRFSGSGSGTDFTLKISRVEAEDVGVYYCMQASIMNRTFGQGTKVEIK

SEQ ID NO: 59 - protein, 16 aa, synthetic construct
  REGION 1..16: note = source = /note="Description of Artificial Sequence: Syntheticpeptide"
RSSQSLLHSNGYNYLD

SEQ ID NO: 60 - protein, 7 aa, synthetic construct
  REGION 1..7: note = source = /note="Description of Artificial Sequence: Syntheticpeptide"
LGSNRAS

SEQ ID NO: 61 - protein, 9 aa, synthetic construct
  REGION 1..9: note = source = /note="Description of Artificial Sequence: Syntheticpeptide"
MQASIMNRT

SEQ ID NO: 62 - protein, 112 aa, synthetic construct
  REGION 1..112: note = source = /note="Description of Artificial Sequence: Syntheticpolypeptide"
DIVMTQSPLSLPVTPGEPASISCRSSQSLLHSNGYNYLDWYLQKPGQSPQLLIYLGSNRASGVPDRFSGSGSGTDFTLKISRVEAEDVGVYYCMQASIMSRTFGQGTKVEIK

SEQ ID NO: 63 - protein, 9 aa, synthetic construct
  REGION 1..9: note = source = /note="Description of Artificial Sequence: Syntheticpeptide"
MQASIMSRT

SEQ ID NO: 64 - protein, 112 aa, synthetic construct
  REGION 1..112: note = source = /note="Description of Artificial Sequence: Syntheticpolypeptide"
DIVMTQSPLSLPVTPGEPASISCRSSQSLLHSNGYNYLDWYLQKPGQSPQLLIYLGSNRASGVPDRFSGSGSGTDFTLKISRVEAEDVGVYYCMQASIMQRTFGQGTKVEIK

SEQ ID NO: 65 - protein, 9 aa, synthetic construct
  REGION 1..9: note = source = /note="Description of Artificial Sequence: Syntheticpeptide"
MQASIMQRT

SEQ ID NO: 66 - protein, 112 aa, synthetic construct
  REGION 1..112: note = source = /note="Description of Artificial Sequence: Syntheticpolypeptide"
DIVMTQSPLSLPVTPGEPASISCRSSQSLLHSNGYNYLDWYLQKPGQSPQLLIYLGSNRASGVPDRFSGSGSGTDFTLKISRVEAEDVGVYYCMQASIMNRAFGQGTKVEIK

SEQ ID NO: 67 - protein, 9 aa, synthetic construct
  REGION 1..9: note = source = /note="Description of Artificial Sequence: Syntheticpeptide"
MQASIMNRA

SEQ ID NO: 68 - protein, 112 aa, synthetic construct
  REGION 1..112: note = source = /note="Description of Artificial Sequence: Syntheticpolypeptide"
DIVMTQSPLSLPVTPGEPASISCRSSQSLLHSNGYNYLDWYLQKPGQSPQLLIYLGSNRASGVPDRFSGSGSGTDFTLKISRVEAEDVGVYYCMQASIMNRNFGQGTKVEIK

SEQ ID NO: 69 - protein, 9 aa, synthetic construct
  REGION 1..9: note = source = /note="Description of Artificial Sequence: Syntheticpeptide"
MQASIMNRN

SEQ ID NO: 70 - protein, 116 aa, synthetic construct
  REGION 1..116: note = source = /note="Description of Artificial Sequence: Syntheticpolypeptide"
QVQLVQSGAEVKKPGASVKVSCKASGYTFTSYYMHWVRQAPGQGLEWMGIINPSGGSTSYAQKFQGRVTMTRDTSTSTVYMELSSLRSEDTAVYYCARSYIDMDYWGQGTLVTVSS

SEQ ID NO: 71 - protein, 7 aa, synthetic construct
  REGION 1..7: note = source = /note="Description of Artificial Sequence: Syntheticpeptide"
SYIDMDY

SEQ ID NO: 72 - protein, 107 aa, synthetic construct
  REGION 1..107: note = source = /note="Description of Artificial Sequence: Syntheticpolypeptide"
EIVLTQSPGTLSLSPGERATLSCRASQSVSSSYLAWYQQKPGQAPRLLIYGASSRATGIPDRFSGSGSGTDFTLTISRLEPEDFAVYYCQQDNWSPTFGQGTKVEIK

SEQ ID NO: 73 - protein, 8 aa, synthetic construct
  REGION 1..8: note = source = /note="Description of Artificial Sequence: Syntheticpeptide"
QQDNWSPT

SEQ ID NO: 74 - protein, 116 aa, synthetic construct
  REGION 1..116: note = source = /note="Description of Artificial Sequence: Syntheticpolypeptide"
QVQLVQSGAEVKKPGASVKVSCKASGYTFTSYYMHWVRQAPGQGLEWMGIINPSGGSTSYAQKFQGRVTMTRDTSTSTVYMELSSLRSEDTAVYYCARSYVDMDYWGQGTLVTVSS

SEQ ID NO: 75 - protein, 7 aa, synthetic construct
  REGION 1..7: note = source = /note="Description of Artificial Sequence: Syntheticpeptide"
SYVDMDY

SEQ ID NO: 76 - protein, 107 aa, synthetic construct
  REGION 1..107: note = source = /note="Description of Artificial Sequence: Syntheticpolypeptide"
EIVLTQSPGTLSLSPGERATLSCRASQSVSSSYLAWYQQKPGQAPRLLIYGASSRATGIPDRFSGSGSGTDFTLTISRLEPEDFAVYYCQQDIWSPTFGQGTKVEIK

SEQ ID NO: 77 - protein, 8 aa, synthetic construct
  REGION 1..8: note = source = /note="Description of Artificial Sequence: Syntheticpeptide"
QQDIWSPT

SEQ ID NO: 78 - protein, 121 aa, synthetic construct
  REGION 1..121: note = source = /note="Description of Artificial Sequence: Syntheticpolypeptide"
EVQLLESGGGLVQPGGSLRLSCAASGFTFSSYAMSWVRQAPGKGLEWVSAISGSGGSTYYADSVKGRFTISRDNSKNTLYLQMNSLRAEDTAVYYCAKDSSYVEWYAFDYWGQGTLVTVSS

SEQ ID NO: 79 - protein, 5 aa, synthetic construct
  REGION 1..5: note = source = /note="Description of Artificial Sequence: Syntheticpeptide"
SYAMS

SEQ ID NO: 80 - protein, 17 aa, synthetic construct
  REGION 1..17: note = source = /note="Description of Artificial Sequence: Syntheticpeptide"
AISGSGGSTYYADSVKG

SEQ ID NO: 81 - protein, 12 aa, synthetic construct
  REGION 1..12: note = source = /note="Description of Artificial Sequence: Syntheticpeptide"
DSSYVEWYAFDY

SEQ ID NO: 82 - protein, 108 aa, synthetic construct
  REGION 1..108: note = source = /note="Description of Artificial Sequence: Syntheticpolypeptide"
EIVLTQSPGTLSLSPGERATLSCRASQSVSSSYLAWYQQKPGQAPRLLIYGASSRATGIPDRFSGSGSGTDSTLTISRLEPEDFAVYYCQQPTSSPITFGQGTKVEIK

SEQ ID NO: 83 - protein, 9 aa, synthetic construct
  REGION 1..9: note = source = /note="Description of Artificial Sequence: Syntheticpeptide"
QQPTSSPIT

SEQ ID NO: 84 - protein, 103 aa, synthetic construct
  REGION 1..103: note = source = /note="Description of Artificial Sequence: Syntheticpolypeptide"
ASTKGPSVFPLAPSSKSTSGGTAALGCLVKDYFPEPVTVSWNSGALTSGVHTFPAVLQSSGLYSLSSVVTVPSSSLGTQTYICNVNHKPSNTKVDKKVEPKSC

SEQ ID NO: 85 - protein, 103 aa, synthetic construct; identical to SEQ ID NO: 84
  REGION 1..103: note = source = /note="Description of Artificial Sequence: Syntheticpolypeptide"

SEQ ID NO: 86 - protein, 214 aa, synthetic construct
  REGION 1..214: note = source = /note="Description of Artificial Sequence: Syntheticpolypeptide"
QAVVTQEPSLTVSPGGTVTLTCGSSTGAVTTSNYANWVQEKPGQAFRGLIGGTNKRAPGTPARFSGSLLGGKAALTLSGAQPEDEAEYYCALWYSNLWVFGGGTKLTVLSSASTKGPSVFPLAPSSKSTSGGTAALGCLVKDYFPEPVTVSWNSGALTSGVHTFPAVLQSSGLYSLSSVVTVPSSSLGTQTYICNVNHKPSNTKVDKKVEPKSC

SEQ ID NO: 87 - protein, 232 aa, synthetic construct
  REGION 1..232: note = source = /note="Description of Artificial Sequence: Syntheticpolypeptide"
EVQLLESGGGLVQPGGSLRLSCAASGFTFSTYAMNWVRQAPGKGLEWVSRIRSKYNNYATYYADSVKGRFTISRDDSKNTLYLQMNSLRAEDTAVYYCVRHGNFGNSYVSWFAYWGQGTLVTVSSASVAAPSVFIFPPSDEQLKSGTASVVCLLNNFYPREAKVQWKVDNALQSGNSQESVTEQDSKDSTYSLSSTLTLSKADYEKHKVYACEVTHQGLSSPVTKSFNRGEC

SEQ ID NO: 88 - protein, 105 aa, synthetic construct [sequence omitted]

SEQ ID NO: 89 - protein, 689 aa, synthetic construct
  REGION 1..689: note = source = /note="Description of Artificial Sequence: Syntheticpolypeptide"
EVQLVESGGGLVKPGGSLRLSCAASGFTFSNAWMSWVRQAPGKGLEWVGRIKSKTDGGTTDYAAPVKGRFTISRDDSKNTLYLQMNSLKTEDTAVYYCTTPWEWSWYDYWGQGTLVTVSSASTKGPSVFPLAPSSKSTSGGTAALGCLVKDYFPEPVTVSWNSGALTSGVHTFPAVLQSSGLYSLSSVVTVPSSSLGTQTYICNVNHKPSNTKVDKKVEPKSCDGGGGSGGGGSEVQLLESGGGLVQPGGSLRLSCAASGFTFSTYAMNWVRQAPGKGLEWVSRIRSKYNNYATYYADSVKGRFTISRDDSKNTLYLQMNSLRAEDTAVYYCVRHGNFGNSYVSWFAYWGQGTLVTVSSASTKGPSVFPLAPSSKSTSGGTAALGCLVKDYFPEPVTVSWNSGALTSGVHTFPAVLQSSGLYSLSSVVTVPSSSLGTQTYICNVNHKPSNTKVDKKVEPKSCDKTHTCPPCPAPEAAGGPSVFLFPPKPKDTLMISRTPEVTCVVVDVSHEDPEVKFNWYVDGVEVHNAKTKPREEQYNSTYRVVSVLTVLHQDWLNGKEYKCKVSNKALGAPIEKTISKAKGQPREPQVYTLPPCRDELTKNQVSLWCLVKGFYPSDIAVEWESNGQPENNYKTTPPVLDSDGSFFLYSKLTVDKSRWQQGNVFSCSVMHEALHNHYTQKSLSLSPGK

SEQ ID NO: 90 - protein, 450 aa, synthetic construct
  REGION 1..450: note = source = /note="Description of Artificial Sequence: Syntheticpolypeptide"
EVQLVESGGGLVKPGGSLRLSCAASGFTFSNAWMSWVRQAPGKGLEWVGRIKSKTDGGTTDYAAPVKGRFTISRDDSKNTLYLQMNSLKTEDTAVYYCTTPWEWSWYDYWGQGTLVTVSSASTKGPSVFPLAPSSKSTSGGTAALGCLVKDYFPEPVTVSWNSGALTSGVHTFPAVLQSSGLYSLSSVVTVPSSSLGTQTYICNVNHKPSNTKVDKKVEPKSCDKTHTCPPCPAPEAAGGPSVFLFPPKPKDTLMISRTPEVTCVVVDVSHEDPEVKFNWYVDGVEVHNAKTKPREEQYNSTYRVVSVLTVLHQDWLNGKEYKCKVSNKALGAPIEKTISKAKGQPREPQVCTLPPSRDELTKNQVSLSCAVKGFYPSDIAVEWESNGQPENNYKTTPPVLDSDGSFFLVSKLTVDKSRWQQGNVFSCSVMHEALHNRFTQKSLSLSPGK

SEQ ID NO: 91 - protein, 689 aa, synthetic construct
  REGION 1..689: note = source = /note="Description of Artificial Sequence: Syntheticpolypeptide"
EVQLLESGGGLVQPGGSLRLSCAASGFTFSTYAMNWVRQAPGKGLEWVSRIRSKYNNYATYYADSVKGRFTISRDDSKNTLYLQMNSLRAEDTAVYYCVRHGNFGNSYVSWFAYWGQGTLVTVSSASTKGPSVFPLAPSSKSTSGGTAALGCLVKDYFPEPVTVSWNSGALTSGVHTFPAVLQSSGLYSLSSVVTVPSSSLGTQTYICNVNHKPSNTKVDKKVEPKSCDGGGGSGGGGSEVQLVESGGGLVKPGGSLRLSCAASGFTFSNAWMSWVRQAPGKGLEWVGRIKSKTDGGTTDYAAPVKGRFTISRDDSKNTLYLQMNSLKTEDTAVYYCTTPWEWSWYDYWGQGTLVTVSSASTKGPSVFPLAPSSKSTSGGTAALGCLVKDYFPEPVTVSWNSGALTSGVHTFPAVLQSSGLYSLSSVVTVPSSSLGTQTYICNVNHKPSNTKVDKKVEPKSCDKTHTCPPCPAPEAAGGPSVFLFPPKPKDTLMISRTPEVTCVVVDVSHEDPEVKFNWYVDGVEVHNAKTKPREEQYNSTYRVVSVLTVLHQDWLNGKEYKCKVSNKALGAPIEKTISKAKGQPREPQVYTLPPCRDELTKNQVSLWCLVKGFYPSDIAVEWESNGQPENNYKTTPPVLDSDGSFFLYSKLTVDKSRWQQGNVFSCSVMHEALHNHYTQKSLSLSPGK

SEQ ID NO: 92 - protein, 455 aa, synthetic construct
  REGION 1..455: note = source = /note="Description of Artificial Sequence: Syntheticpolypeptide"
EVQLLESGGGLVQPGGSLRLSCAASGFTFSTYAMNWVRQAPGKGLEWVSRIRSKYNNYATYYADSVKGRFTISRDDSKNTLYLQMNSLRAEDTAVYYCVRHGNFGNSYVSWFAYWGQGTLVTVSSASTKGPSVFPLAPSSKSTSGGTAALGCLVKDYFPEPVTVSWNSGALTSGVHTFPAVLQSSGLYSLSSVVTVPSSSLGTQTYICNVNHKPSNTKVDKKVEPKSCDKTHTCPPCPAPEAAGGPSVFLFPPKPKDTLMISRTPEVTCVVVDVSHEDPEVKFNWYVDGVEVHNAKTKPREEQYNSTYRVVSVLTVLHQDWLNGKEYKCKVSNKALGAPIEKTISKAKGQPREPQVYTLPPCRDELTKNQVSLWCLVKGFYPSDIAVEWESNGQPENNYKTTPPVLDSDGSFFLYSKLTVDKSRWQQGNVFSCSVMHEALHNHYTQKSLSLSPGK

SEQ ID NO: 93 - protein, 227 aa, synthetic construct
  REGION 1..227: note = source = /note="Description of Artificial Sequence: Syntheticpolypeptide"
DKTHTCPPCPAPELLGGPSVFLFPPKPKDTLMISRTPEVTCVVVDVSHEDPEVKFNWYVDGVEVHNAKTKPREEQYNSTYRVVSVLTVLHQDWLNGKEYKCKVSNKALPAPIEKTISKAKGQPREPQVCTLPPSRDELTKNQVSLSCAVKGFYPSDIAVEWESNGQPENNYKTTPPVLDSDGSFFLVSKLTVDKSRWQQGNVFSCSVMHEALHNRFTQKSLSLSPGK

SEQ ID NO: 94 - protein, 690 aa, synthetic construct
  REGION 1..690: note = source = /note="Description of Artificial Sequence: Syntheticpolypeptide"
QVQLVQSGAEVKKPGASVKVSCKASGYTFTSYYMHWVRQAPGQGLEWMGIINPSGGPTSYAQKFQGRVTMTRDTSTSTVYMELSSLRSEDTAVYYCARGDFAWLDYWGQGTLVTVSSASTKGPSVFPLAPSSKSTSGGTAALGCLVKDYFPEPVTVSWNSGALTSGVHTFPAVLQSSGLYSLSSVVTVPSSSLGTQTYICNVNHKPSNTKVDKKVEPKSCDGGGGSGGGGSEVQLLESGGGLVQPGGSLRLSCAASGFTFSTYAMNWVRQAPGKGLEWVSRIRSKYNNYATYYADSVKGRFTISRDDSKNTLYLQMNSLRAEDTAVYYCVRHGNFGNSYVSWFAYWGQGTLVTVSSASVAAPSVFIFPPSDEQLKSGTASVVCLLNNFYPREAKVQWKVDNALQSGNSQESVTEQDSKDSTYSLSSTLTLSKADYEKHKVYACEVTHQGLSSPVTKSFNRGECDKTHTCPPCPAPEAAGGPSVFLFPPKPKDTLMISRTPEVTCVVVDVSHEDPEVKFNWYVDGVEVHNAKTKPREEQYNSTYRVVSVLTVLHQDWLNGKEYKCKVSNKALGAPIEKTISKAKGQPREPQVYTLPPCRDELTKNQVSLWCLVKGFYPSDIAVEWESNGQPENNYKTTPPVLDSDGSFFLYSKLTVDKSRWQQGNVFSCSVMHEALHNHYTQKSLSLSPGK

SEQ ID NO: 95 - protein, 447 aa, synthetic construct
  REGION 1..447: note = source = /note="Description of Artificial Sequence: Syntheticpolypeptide"
QVQLVQSGAEVKKPGASVKVSCKASGYTFTSYYMHWVRQAPGQGLEWMGIINPSGGPTSYAQKFQGRVTMTRDTSTSTVYMELSSLRSEDTAVYYCARGDFAWLDYWGQGTLVTVSSASTKGPSVFPLAPSSKSTSGGTAALGCLVKDYFPEPVTVSWNSGALTSGVHTFPAVLQSSGLYSLSSVVTVPSSSLGTQTYICNVNHKPSNTKVDKKVEPKSCDKTHTCPPCPAPEAAGGPSVFLFPPKPKDTLMISRTPEVTCVVVDVSHEDPEVKFNWYVDGVEVHNAKTKPREEQYNSTYRVVSVLTVLHQDWLNGKEYKCKVSNKALGAPIEKTISKAKGQPREPQVCTLPPSRDELTKNQVSLSCAVKGFYPSDIAVEWESNGQPENNYKTTPPVLDSDGSFFLVSKLTVDKSRWQQGNVFSCSVMHEALHNHYTQKSLSLSPGK

SEQ ID NO: 96 - protein, 219 aa, synthetic construct
  REGION 1..219: note = source = /note="Description of Artificial Sequence: Syntheticpolypeptide"
DIVMTQSPLSLPVTPGEPASISCRSSQSLLHSNGYNYLDWYLQKPGQSPQLLIYLGSNRASGVPDRFSGSGSGTDFTLKISRVEAEDVGVYYCMQASIMNRTFGQGTKVEIKRTVAAPSVFIFPPSDEQLKSGTASVVCLLNNFYPREAKVQWKVDNALQSGNSQESVTEQDSKDSTYSLSSTLTLSKADYEKHKVYACEVTHQGLSSPVTKSFNRGEC

SEQ ID NO: 97 - DNA, 648 bp, synthetic construct
  modified_base 603: mod_base = OTHER; note = a, c, t, g, unknown or other
  misc_feature 1..648: note = source = /note="Description of Artificial Sequence: Syntheticpolynucleotide"
  source 1..648: mol_type = other DNA
gaaatcgtgttaacgcagtctccaggcaccctgtctttgtctccaggggaaagagccaccctctcttgcagggccagtcagagtgttagcagcagctacttagcctggtaccagcagaaacctggccaggctcccaggctcctcatctatggagcatccagcagggccactggcatcccagacaggttcagtggcagtggatccgggacagacttcactctcaccatcagcagactggagcctgaagattttgcagtgtattactgtcagcagtataccaacgaacattattatacgttcggccaggggaccaaagtggaaatcaaacgtacggtggctgcaccatctgtcttcatcttcccgccatctgatgagcagttgaaatctggaactgcctctgttgtgtgcctgctgaataacttctatcccagagaggccaaagtacagtggaaggtggataacgccctccaatcgggtaactcccaggagagtgtcacagagcaggacagcaaggacagcacctacagcctcagcagcaccctgacgctgagcaaagcagactacgagaaacacaaagtctacgcctgcgaagtcacccatcanggcctgagctcgcccgtcacaaagagcttcaacaggggagagtgt

SEQ ID NO: 98 - protein, 459 aa, synthetic construct
  REGION 1..459: note = source = /note="Description of Artificial Sequence: Syntheticpolypeptide"
EVQLLESGGGLVQPGGSLRLSCAASGFTFSTYAMNWVRQAPGKGLEWVSRIRSKYNNYATYYADSVKGRFTISRDDSKNTLYLQMNSLRAEDTAVYYCVRHGNFGNSYVSWFAYWGQGTLVTVSSASVAAPSVFIFPPSDEQLKSGTASVVCLLNNFYPREAKVQWKVDNALQSGNSQESVTEQDSKDSTYSLSSTLTLSKADYEKHKVYACEVTHQGLSSPVTKSFNRGECDKTHTCPPCPAPEAAGGPSVFLFPPKPKDTLMISRTPEVTCVVVDVSHEDPEVKFNWYVDGVEVHNAKTKPREEQYNSTYRVVSVLTVLHQDWLNGKEYKCKVSNKALGAPIEKTISKAKGQPREPQVYTLPPCRDELTKNQVSLWCLVKGFYPSDIAVEWESNGQPENNYKTTPPVLDSDGSFFLYSKLTVDKSRWQQGNVFSCSVMHEALHNHYTQKSLSLSPGK

SEQ ID NO: 99 - protein, 689 aa, synthetic construct
  REGION 1..689: note = source = /note="Description of Artificial Sequence: Syntheticpolypeptide"
EVQLVESGGGLVKPGGSLRLSCAASGFTFSNAWMSWVRQAPGKGLEWVGRIKSKTDGGTTDYAAPVKGRFTISRDDSKNTLYLQMNSLKTEDTAVYYCTTPWEWSWYDYWGQGTLVTVSSASTKGPSVFPLAPSSKSTSGGTAALGCLVKDYFPEPVTVSWNSGALTSGVHTFPAVLQSSGLYSLSSVVTVPSSSLGTQTYICNVNHKPSNTKVDKKVEPKSCDGGGGSGGGGSEVQLLESGGGLVQPGGSLRLSCAASGFTFSTYAMNWVRQAPGKGLEWVSRIRSKYNNYATYYADSVKGRFTISRDDSKNTLYLQMNSLRAEDTAVYYCVRHGNFGASYVSWFAYWGQGTLVTVSSASTKGPSVFPLAPSSKSTSGGTAALGCLVKDYFPEPVTVSWNSGALTSGVHTFPAVLQSSGLYSLSSVVTVPSSSLGTQTYICNVNHKPSNTKVDKKVEPKSCDKTHTCPPCPAPEAAGGPSVFLFPPKPKDTLMISRTPEVTCVVVDVSHEDPEVKFNWYVDGVEVHNAKTKPREEQYNSTYRVVSVLTVLHQDWLNGKEYKCKVSNKALGAPIEKTISKAKGQPREPQVYTLPPCRDELTKNQVSLWCLVKGFYPSDIAVEWESNGQPENNYKTTPPVLDSDGSFFLYSKLTVDKSRWQQGNVFSCSVMHEALHNHYTQKSLSLSPGK

SEQ ID NO: 100 - protein, 689 aa, synthetic construct
  REGION 1..689: note = source = /note="Description of Artificial Sequence: Syntheticpolypeptide"
EVQLVESGGGLVKPGGSLRLSCAASGFTFSNAWMSWVRQAPGKGLEWVGRIKSKTDGGTTDYAAPVKGRFTISRDDSKNTLYLQMNSLKTEDTAVYYCTTPWEWSWYDYWGQGTLVTVSSASTKGPSVFPLAPSSKSTSGGTAALGCLVKDYFPEPVTVSWNSGALTSGVHTFPAVLQSSGLYSLSSVVTVPSSSLGTQTYICNVNHKPSNTKVDKKVEPKSCDGGGGSGGGGSEVQLLESGGGLVQPGGSLRLSCAASGFTFSTYAMNWVRQAPGKGLEWVSRIRSKYNNYATYYADSVKGRFTISRDDSKNTLYLQMNSLRAEDTAVYYCVRHGNFGNAYVSWFAYWGQGTLVTVSSASTKGPSVFPLAPSSKSTSGGTAALGCLVKDYFPEPVTVSWNSGALTSGVHTFPAVLQSSGLYSLSSVVTVPSSSLGTQTYICNVNHKPSNTKVDKKVEPKSCDKTHTCPPCPAPEAAGGPSVFLFPPKPKDTLMISRTPEVTCVVVDVSHEDPEVKFNWYVDGVEVHNAKTKPREEQYNSTYRVVSVLTVLHQDWLNGKEYKCKVSNKALGAPIEKTISKAKGQPREPQVYTLPPCRDELTKNQVSLWCLVKGFYPSDIAVEWESNGQPENNYKTTPPVLDSDGSFFLYSKLTVDKSRWQQGNVFSCSVMHEALHNHYTQKSLSLSPGK

SEQ ID NO: 101 - protein, 441 aa, synthetic construct
  REGION 1..441: note = source = /note="Description of Artificial Sequence: Syntheticpolypeptide"
QAVVTQEPSLTVSPGGTVTLTCGSSTGAVTTSNYANWVQEKPGQAFRGLIGGTNKRAPGTPARFSGSLLGGKAALTLSGAQPEDEAEYYCALWYSNLWVFGGGTKLTVLSSASTKGPSVFPLAPSSKSTSGGTAALGCLVKDYFPEPVTVSWNSGALTSGVHTFPAVLQSSGLYSLSSVVTVPSSSLGTQTYICNVNHKPSNTKVDKKVEPKSCDKTHTCPPCPAPEAAGGPSVFLFPPKPKDTLMISRTPEVTCVVVDVSHEDPEVKFNWYVDGVEVHNAKTKPREEQYNSTYRVVSVLTVLHQDWLNGKEYKCKVSNKALGAPIEKTISKAKGQPREPQVYTLPPSRDELTKNQVSLTCLVKGFYPSDIAVEWESNGQPENNYKTTPPVLDSDGSFFLYSKLTVDKSRWQQGNVFSCSVMHEALHNHYTQKSLSLSPGK

SEQ ID NO: 102 - protein, 227 aa, synthetic construct
  REGION 1..227: note = source = /note="Description of Artificial Sequence: Syntheticpolypeptide"
EVQLVESGGGLVKPGGSLRLSCAASGFTFSNAWMSWVRQAPGKGLEWVGRIKSKTDGGTTDYAAPVKGRFTISRDDSKNTLYLQMNSLKTEDTAVYYCTTPWEWSWYDYWGQGTLVTVSSASVAAPSVFIFPPSDEQLKSGTASVVCLLNNFYPREAKVQWKVDNALQSGNSQESVTEQDSKDSTYSLSSTLTLSKADYEKHKVYACEVTHQGLSSPVTKSFNRGEC

SEQ ID NO: 103 - protein, 231 aa, synthetic construct
  REGION 1..231: note = source = /note="Description of Artificial Sequence: Syntheticpolypeptide"
EVQLLESGGGLVQPGGSLRLSCAASGFTFSTYAMNWVRQAPGKGLEWVSRIRSKYNNYATYYADSVKGRFTISRDDSKNTLYLQMNSLRAEDTAVYYCVRHGNFGNSYVSWFAYWGQGTLVTVSSASPKAAPSVTLFPPSSEELQANKATLVCLISDFYPGAVTVAWKADSSPVKAGVETTTPSKQSNNKYAASSYLSLTPEQWKSHRSYSCQVTHEGSTVEKTVAPTECS

SEQ ID NO: 104 - protein, 118 aa, synthetic construct
  REGION 1..118: note = source = /note="Description of Artificial Sequence: Syntheticpolypeptide"
QVQLVQSGAEVKKPGASVKVSCKASGYTFTSYYMHWVRQAPGQGLEWMGIINPSGGSTSYAQKFQGRVTMTRDTSTSTVYMELSSLRSEDTAVYYCARGGSGGSFDYWGQGTLVTVSS

SEQ ID NO: 105 - protein, 118 aa, synthetic construct
  REGION 1..118: note = source = /note="Description of Artificial Sequence: Syntheticpolypeptide"
QVQLVQSGAEVKKPGSSVKVSCKASGGTFSSYAISWVRQAPGQGLEWMGGIIPIFGTANYAQKFQGRVTITADKSTSTAYMELSSLRSEDTAVYYCARGGSGGSMDAWGQGTTVTVSS

SEQ ID NO: 106 - protein, 120 aa, synthetic construct
  REGION 1..120: note = source = /note="Description of Artificial Sequence: Syntheticpolypeptide"
EVQLVESGGGLVKPGGSLRLSCAASGFTFSNAWMSWVRQAPGKGLEWVGRIKSKTDGGTTDYAAPVKGRFTISRDDSKNTLYLQMNSLKTEDTAVYYCTTGGSGGSFDYWGQGTLVTVSS

SEQ ID NO: 107 - protein, 118 aa, synthetic construct
  REGION 1..118: note = source = /note="Description of Artificial Sequence: Syntheticpolypeptide"
EVQLLESGGGLVQPGGSLRLSCAASGFTFSSYAMSWVRQAPGKGLEWVSAISGSGGSTYYADSVKGRFTISRDNSKNTLYLQMNSLRAEDTAVYYCAKGGSGGSFDYWGQGTLVTVSS

SEQ ID NO: 108 - protein, 117 aa, synthetic construct
  REGION 1..117: note = source = /note="Description of Artificial Sequence: Syntheticpolypeptide"
QVQLQESGPGLVKPSETLSLTCTVSGGSISSYYWSWIRQPPGKGLEWIGYIYYSGSTNYNPSLKSRVTISVDTSKNQFSLKLSSVTAADTAVYYCARGGSGGSFDYWGQGTLVTVSS

SEQ ID NO: 109 - protein, 118 aa, synthetic construct
  REGION 1..118: note = source = /note="Description of Artificial Sequence: Syntheticpolypeptide"
EVQLVQSGAEVKKPGESLKISCKGSGYSFTSYWIGWVRQMPGKGLEWMGIIYPGDSDTRYSPSFQGQVTISADKSISTAYLQWSSLKASDTAMYYCARGGSGGSFDYWGQGTLVTVSS

SEQ ID NO: 110 - protein, 109 aa, synthetic construct
  REGION 1..109: note = source = /note="Description of Artificial Sequence: Syntheticpolypeptide"
QTVVTQEPSLTVSPGGTVTLTCGSSTGAVTTSNYANWVQEKPGQAFRGLIGGTNKRAPGTPARFSGSLLGGKAALTLSGAQPEDEAEYYCALWYSNLWVFGGGTKLTVL

SEQ ID NO: 111 - protein, 107 aa, synthetic construct [sequence omitted]

SEQ ID NO: 112 - protein, 109 aa, synthetic construct; identical to SEQ ID NO: 31
  REGION 1..109: note = source = /note="Description of Artificial Sequence: Syntheticpolypeptide"

SEQ ID NO: 113 - protein, 109 aa, synthetic construct
  REGION 1..109: note = source = /note="Description of Artificial Sequence: Syntheticpolypeptide"
QTVVTQEPSLTVSPGGTVTLTCGSSTGAVTTSNYANWVQQKPGQAPRGLIGGTNARAPGTPARFSGSLLGGKAALTLSGVQPEDEAEYYCALWYSNLWVFGGGTKLTVL

SEQ ID NO: 114 - protein, 109 aa, synthetic construct
  REGION 1..109: note = source = /note="Description of Artificial Sequence: Syntheticpolypeptide"
QTVVTQEPSLTVSPGGTVTLTCGSSTGAVTTSNYANWVQQKPGQAPRGLIGGTNKRAPGTPARFSGSLLGGKAALTLSGVQPEDEAEYYCALWYANLWVFGGGTKLTVL

SEQ ID NO: 115 - protein, 122 aa, synthetic construct
  REGION 1..122: note = source = /note="Description of Artificial Sequence: Syntheticpolypeptide"
EVQLVESGGGLVKPGGSLRLSCAASGFTFSNAWMHWVRQAPGKGLEWVGRIKSKTDGGTTDYAAPVKGRFTISRDDSKNTLYLQMNSLKTEDTAVYYCTTPWEWSWYDYWGQGTLVTVSSAS

SEQ ID NO: 116 - protein, 122 aa, synthetic construct
  REGION 1..122: note = source = /note="Description of Artificial Sequence: Syntheticpolypeptide"
EVQLVESGGGLVKPGGSLRLSCAASGFTFSNAWMSWVRQAPGKGLEWVSRIKSKTDGGTTDYAAPVKGRFTISRDDSKNTLYLQMNSLKTEDTAVYYCTTPWEWSWYDYWGQGTLVTVSSAS

SEQ ID NO: 117 - protein, 122 aa, synthetic construct
  REGION 1..122: note = source = /note="Description of Artificial Sequence: Syntheticpolypeptide"
EVQLVESGGGLVKPGGSLRLSCAASGFTFSNAWMSWVRQAPGKGLEWVGSIKSKTDGGTTDYAAPVKGRFTISRDDSKNTLYLQMNSLKTEDTAVYYCTTPWEWSWYDYWGQGTLVTVSSAS

SEQ ID NO: 118 - protein, 122 aa, synthetic construct
  REGION 1..122: note = source = /note="Description of Artificial Sequence: Syntheticpolypeptide"
EVQLVESGGGLVKPGGSLRLSCAASGFTFSNAWMSWVRQAPGKGLEWVGRIKSKTDGGTTDYAAPVKGRFTISRDDSKNTLYLQMNSLKTEDTAVYYCTTPYEWSWYDYWGQGTLVTVSSAS

SEQ ID NO: 119 - protein, 122 aa, synthetic construct
  REGION 1..122: note = source = /note="Description of Artificial Sequence: Syntheticpolypeptide"
EVQLVESGGGLVKPGGSLRLSCAASGFTFSNAWMSWVRQAPGKGLEWVGRIKSKTDGGTTDYAAPVKGRFTISRDDSKNTLYLQMNSLKTEDTAVYYCTTPWEYSWYDYWGQGTLVTVSSAS

SEQ ID NO: 120 - protein, 122 aa, synthetic construct
  REGION 1..122: note = source = /note="Description of Artificial Sequence: Syntheticpolypeptide"
QVQLVQSGAEVKKPGASVKVSCKASGYTFTSYYMHWVRQAPGQGLEWMGIINPSGGSTSYAQKFQGRVTMTRDTSTSTVYMELSSLRSEDTAVYYCARNYTIVVSPFDYWGQGTLVTVSSAS

SEQ ID NO: 121 - protein, 122 aa, synthetic construct
  REGION 1..122: note = source = /note="Description of Artificial Sequence: Syntheticpolypeptide"
QVQLVQSGAEVKKPGASVKVSCKASGYTFTSYYMHWVRQAPGQGLEWMGIINPSGGSTSYAQKFQGRVTMTRDTSTSTVYMELSSLRSEDTAVYYCARNYFIGSVAMDYWGQGTLVTVSSAS

SEQ ID NO: 122 - protein, 119 aa, synthetic construct
  REGION 1..119: note = source = /note="Description of Artificial Sequence: Syntheticpolypeptide"
QVQLVQSGAEVKKPGASVKVSCKASGYTFTSYYMHWVRQAPGQGLEWMGIINPSGGSTSYAQKFQGRVTMTRDTSTSTVYMELSSLRSEDTAVYYCARGLTYSMDYWGQGTLVTVSSAS

SEQ ID NO: 123 - protein, 114 aa, synthetic construct
  REGION 1..114: note = source = /note="Description of Artificial Sequence: Syntheticpolypeptide"
DIVMTQSPLSLPVTPGEPASISCRSSQSLLHSNGYNYLDWYLQKPGQSPQLLIYLGSNRASGVPDRFSGSGSGTDFTLKISRVEAEDVGVYYCMQALQIPNTFGQGTKVEIKRT

SEQ ID NO: 124 - protein, 118 aa, synthetic construct
  REGION 1..118: note = source = /note="Description of Artificial Sequence: Syntheticpolypeptide"
EVQLLESGGGLVQPGGSLRLSCAASGFTFSSYAMSWVRQAPGKGLEWVSAISGSGGSTYYADSVKGRFTISRDNSKNTLYLQMNSLRAEDTAVYYCAKYAYALDYWGQGTLVTVSSAS

SEQ ID NO: 125 - protein, 109 aa, synthetic construct
  REGION 1..109: note = source = /note="Description of Artificial Sequence: Syntheticpolypeptide"
EIVLTQSPGTLSLSPGERATLSCRASQSVSSSYLAWYQQKPGQAPRLLIYGASSRATGIPDRFSGSGSGTDFTLTISRLEPEDFAVYYCQQHGSSSTFGQGTKVEIKRT

SEQ ID NO: 126 - protein, 122 aa, synthetic construct
  REGION 1..122: note = source = /note="Description of Artificial Sequence: Syntheticpolypeptide"
QVQLVQSGAEVKKPGASVKVSCKASGYTFTSYYMHWVRQAPGQGLEWMGIINPSGGSTSYAQKFQGRVTMTRDTSTSTVYMELSSLRSEDTAVYYCARGDFSAGRLMDYWGQGTLVTVSSAS

SEQ ID NO: 127 - protein, 115 aa, synthetic construct
  REGION 1..115: note = source = /note="Description of Artificial Sequence: Syntheticpolypeptide"
DIVMTQSPLSLPVTPGEPASISCRSSQSLLHSNGYNYLDWYLQKPGQSPQLLIYLGSNRASGVPDRFSGSGSGTDFTLKISRVEAEDVGVYYCMQALQTPPITFGQGTKVEIKRT

SEQ ID NO: 128 - protein, 119 aa, synthetic construct
  REGION 1..119: note = source = /note="Description of Artificial Sequence: Syntheticpolypeptide"
QVQLVQSGAEVKKPGASVKVSCKASGYTFTSYYMHWVRQAPGQGLEWMGIINPSGGSTSYAQKFQGRVTMTRDTSTSTVYMELSSLRSEDTAVYYCARGDYNAFDYWGHGTLVTVSSAS

SEQ ID NO: 129 - protein, 113 aa, synthetic construct
  REGION 1..113: note = source = /note="Description of Artificial Sequence: Syntheticpolypeptide"
DIVMTQSPLSLPVTPGEPASISCRSSQSLLHSNGYNYLDWYLQKPGQSPQLLIYLGSNRASGVPDRFSGSGSGTDFTLKISRVEAEDVGVYYCMQAWHSPTFGQGTKVEIKRT

SEQ ID NO: 130 - protein, 119 aa, synthetic construct
  REGION 1..119: note = source = /note="Description of Artificial Sequence: Syntheticpolypeptide"
QVQLVQSGAEVKKPGASVKVSCKASGYTFTSYYMHWVRQAPGQGLEWMGIINPSGGSTSYAQKFQGRVTMTRDTSTSTVYMELSSLRSEDTAVYYCARGATYTMDYWGQGTLVTVSSAS

SEQ ID NO: 131 - protein, 114 aa, synthetic construct
  REGION 1..114: note = source = /note="Description of Artificial Sequence: Syntheticpolypeptide"
DIVMTQSPLSLPVTPGEPASISCRSSQSLLHSNGYNYLDWYLQKPGQSPQLLIYLGSNRASGVPDRFSGSGSGTDFTLKISRVEAEDVGVYYCMQALQTPITFGQGTKVEIKRT

SEQ ID NO: 132 - protein, 112 aa, synthetic construct; identical to SEQ ID NO: 62
  REGION 1..112: note = source = /note="Description of Artificial Sequence: Syntheticpolypeptide"

SEQ ID NO: 133 - protein, 112 aa, synthetic construct; identical to SEQ ID NO: 64
  REGION 1..112: note = source = /note="Description of Artificial Sequence: Syntheticpolypeptide"

SEQ ID NO: 134 - protein, 112 aa, synthetic construct; identical to SEQ ID NO: 66
  REGION 1..112: note = source = /note="Description of Artificial Sequence: Syntheticpolypeptide"

SEQ ID NO: 135 - protein, 112 aa, synthetic construct; identical to SEQ ID NO: 68
  REGION 1..112: note = source = /note="Description of Artificial Sequence: Syntheticpolypeptide"

SEQ ID NO: 136 - protein, 448 aa, synthetic construct
  REGION 1..448: note = source = /note="Description of Artificial Sequence: Syntheticpolypeptide"
QVQLQQSGAELVKPGASVKISCKASGYSFTGYFMNWVKQSHGKSLEWIGRIHPYDGDTFYNQNFKDKATLTVDKSSNTAHMELLSLTSEDFAVYYCTRYDGSRAMDYWGQGTTVTVSSASTKGPSVFPLAPSSKSTSGGTAALGCLVKDYFPEPVTVSWNSGALTSGVHTFPAVLQSSGLYSLSSVVTVPSSSLGTQTYICNVNHKPSNTKVDKKVEPKSCDKTHTCPPCPAPEAAGGPSVFLFPPKPKDTLMISRTPEVTCVVVDVSHEDPEVKFNWYVDGVEVHNAKTKPREEQYNSTYRVVSVLTVLHQDWLNGKEYKCKVSNKALGAPIEKTISKAKGQPREPQVCTLPPSRDELTKNQVSLSCAVKGFYPSDIAVEWESNGQPENNYKTTPPVLDSDGSFFLVSKLTVDKSRWQQGNVFSCSVMHEALHNHYTQKSLSLSPGK

SEQ ID NO: 137 - protein, 691 aa, synthetic construct
  REGION 1..691: note = source = /note="Description of Artificial Sequence: Syntheticpolypeptide"
QVQLQQSGAELVKPGASVKISCKASGYSFTGYFMNWVKQSHGKSLEWIGRIHPYDGDTFYNQNFKDKATLTVDKSSNTAHMELLSLTSEDFAVYYCTRYDGSRAMDYWGQGTTVTVSSASTKGPSVFPLAPSSKSTSGGTAALGCLVKDYFPEPVTVSWNSGALTSGVHTFPAVLQSSGLYSLSSVVTVPSSSLGTQTYICNVNHKPSNTKVDKKVEPKSCDGGGGSGGGGSEVQLVESGGGLVQPKGSLKLSCAASGFTFNTYAMNWVRQAPGKGLEWVARIRSKYNNYATYYADSVKDRFTISRDDSQSILYLQMNNLKTEDTAMYYCVRHGNFGNSYVSWFAYWGQGTLVTVSAASVAAPSVFIFPPSDEQLKSGTASVVCLLNNFYPREAKVQWKVDNALQSGNSQESVTEQDSKDSTYSLSSTLTLSKADYEKHKVYACEVTHQGLSSPVTKSFNRGECDKTHTCPPCPAPEAAGGPSVFLFPPKPKDTLMISRTPEVTCVVVDVSHEDPEVKFNWYVDGVEVHNAKTKPREEQYNSTYRVVSVLTVLHQDWLNGKEYKCKVSNKALGAPIEKTISKAKGQPREPQVYTLPPCRDELTKNQVSLWCLVKGFYPSDIAVEWESNGQPENNYKTTPPVLDSDGSFFLYSKLTVDKSRWQQGNVFSCSVMHEALHNHYTQKSLSLSPGK

SEQ ID NO: 138 - protein, 218 aa, synthetic construct
  REGION 1..218: note = source = /note="Description of Artificial Sequence: Syntheticpolypeptide"
DIELTQSPASLAVSLGQRAIISCKASQSVSFAGTSLMHWYHQKPGQQPKLLIYRASNLEAGVPTRFSGSGSKTDFTLNIHPVEEEDAATYYCQQSREYPYTFGGGTKLEIKRTVAAPSVFIFPPSDEQLKSGTASVVCLLNNFYPREAKVQWKVDNALQSGNSQESVTEQDSKDSTYSLSSTLTLSKADYEKHKVYACEVTHQGLSSPVTKSFNRGEC

SEQ ID NO: 139 - protein, 257 aa, Homo sapiens
MAQRMTTQLLLLLVWVAVVGEAQTRIAWARTELLNVCMNAKHHKEKPGPEDKLHEQCRPWRKNACCSTNTSQEAHKDVSYLYRFNWNHCGEMAPACKRHFIQDTCLYECSPNLGPWIQQVDQSWRKERVLNVPLCKEDCEQWWEDCRTSYTCKSNWHKGWNWTSGFNKCAVGAACQPFHFYFPTPTVLCNEIWTHSYKVSNYSRGSGRCIQMWFDPAQGNPNEEVARFYAAAMSGAGPWAAWPFLLSLALMLLWLLS

SEQ ID NO: 140 - protein, 468 aa, synthetic construct
  REGION 1..468: note = source = /note="Description of Artificial Sequence: Syntheticpolypeptide"
RIAWARTELLNVCMNAKHHKEKPGPEDKLHEQCRPWRKNACCSTNTSQEAHKDVSYLYRFNWNHCGEMAPACKRHFIQDTCLYECSPNLGPWIQQVDQSWRKERVLNVPLCKEDCEQWWEDCRTSYTCKSNWHKGWNWTSGFNKCAVGAACQPFHFYFPTPTVLCNEIWTHSYKVSNYSRGSGRCIQMWFDPAQGNPNEEVARFYAAAMVDEQLYFQGGSPKSADKTHTCPPCPAPELLGGPSVFLFPPKPKDTLMISRTPEVTCVVVDVSHEDPEVKFNWYVDGVEVHNAKTKPREEQYNSTYRVVSVLTVLHQDWLNGKEYKCKVSNKALPAPIEKTISKAKGQPREPQVYTLPPCRDELTKNQVSLWCLVKGFYPSDIAVEWESNGQPENNYKTTPPVLDSDGSFFLYSKLTVDKSRWQQGNVFSCSVMHEALHNHYTQKSLSLSPGKSGGLNDIFEAQKIEWHE

SEQ ID NO: 141 - protein, 227 aa, synthetic construct; identical to SEQ ID NO: 93
  REGION 1..227: note = source = /note="Description of Artificial Sequence: Syntheticpolypeptide"

SEQ ID NO: 142 - protein, 255 aa, Mus musculus
MAHLMTVQLLLLVMWMAECAQSRATRARTELLNVCMDAKHHKEKPGPEDNLHDQCSPWKTNSCCSTNTSQEAHKDISYLYRFNWNHCGTMTSECKRHFIQDTCLYECSPNLGPWIQQVDQSWRKERILDVPLCKEDCQQWWEDCQSSFTCKSNWHKGWNWSSGHNECPVGASCHPFTFYFPTSAALCEEIWSHSYKLSNYSRGSGRCIQMWFDPAQGNPNEEVARFYAEAMSGAGLHGTWPLLCSLSLVLLWVIS

SEQ ID NO: 143 - protein, 466 aa, synthetic construct
  REGION 1..466: note = source = /note="Description of Artificial Sequence: Syntheticpolypeptide"
TRARTELLNVCMDAKHHKEKPGPEDNLHDQCSPWKTNSCCSTNTSQEAHKDISYLYRFNWNHCGTMTSECKRHFIQDTCLYECSPNLGPWIQQVDQSWRKERILDVPLCKEDCQQWWEDCQSSFTCKSNWHKGWNWSSGHNECPVGASCHPFTFYFPTSAALCEEIWSHSYKLSNYSRGSGRCIQMWFDPAQGNPNEEVARFYAEAMVDEQLYFQGGSPKSADKTHTCPPCPAPELLGGPSVFLFPPKPKDTLMISRTPEVTCVVVDVSHEDPEVKFNWYVDGVEVHNAKTKPREEQYNSTYRVVSVLTVLHQDWLNGKEYKCKVSNKALPAPIEKTISKAKGQPREPQVYTLPPCRDELTKNQVSLWCLVKGFYPSDIAVEWESNGQPENNYKTTPPVLDSDGSFFLYSKLTVDKSRWQQGNVFSCSVMHEALHNHYTQKSLSLSPGKSGGLNDIFEAQKIEWHE

SEQ ID NO: 144 - protein, 257 aa, Macaca fascicularis
MAQRMTTQLLLLLVWVAVVGEAQTRTARARTELLNVCMNAKHHKEKPGPEDKLHEQCRPWKKNACCSTNTSQEAHKDVSYLYRFNWNHCGEMAPACKRHFIQDTCLYECSPNLGPWIQQVDQSWRKERVLNVPLCKEDCERWWEDCRTSYTCKSNWHKGWNWTSGFNKCPVGAACQPFHFYFPTPTVLCNEIWTYSYKVSNYSRGSGRCIQMWFDPAQGNPNEEVARFYAAAMSGAGPWAAWPLLLSLALTLLWLLS

SEQ ID NO: 145 - protein, 468 aa, synthetic construct
  REGION 1..468: note = source = /note="Description of Artificial Sequence: Syntheticpolypeptide"
RTARARTELLNVCMNAKHHKEKPGPEDKLHEQCRPWKKNACCSTNTSQEAHKDVSYLYRFNWNHCGEMAPACKRHFIQDTCLYECSPNLGPWIQQVDQSWRKERVLNVPLCKEDCEQWWEDCRTSYTCKSNWHKGWNWTSGFNKCPVGAACQPFHFYFPTPTVLCNEIWTYSYKVSNYSRGSGRCIQMWFDPAQGNPNEEVARFYAAAMVDEQLYFQGGSPKSADKTHTCPPCPAPELLGGPSVFLFPPKPKDTLMISRTPEVTCVVVDVSHEDPEVKFNWYVDGVEVHNAKTKPREEQYNSTYRVVSVLTVLHQDWLNGKEYKCKVSNKALPAPIEKTISKAKGQPREPQVYTLPPCRDELTKNQVSLWCLVKGFYPSDIAVEWESNGQPENNYKTTPPVLDSDGSFFLYSKLTVDKSRWQQGNVFSCSVMHEALHNHYTQKSLSLSPGKSGGLNDIFEAQKIEWHE

SEQ ID NO: 146 - protein, 255 aa, Homo sapiens
MVWKWMPLLLLLVCVATMCSAQDRTDLLNVCMDAKHHKTKPGPEDKLHDQCSPWKKNACCTASTSQELHKDTSRLYNFNWDHCGKMEPACKRHFIQDTCLYECSPNLGPWIQQVNQSWRKERFLDVPLCKEDCQRWWEDCHTSHTCKSNWHRGWDWTSGVNKCPAGALCRTFESYFPTPAALCEGLWSHSYKVSNYSRGSGRCIQMWFDSAQGNPNEEVARFYAAAMHVNAGEMLHGTGGLLLSLALMLQLWLLG

SEQ ID NO: 147 - protein, 472 aa, synthetic construct
  REGION 1..472: note = source = /note="Description of Artificial Sequence: Syntheticpolypeptide"
TMCSAQDRTDLLNVCMDAKHHKTKPGPEDKLHDQCSPWKKNACCTASTSQELHKDTSRLYNFNWDHCGKMEPACKRHFIQDTCLYECSPNLGPWIQQVNQSWRKERFLDVPLCKEDCQRWWEDCHTSHTCKSNWHRGWDWTSGVNKCPAGALCRTFESYFPTPAALCEGLWSHSYKVSNYSRGSGRCIQMWFDSAQGNPNEEVARFYAAAMHVVDEQLYFQGGSPKSADKTHTCPPCPAPELLGGPSVFLFPPKPKDTLMISRTPEVTCVVVDVSHEDPEVKFNWYVDGVEVHNAKTKPREEQYNSTYRVVSVLTVLHQDWLNGKEYKCKVSNKALPAPIEKTISKAKGQPREPQVYTLPPCRDELTKNQVSLWCLVKGFYPSDIAVEWESNGQPENNYKTTPPVLDSDGSFFLYSKLTVDKSRWQQGNVFSCSVMHEALHNHYTQKSLSLSPGKSGGLNDIFEAQKIEWHE

SEQ ID NO: 148 - protein, 243 aa, Homo sapiens
MAWQMMQLLLLALVTAAGSAQPRSARARTDLLNVCMNAKHHKTQPSPEDELYGQCSPWKKNACCTASTSQELHKDTSRLYNFNWDHCGKMEPTCKRHFIQDSCLYECSPNLGPWIRQVNQSWRKERILNVPLCKEDCERWWEDCRTSYTCKSNWHKGWNWTSGINECPAGALCSTFESYFPTPAALCEGLWSHSFKVSNYSRGSGRCIQMWFDSAQGNPNEEVAKFYAAAMNAGAPSRGIIDS

SEQ ID NO: 149 - protein, 479 aa, synthetic construct
  REGION 1..479: note = source = /note="Description of Artificial Sequence: Syntheticpolypeptide"
SARARTDLLNVCMNAKHHKTQPSPEDELYGQCSPWKKNACCTASTSQELHKDTSRLYNFNWDHCGKMEPTCKRHFIQDSCLYECSPNLGPWIRQVNQSWRKERILNVPLCKEDCERWWEDCRTSYTCKSNWHKGWNWTSGINECPAGALCSTFESYFPTPAALCEGLWSHSFKVSNYSRGSGRCIQMWFDSAQGNPNEEVAKFYAAAMNAGAPSRGIIDSVDEQLYFQGGSPKSADKTHTCPPCPAPELLGGPSVFLFPPKPKDTLMISRTPEVTCVVVDVSHEDPEVKFNWYVDGVEVHNAKTKPREEQYNSTYRVVSVLTVLHQDWLNGKEYKCKVSNKALPAPIEKTISKAKGQPREPQVYTLPPCRDELTKNQVSLWCLVKGFYPSDIAVEWESNGQPENNYKTTPPVLDSDGSFFLYSKLTVDKSRWQQGNVFSCSVMHEALHNHYTQKSLSLSPGKSGGLNDIFEAQKIEWHE

SEQ ID NO: 150 - protein, 207 aa, Homo sapiens
MQSGTHWRVLGLCLLSVGVWGQDGNEEMGGITQTPYKVSISGTTVILTCPQYPGSEILWQHNDKNIGGDEDDKNIGSDEDHLSLKEFSELEQSGYYVCYPRGSKPEDANFYLYLRARVCENCMEMDVMSVATIVIVDICITGGLLLLVYYWSKNRKAKAKPVTRGAGAGGRQRGQNKERPPPVPNPDYEPIRKGQRDLYSGLNQRRI

SEQ ID NO: 151 - DNA, 360 bp, synthetic construct
  misc_feature 1..360: note = source = /note="Description of Artificial Sequence: Syntheticpolynucleotide"
  source 1..360: mol_type = other DNA
caggtgcaattggttcaatctggtgctgaagtaaaaaaaccgggcgcttccgttaaagtgagctgcaaagcatccggatacaccttcacttcctattacatgcactgggttcgtcaagccccgggccagggtctggaatggatgggcatcattaacccaagcggtggctctacctcctacgcgcagaaattccagggtcgcgtcacgatgacccgtgacactagcacctctaccgtttatatggagctgtccagcctgcgttctgaagatactgcagtgtactactgtgcacgcaactactacgctggtgttactccgttcgactattggggtcaaggcaccctcgtaacggtttcttct

SEQ ID NO: 152 - DNA, 360 bp, synthetic construct
  misc_feature 1..360: note = source = /note="Description of Artificial Sequence: Syntheticpolynucleotide"
  source 1..360: mol_type = other DNA
caggtgcaattggttcaatctggtgctgaagtaaaaaaaccgggcgcttccgttaaagtgagctgcaaagcatccggatacaccttcacttcctattacatgcactgggttcgtcaagccccgggccagggtctggaatggatgggcatcattaacccaagcggtggctctacctcctacgcgcagaaattccagggtcgcgtcacgatgacccgtgacactagcacctctaccgtttatatggagctgtccagcctgcgttctgaagatactgcagtgtactactgtgcacgcaactactacatcggtgttgttactttcgactattggggtcaaggcaccctcgtaacggtttcttct

SEQ ID NO: 153 - DNA, 363 bp, synthetic construct
  misc_feature 1..363: note = source = /note="Description of Artificial Sequence: Syntheticpolynucleotide"
  source 1..363: mol_type = other DNA
caggtgcaattggttcaatctggtgctgaagtaaaaaaaccgggcgcttccgttaaagtgagctgcaaagcatccggatacaccttcacttcctattacatgcactgggttcgtcaagccccgggccagggtctggaatggatgggcatcattaacccaagcggtggctctacctcctacgcgcagaaattccagggtcgcgtcacgatgacccgtgacactagcacctctaccgtttatatggagctgtccagcctgcgttctgaagatactgcagtgtactactgtgcacgcaactactacactggtggttcttctgctttcgactattggggtcaaggcaccctcgtaacggtttcttct

SEQ ID NO: 154 - DNA, 360 bp, synthetic construct
  modified_base 47: mod_base = OTHER; note = a, c, t, g, unknown or other
  misc_feature 1..360: note = source = /note="Description of Artificial Sequence: Syntheticpolynucleotide"
  source 1..360: mol_type = other DNA
caggtgcaattggttcaatctggtgctgaagtaaaaaaaccgggcgnttccgttaaagtgagctgcaaagcatccggatacaccttcacttcctattacatgcactgggttcgtcaagccccgggccagggtctggaatggatgggcatcattaacccaagcggtggctctacctcctacgcgcagaaattccagggtcgcgtcacgatgacccgtgacactagcacctctaccgtttatatggagctgtccagcctgcgttctgaagatactgcagtgtactactgtgcacgcggtgaatggcgtcgttacacttctttcgactattggggtcaaggcaccctcgtaacggtttcttct

SEQ ID NO: 155 - DNA, 360 bp, synthetic construct
  misc_feature 1..360: note = source = /note="Description of Artificial Sequence: Syntheticpolynucleotide"
  source 1..360: mol_type = other DNA
caggtgcaattggttcaatctggtgctgaagtaaaaaaaccgggcgcttccgttaaagtgagctgcaaagcatccggatacaccttcacttcctattacatgcactgggttcgtcaagccccgggccagggtctggaatggatgggcatcattaacccaagcggtggctctacctcctacgcgcagaaattccagggtcgcgtcacgatgacccgtgacactagcacctctaccgtttatatggagctgtccagcctgcgttctgaagatactgcagtgtactactgtgcacgcggtggttggatccgttgggaacatttcgactattggggtcaaggcaccctcgtaacggtttcttct

SEQ ID NO: 156 - DNA, 360 bp, synthetic construct
  misc_feature 1..360: note = source = /note="Description of Artificial Sequence: Syntheticpolynucleotide"
  source 1..360: mol_type = other DNA
caggtgcaattggttcaatctggtgctgaagtaaaaaaaccgggcgcttccgttaaagtgagctgcaaagcatccggatacaccttcacttcctattacatgcactgggttcgtcaagccccgggccagggtctggaatggatgggcatcattaacccaagcggtggctctacctcctacgcgcagaaattccagggtcgcgtcacgatgacccgtgacactagcacctctaccgtttatatggagctgtccagcctgcgttctgaagatactgcagtgtactactgtgcacgcaactactacctgttctctacttctttcgactattggggtcaaggcaccctcgtaacggtttcttct

SEQ ID NO: 157 - DNA, 360 bp, synthetic construct
  misc_feature 1..360: note = source = /note="Description of Artificial Sequence: Syntheticpolynucleotide"
  source 1..360: mol_type = other DNA
caggtgcaattggttcaatctggtgctgaggtaaaaaaaccgggcgcttccgttaaagtgagctgcaaagcatccggatacaccttcacttcctattacatgcactgggttcgtcaagccccgggccagggtctggaatggatgggcatcattaacccaagcggtggctctacctcctacgcgcagaaattccagggtcgcgtcacgatgacccgtgacactagcacctctaccgtttatatggagctgtccagcctgcgttctgaagatactgcagtgtactactgtgcacgcaactactacatcggtatcgttccgttcgactattggggtcaaggcaccctcgtaacggtttcttct

SEQ ID NO: 158 - DNA, 360 bp, synthetic construct
  misc_feature 1..360: note = source = /note="Description of Artificial Sequence: Syntheticpolynucleotide"
  source 1..360: mol_type = other DNA
gaggtgcaattggttgaatctggtggtggtctggtaaaaccgggcggttccctgcgtctgagctgcgcggcttccggattcaccttctccaacgcgtggatgagctgggttcgccaggccccgggcaaaggcctcgagtgggttggtcgtatcaagtctaaaactgacggtggcaccacggattacgcggctccagttaaaggtcgttttaccatttcccgcgacgatagcaaaaacactctgtatctgcagatgaactctctgaaaactgaagacaccgcagtctactactgtactaccccgtgggaatggtcttggtacgattattggggccagggcacgctggttacggtgtcttcc

SEQ ID NO: 159 - DNA, 360 bp, synthetic construct
  modified_base 53: mod_base = OTHER; note = a, c, t, g, unknown or other
  misc_feature 1..360: note = source = /note="Description of Artificial Sequence: Syntheticpolynucleotide"
  source 1..360: mol_type = other DNA
gaggtgcaattggttgaatctggtggtggtctggtaaaaccgggcggttcccngcgtctgagctgcgcggcttccggattcaccttctccaacgcgtggatgagctgggttcgccaggccccgggcaaaggcctcgagtgggttggtcgtatcaagtctaaaactgacggtggcaccacggattacgcggctccagttaaaggtcgttttaccatttcccgcgacgatagcaaaaacactctgtatctgcagatgaactctctgaaaaccgaagacaccgcagtctactactgtactaccccgtgggaatggtcttacttcgattattggggccagggcacgctggttacggtgtcttcc

SEQ ID NO: 160 - DNA, 360 bp, synthetic construct
  misc_feature 1..360: note = source = /note="Description of Artificial Sequence: Syntheticpolynucleotide"
  source 1..360: mol_type = other DNA
caggtgcaattggttcaatctggtgctgaagtaaaaaaaccgggcgcttccgttaaagtgagctgcaaagcatccggatacaccttcacttcctattacatgcactgggttcgtcaagccccgggccagggtctggaatggatgggcatcattaacccaagcggtggctctacctcctacgcgcagaaattccagggtcgcgtcacgatgacccgtgacactagcacctctaccgtttatatggagctgtccagcctgcgttctgaagatactgcagtgtactactgtgcacgcaactactacgttggtgtttctccgttcgactattggggtcaaggcaccctcgtaacggtttcttct

SEQ ID NO: 161 - DNA, 360 bp, synthetic construct
  modified_base 47: mod_base = OTHER; note = a, c, t, g, unknown or other
  modified_base 177: mod_base = OTHER; note = a, c, t, g, unknown or other
  misc_feature 1..360: note = source = /note="Description of Artificial Sequence: Syntheticpolynucleotide"
  source 1..360: mol_type = other DNA
caggtgcaattggttcaatctggtgctgaagtaaaaaaaccgggcgnttccgttaaagtgagctgcaaagcatccggatacaccttcacttcctattacatgcactgggttcgtcaagccccgggccagggtctggaatggatgggcatcattaacccaagcggtggctctacctcntacgcgcagaaattccagggtcgcgtcacgatgacccgtgacactagcacctctaccgtttatatggagctgtccagcctgcgttctgaagatactgcagtgtactactgtgcacgcaacttcactgttctgcgtgttccgttcgactattggggtcaaggcaccctcgtaacggtttcttct

SEQ ID NO: 162 - DNA, 360 bp, synthetic construct
  misc_feature 1..360: note = source = /note="Description of Artificial Sequence: Syntheticpolynucleotide"
  source 1..360: mol_type = other DNA
gaggtgcaattggttgaatctggtggtggtctggtaaaaccgggcggttccctgcgtctgagctgcgcggcttccggattcaccttctccaacgcgtggatgagctgggttcgccaggccccgggcaaaggcctcgagtgggttggtcgtatcaagtctaaaactgacggtggcaccacggattacgcggctccagttaaaggtcgttttaccatttcccgcgacgatagcaaaaacactctgtatctgcagatgaactctctgaaaactgaagacaccgcagtctactactgtactaccccgtgggaatgggcttggttcgattattggggccagggcacgctggttacggtgtcttcc

SEQ ID NO: 163 - DNA, 360 bp, synthetic construct
  misc_feature 1..360: note = source = /note="Description of Artificial Sequence: Syntheticpolynucleotide"
  source 1..360: mol_type = other DNA
gaggtgcaattggttgaatctggtggtggtctggtaaaaccgggcggttccctgcgtctgagctgcgcggcttccggattcaccttctccaacgcgtggatgagctgggttcgccaggccccgggcaaaggcctcgagtgggttggtcgtatcaagtctaaaactgacggtggcaccacggattacgcggctccagttaaaggtcgttttaccatttcccgcgacgatagcaaaaacactctgtatctgcagatgaactctctgaaaaccgaagacaccgcagtctactactgtactaccccttgggaatgggcttacttcgattattggggccagggcacgctggttacggtgtcttcc

SEQ ID NO: 164 - DNA, 360 bp, synthetic construct
  misc_feature 1..360: note = source = /note="Description of Artificial Sequence: Syntheticpolynucleotide"
  source 1..360: mol_type = other DNA
caggtgcaattggttcaatctggtgctgaagtaaaaaaaccgggcgcttccgttaaagtgagctgcaaagcatccggatacaccttcacttcctattacatgcactgggttcgtcaagccccgggccagggtctggaatggatgggcatcattaacccaagcggtggctctacctcctacgcgcagaaattccagggtcgcgtcacgatgacccgtgacactagcacctctaccgtttatatggagctgtccagcctgcgttctgaagatactgcagtgtactactgtgcacgcactggttggtctcgttggggttacatggactattggggccaaggcaccctcgtaacggtttcttct

SEQ ID NO: 165 - DNA, 360 bp, synthetic construct
  misc_feature 1..360: note = source = /note="Description of Artificial Sequence: Syntheticpolynucleotide"
  source 1..360: mol_type = other DNA
caggtgcaattggttcaatctggtgctgaagtaaaaaaaccgggcgcttccgttaaagtgagctgcaaagcatccggatacaccttcacttcctattacatgcactgggttcgtcaagccccgggccagggtctggaatggatgggcatcattaacccaagcggtggctctacctcctacgcgcagaaattccagggtcgcgtcacgatgacccgtgacactagcacctctaccgtttatatggagctgtccagcctgcgttctgaagatactgcagtgtactactgtgcacgcggtgaatggatccgttactaccatttcgactattggggtcaaggcaccctcgtaacggtttcttct

SEQ ID NO: 166 - DNA, 360 bp, synthetic construct
  misc_feature 1..360: note = source = /note="Description of Artificial Sequence: Syntheticpolynucleotide"
  source 1..360: mol_type = other DNA
caggtgcaattggttcaatctggtgctgaagtaaaaaaaccgggcgcttccgttaaagtgagctgcaaagcatccggatacaccttcacttcctattacatgcactgggttcgtcaagccccgggccagggtctggaatggatgggcatcattaacccaagcggtggctctacctcctacgcgcagaaattccagggtcgcgtcacgatgacccgtgacactagcacctctaccgtttatatggagctgtccagcctgcgttctgaagatactgcagtgtactactgtgcacgcgttggttggtaccgttggggttacatggactattggggtcaaggcaccctcgtaacggtttcttct

SEQ ID NO: 167 - DNA, 363 bp, synthetic construct
  misc_feature 1..363: note = source = /note="Description of Artificial Sequence: Syntheticpolynucleotide"
  source 1..363: mol_type = other DNA
caggtgcaattggtgcagtctggggctgaggtgaagaagcctgggtcctcggtgaaggtctcctgcaaggcctccggaggcacattcagcagctacgctataagctgggtgcgacaggcccctggacaagggctcgagtggatgggagggatcatccctatctttggtacagcaaactacgcacagaagttccagggcagggtaaccattactgcagacaaatccacgagcacagcctacatggagctgagcagcctgagatctgaggacaccgccgtgtattactgtgcgagagctgttttctaccgtgcttggtactctttcgactactggggccaagggaccaccgtgaccgtctcctca

SEQ ID NO: 168 - DNA, 321 bp, synthetic construct
  misc_feature 1..321: note = source = /note="Description of Artificial Sequence: Syntheticpolynucleotide"
  source 1..321: mol_type = other DNA
gacatccagatgacccagtctccttccaccctgtctgcatctgtaggagaccgtgtcaccatcacttgccgtgccagtcagagtattagtagctggttggcctggtatcagcagaaaccagggaaagcccctaagctcctgatctatgatgcctccagtttggaaagtggggtcccatcacgtttcagcggcagtggatccgggacagaattcactctcaccatcagcagcttgcagcctgatgattttgcaacttattactgccaacagtataccagcccaccaccaacgtttggccagggcaccaaagtcgagatcaag

SEQ ID NO: 169 - DNA, 357 bp, synthetic construct
  misc_feature 1..357: note = source = /note="Description of Artificial Sequence: Syntheticpolynucleotide"
  source 1..357: mol_type = other DNA
caggtgcaattggttcaatctggtgctgaagtaaaaaaaccgggcgcttccgttaaagtgagctgcaaagcatccggatacaccttcacttcctattacatgcactgggttcgtcaagccccgggccagggtctggaatggatgggcatcattaacccaagcggtggctctacctcctacgcgcagaaattccagggtcgcgtcacgatgacccatgacactagcacctctaccgtttatatggagctgtccagcctgcgttctgaagatactgcagtgtactactgtgcacgctctttcttcactggtttccatctggactattggggtcaaggcaccctcgtaacggtttcttct

SEQ ID NO: 170 - DNA, 327 bp, synthetic construct
  misc_feature 1..327: note = source = /note="Description of Artificial Sequence: Syntheticpolynucleotide"
  source 1..327: mol_type = other DNA
gaaatcgtgttaacgcagtctccaggcaccctgtctttgtctccaggggaaagagccaccctctcttgcagggccagtcagagtgttagcagcagctacttagcctggtaccagcagaaacctggccaggctcccaggctcctcatctatggagcatccagcagggccactggcatcccagacaggttcagtggcagtggatccgggacagacttcactctcaccatcagcagactggagcctgaagattttgcagtgtattactgtcagcagtataccaacgaacattattatacgttcggccaggggaccaaagtggaaatcaaa

SEQ ID NO: 171 - DNA, 351 bp, synthetic construct
  misc_feature 1..351: note = source = /note="Description of Artificial Sequence: Syntheticpolynucleotide"
  source 1..351: mol_type = other DNA
caggtgcaattggttcaatctggtgctgaagtaaaaaaaccgggcgcttccgttaaagtgagctgcaaagcatccggatacaccttcacttcctattacatgcactgggttcgtcaagccccgggccagggtctggaatggatgggcatcattaacccaagcggtggccctacctcctacgcgcagaaattccagggtcgcgtcacgatgacccgtgacactagcacctctaccgtttatatggagctgtccagcctgcgttctgaagatactgcagtgtactactgtgcacgcggtgacttcgcttggctggactattggggtcaaggcaccctcgtaacggtttcttct

SEQ ID NO: 172 - DNA, 336 bp, synthetic construct
  misc_feature 1..336: note = source = /note="Description of Artificial Sequence: Syntheticpolynucleotide"
  source 1..336: mol_type = other DNA
gatattgttatgactcaatctccactgtctctgccggtgactccaggcgaaccggcgagcatttcttgccgttccagccagtctctgctgcactccaacggctacaactatctcgattggtacctgcaaaaaccgggtcagagccctcagctgctgatctacctgggctctaaccgcgcttccggtgtaccggaccgtttcagcggctctggatccggcaccgatttcacgttgaaaatcagccgtgttgaagcagaagacgtgggcgtttattactgtatgcaggcaagcattatgaaccggacttttggtcaaggcaccaaggtcgaaattaaa

SEQ ID NO: 173 - DNA, 336 bp, synthetic construct
  misc_feature 1..336: note = source = /note="Description of Artificial Sequence: Syntheticpolynucleotide"
  source 1..336: mol_type = other DNA
gatattgttatgactcaatctccactgtctctgccggtgactccaggcgaaccggcgagcatttcttgccgttccagccagtctctgctgcactccaacggctacaactatctcgattggtacctgcaaaaaccgggtcagagccctcagctgctgatctacctgggctctaaccgcgcttccggtgtaccggaccgtttcagcggctctggatccggcaccgatttcacgttgaaaatcagccgtgttgaagcagaagacgtgggcgtttattactgtatgcaggcaagcattatgagccggacttttggtcaaggcaccaaggtcgaaattaaa

SEQ ID NO: 174 - DNA, 336 bp, synthetic construct
  misc_feature 1..336: note = source = /note="Description of Artificial Sequence: Syntheticpolynucleotide"
  source 1..336: mol_type = other DNA
gatattgttatgactcaatctccactgtctctgccggtgactccaggcgaaccggcgagcatttcttgccgttccagccagtctctgctgcactccaacggctacaactatctcgattggtacctgcaaaaaccgggtcagagccctcagctgctgatctacctgggctctaaccgcgcttccggtgtaccggaccgtttcagcggctctggatccggcaccgatttcacgttgaaaatcagccgtgttgaagcagaagacgtgggcgtttattactgtatgcaggcaagcattatgcagcggacttttggtcaaggcaccaaggtcgaaattaaa

SEQ ID NO: 175 - DNA, 336 bp, synthetic construct
  misc_feature 1..336: note = source = /note="Description of Artificial Sequence: Syntheticpolynucleotide"
  source 1..336: mol_type = other DNA
gatattgttatgactcaatctccactgtctctgccggtgactccaggcgaaccggcgagcatttcttgccgttccagccagtctctgctgcactccaacggctacaactatctcgattggtacctgcaaaaaccgggtcagagccctcagctgctgatctacctgggctctaaccgcgcttccggtgtaccggaccgtttcagcggctctggatccggcaccgatttcacgttgaaaatcagccgtgttgaagcagaagacgtgggcgtttattactgtatgcaggcaagcattatgaaccgggcttttggtcaaggcaccaaggtcgaaattaaa

SEQ ID NO: 176 - DNA, 336 bp, synthetic construct
  misc_feature 1..336: note = source = /note="Description of Artificial Sequence: Syntheticpolynucleotide"
  source 1..336: mol_type = other DNA
gatattgttatgactcaatctccactgtctctgccggtgactccaggcgaaccggcgagcatttcttgccgttccagccagtctctgctgcactccaacggctacaactatctcgattggtacctgcaaaaaccgggtcagagccctcagctgctgatctacctgggctctaaccgcgcttccggtgtaccggaccgtttcagcggctctggatccggcaccgatttcacgttgaaaatcagccgtgttgaagcagaagacgtgggcgtttattactgtatgcaggcaagcattatgaaccggaattttggtcaaggcaccaaggtcgaaattaaa

SEQ ID NO: 177 - DNA, 348 bp, synthetic construct
  misc_feature 1..348: note = source = /note="Description of Artificial Sequence: Syntheticpolynucleotide"
  source 1..348: mol_type = other DNA
caggtgcaattggttcaatctggtgctgaagtaaaaaaaccgggcgcttccgttaaagtgagctgcaaagcatccggatacaccttcacttcctattacatgcactgggttcgtcaagccccgggccagggtctggaatggatgggcatcattaacccaagcggtggctctacctcctacgcgcagaaattccagggtcgcgtcacgatgacccgtgacactagcacctctaccgtttatatggagctgtccagcctgcgttctgaagatactgcagtgtactactgtgcacgctcttacatcgacatggactattggggtcaaggcaccctcgtaacggtttcttct

SEQ ID NO: 178 - DNA, 321 bp, synthetic construct
  misc_feature 1..321: note = source = /note="Description of Artificial Sequence: Syntheticpolynucleotide"
  source 1..321: mol_type = other DNA
gaaatcgtgttaacgcagtctccaggcaccctgtctttgtctccaggggaaagagccaccctctcttgcagggccagtcagagtgttagcagcagctacttagcctggtaccagcagaaacctggccaggctcccaggctcctcatctatggagcatccagcagggccactggcatcccagacaggttcagtggcagtggatccgggacagacttcactctcaccatcagcagactggagcctgaagattttgcagtgtattactgtcagcaggataactggagcccaacgttcggccaggggaccaaagtggaaatcaaa

SEQ ID NO: 179 - DNA, 348 bp, synthetic construct
  misc_feature 1..348: note = source = /note="Description of Artificial Sequence: Syntheticpolynucleotide"
  source 1..348: mol_type = other DNA
caggtgcaattggttcaatctggtgctgaagtaaaaaaaccgggcgcttccgttaaagtgagctgcaaagcatccggatacaccttcacttcctattacatgcactgggttcgtcaagccccgggccagggtctggaatggatgggcatcattaacccaagcggtggctctacctcctacgcgcagaaattccagggtcgcgtcacgatgacccgtgacactagcacctctaccgtttatatggagctgtccagcctgcgttctgaagatactgcagtgtactactgtgcacgctcttacgttgacatggactattggggtcaaggcaccctcgtaacggtttcttct

SEQ ID NO: 180 - DNA, 321 bp, synthetic construct
  misc_feature 1..321: note = source = /note="Description of Artificial Sequence: Syntheticpolynucleotide"
  source 1..321: mol_type = other DNA
gaaatcgtgttaacgcagtctccaggcaccctgtctttgtctccaggggaaagagccaccctctcttgcagggccagtcagagtgttagcagcagctacctagcctggtaccagcagaaacctggccaggctcccaggctcctcatctatggagcatccagcagggccactggcatcccagacaggttcagtggcagtggatccgggacagacttcactctcaccatcagcagactggagcctgaagattttgcagtgtattactgtcagcaggatatttggagcccaacgttcggccaggggaccaaagtggaaatcaaa

SEQ ID NO: 181 - DNA, 363 bp, synthetic construct
  misc_feature 1..363: note = source = /note="Description of Artificial Sequence: Syntheticpolynucleotide"
  source 1..363: mol_type = other DNA
gaggtgcaattgttggagtctgggggaggcttggtacagcctggggggtccctgagactctcctgtgcagcctccggattcacctttagcagttatgccatgagctgggtccgccaggctccagggaaggggctggagtgggtctcagctattagtggtagtggtggtagcacatactacgcagactccgtgaagggccggttcaccatctccagagacaattccaagaacacgctgtatctgcagatgaacagcctgagagccgaggacacggccgtatattactgtgcgaaagactcttcttacgttgaatggtacgctttcgactactggggccaaggaaccctggtcaccgtctcgagt

SEQ ID NO: 182 - DNA, 324 bp, synthetic construct
  misc_feature 1..324: note = source = /note="Description of Artificial Sequence: Syntheticpolynucleotide"
  source 1..324: mol_type = other DNA
gaaatcgtgttaacgcagtctccaggcaccctgtctttgtctccaggggaaagagccaccctctcttgcagggccagtcagagtgttagcagcagctacttagcctggtaccagcagaaacctggccaggctcccaggctcctcatctatggagcatccagcagggccactggcatcccagacaggttcagtggcagtggatccgggacagactccactctcaccatcagcagactggagcctgaagattttgcagtgtattactgtcagcagccaaccagcagcccaattacgttcggccaggggaccaaagtggaaatcaaa

SEQ ID NO: 183 - DNA, 684 bp, synthetic construct
  misc_feature 1..684: note = source = /note="Description of Artificial Sequence: Syntheticpolynucleotide"
  source 1..684: mol_type = other DNA
gaggtgcagctgctggaatctggcggcggactggtgcagcctggcggatctctgagactgagctgtgccgccagcggcttcaccttcagcacctacgccatgaactgggtgcgccaggcccctggcaaaggcctggaatgggtgtcccggatcagaagcaagtacaacaactacgccacctactacgccgacagcgtgaagggccggttcaccatcagccgggacgacagcaagaacaccctgtacctgcagatgaacagcctgcgggccgaggacaccgccgtgtactattgtgtgcggcacggcaacttcggcaacagctatgtgtcttggtttgcctactggggccagggcaccctcgtgaccgtgtcaagcgctagtaccaagggccccagcgtgttccccctggcacccagcagcaagagcacatctggcggaacagccgctctgggctgtctggtgaaagactacttccccgagcccgtgaccgtgtcttggaactctggcgccctgaccagcggcgtgcacacctttccagccgtgctgcagagcagcggcctgtactccctgtcctccgtggtcaccgtgccctctagctccctgggaacacagacatatatctgtaatgtcaatcacaagccttccaacaccaaagtcgataagaaagtcgagcccaagagctgc

SEQ ID NO: 184 - DNA, 696 bp, synthetic construct
  misc_feature 1..696: note = source = /note="Description of Artificial Sequence: Syntheticpolynucleotide"
  source 1..696: mol_type = other DNA
gaggtgcagctgctggaatctggcggcggactggtgcagcctggcggatctctgagactgagctgtgccgccagcggcttcaccttcagcacctacgccatgaactgggtgcgccaggcccctggcaaaggcctggaatgggtgtcccggatcagaagcaagtacaacaactacgccacctactacgccgacagcgtgaagggccggttcaccatcagccgggacgacagcaagaacaccctgtacctgcagatgaacagcctgcgggccgaggacaccgccgtgtactattgtgtgcggcacggcaacttcggcaacagctatgtgtcttggtttgcctactggggccagggcaccctcgtgaccgtgtcaagcgctagtgtggccgctccctccgtgtttatctttcccccatccgatgaacagctgaaaagcggcaccgcctccgtcgtgtgtctgctgaacaatttttaccctagggaagctaaagtgcagtggaaagtggataacgcactgcagtccggcaactcccaggaatctgtgacagaacaggactccaaggacagcacctactccctgtcctccaccctgacactgtctaaggctgattatgagaaacacaaagtctacgcctgcgaagtcacccatcagggcctgagctcgcccgtcacaaagagcttcaacaggggagagtgt

SEQ ID NO: 185 - DNA, 36 bp, synthetic construct
  misc_feature 1..36: note = source = /note="Description of Artificial Sequence: Syntheticprimer"
  source 1..36: mol_type = other DNA
gcaggcaagcattatgcagcggacttttggtcaagg

SEQ ID NO: 186 - DNA, 35 bp, synthetic construct
  misc_feature 1..35: note = source = /note="Description of Artificial Sequence: Syntheticprimer"
  source 1..35: mol_type = other DNA
caggcaagcattatgagccggacttttggtcaagg

SEQ ID NO: 187 - DNA, 37 bp, synthetic construct
  misc_feature 1..37: note = source = /note="Description of Artificial Sequence: Syntheticprimer"
  source 1..37: mol_type = other DNA
cattatgaaccgggcttttggtcaaggcaccaaggtc

SEQ ID NO: 188 - DNA, 37 bp, synthetic construct
  misc_feature 1..37: note = source = /note="Description of Artificial Sequence: Syntheticprimer"
  source 1..37: mol_type = other DNA
cattatgaaccggaattttggtcaaggcaccaaggtc

SEQ ID NO: 189 - DNA, 2067 bp, synthetic construct
  misc_feature 1..2067: note = source = /note="Description of Artificial Sequence: Syntheticpolynucleotide"
  source 1..2067: mol_type = other DNA
gaggtgcaattggttgaatctggtggtggtctggtaaaaccgggcggttccctgcgtctgagctgcgcggcttccggattcaccttctccaacgcgtggatgagctgggttcgccaggccccgggcaaaggcctcgagtgggttggtcgtatcaagtctaaaactgacggtggcaccacggattacgcggctccagttaaaggtcgttttaccatttcccgcgacgatagcaaaaacactctgtatctgcagatgaactctctgaaaactgaagacaccgcagtctactactgtactaccccgtgggaatggtcttggtacgattattggggccagggcacgctggttacggtgtcttccgctagcacaaagggccctagcgtgttccctctggcccccagcagcaagagcacaagcggcggaacagccgccctgggctgcctcgtgaaggactacttccccgagcccgtgacagtgtcttggaacagcggagccctgacaagcggcgtgcacactttccctgccgtgctgcagagcagcggcctgtactccctgagcagcgtggtcaccgtgcctagcagcagcctgggcacccagacctacatctgcaacgtgaaccacaagcccagcaacaccaaagtggacaagaaggtggagcccaagagctgtgatggcggaggagggtccggaggcggaggatccgaggtgcagctgctggaatctggcggcggactggtgcagcctggcggatctctgagactgagctgtgccgccagcggcttcaccttcagcacctacgccatgaactgggtgcgccaggcccctggcaaaggcctggaatgggtgtcccggatcagaagcaagtacaacaactacgccacctactacgccgacagcgtgaagggccggttcaccatcagccgggacgacagcaagaacaccctgtacctgcagatgaacagcctgcgggccgaggacaccgccgtgtactattgtgtgcggcacggcaacttcggcaacagctatgtgtcttggtttgcctactggggccagggcaccctcgtgaccgtgtcaagcgctagtaccaagggccccagcgtgttccccctggcacccagcagcaagagcacatctggcggaacagccgctctgggctgtctggtgaaagactacttccccgagcccgtgaccgtgtcttggaactctggcgccctgaccagcggcgtgcacacctttccagccgtgctgcagagcagcggcctgtactccctgtcctccgtggtcaccgtgccctctagctccctgggaacacagacatatatctgtaatgtcaatcacaagccttccaacaccaaagtcgataagaaagtcgagcccaagagctgcgacaaaactcacacatgcccaccgtgcccagcacctgaagctgcagggggaccgtcagtcttcctcttccccccaaaacccaaggacaccctcatgatctcccggacccctgaggtcacatgcgtggtggtggacgtgagccacgaagaccctgaggtcaagttcaactggtacgtggacggcgtggaggtgcataatgccaagacaaagccgcgggaggagcagtacaacagcacgtaccgtgtggtcagcgtcctcaccgtcctgcaccaggactggctgaatggcaaggagtacaagtgcaaggtctccaacaaagccctcggcgcccccatcgagaaaaccatctccaaagccaaagggcagccccgagaaccacaggtgtacaccctgcccccatgccgggatgagctgaccaagaaccaggtcagcctgtggtgcctggtcaaaggcttctatcccagcgacatcgccgtggagtgggagagcaatgggcagccggagaacaactacaagaccacgcctcccgtgctggactccgacggctccttcttcctctacagcaagctcaccgtggacaagagcaggtggcagcaggggaacgtcttctcatgctccgtgatgcatgaggctctgcacaaccactacacgcagaagagcctctccctgtctccgggtaaa

SEQ ID NO: 190 - DNA, 1350 bp, synthetic construct
  misc_feature 1..1350: note = source = /note="Description of Artificial Sequence: Syntheticpolynucleotide"
  source 1..1350: mol_type = other DNA
gaggtgcaattggttgaatctggtggtggtctggtaaaaccgggcggttccctgcgtctgagctgcgcggcttccggattcaccttctccaacgcgtggatgagctgggttcgccaggccccgggcaaaggcctcgagtgggttggtcgtatcaagtctaaaactgacggtggcaccacggattacgcggctccagttaaaggtcgttttaccatttcccgcgacgatagcaaaaacactctgtatctgcagatgaactctctgaaaactgaagacaccgcagtctactactgtactaccccgtgggaatggtcttggtacgattattggggccagggcacgctggttacggtgtcttccgctagcaccaagggcccctccgtgttccccctggcccccagcagcaagagcaccagcggcggcacagccgctctgggctgcctggtcaaggactacttccccgagcccgtgaccgtgtcctggaacagcggagccctgacctccggcgtgcacaccttccccgccgtgctgcagagttctggcctgtatagcctgagcagcgtggtcaccgtgccttctagcagcctgggcacccagacctacatctgcaacgtgaaccacaagcccagcaacaccaaggtggacaagaaggtggagcccaagagctgcgacaaaactcacacatgcccaccgtgcccagcacctgaagctgcagggggaccgtcagtcttcctcttccccccaaaacccaaggacaccctcatgatctcccggacccctgaggtcacatgcgtggtggtggacgtgagccacgaagaccctgaggtcaagttcaactggtacgtggacggcgtggaggtgcataatgccaagacaaagccgcgggaggagcagtacaacagcacgtaccgtgtggtcagcgtcctcaccgtcctgcaccaggactggctgaatggcaaggagtacaagtgcaaggtctccaacaaagccctcggcgcccccatcgagaaaaccatctccaaagccaaagggcagccccgagaaccacaggtgtgcaccctgcccccatcccgggatgagctgaccaagaaccaggtcagcctctcgtgcgcagtcaaaggcttctatcccagcgacatcgccgtggagtgggagagcaatgggcagccggagaacaactacaagaccacgcctcccgtgctggactccgacggctccttcttcctcgtgagcaagctcaccgtggacaagagcaggtggcagcaggggaacgtcttctcatgctccgtgatgcatgaggctctgcacaaccgcttcacgcagaagagcctctccctgtctccgggtaaa

SEQ ID NO: 191 - DNA, 645 bp, synthetic construct
  misc_feature 1..645: note = source = /note="Description of Artificial Sequence: Syntheticpolynucleotide"
  source 1..645: mol_type = other DNA
caggccgtcgtgacccaggaacccagcctgacagtgtctcctggcggcaccgtgaccctgacatgtggcagttctacaggcgccgtgaccaccagcaactacgccaactgggtgcaggaaaagcccggccaggccttcagaggactgatcggcggcaccaacaagagagcccctggcacccctgccagattcagcggatctctgctgggaggaaaggccgccctgacactgtctggcgcccagccagaagatgaggccgagtactactgcgccctgtggtacagcaacctgtgggtgttcggcggaggcaccaagctgacagtcctaggtcaacccaaggctgcccccagcgtgaccctgttcccccccagcagcgaggaactgcaggccaacaaggccaccctggtctgcctgatcagcgacttctacccaggcgccgtgaccgtggcctggaaggccgacagcagccccgtgaaggccggcgtggagaccaccacccccagcaagcagagcaacaacaagtacgccgccagcagctacctgagcctgacccccgagcagtggaagagccacaggtcctacagctgccaggtgacccacgagggcagcaccgtggagaaaaccgtggcccccaccgagtgcagc

SEQ ID NO: 192 - DNA, 2067 bp, synthetic construct
  misc_feature 1..2067: note = source = /note="Description of Artificial Sequence: Syntheticpolynucleotide"
  source 1..2067: mol_type = other DNA
gaggtgcagctgctggaatctggcggcggactggtgcagcctggcggatctctgagactgagctgtgccgccagcggcttcaccttcagcacctacgccatgaactgggtgcgccaggcccctggcaaaggcctggaatgggtgtcccggatcagaagcaagtacaacaactacgccacctactacgccgacagcgtgaagggccggttcaccatcagccgggacgacagcaagaacaccctgtacctgcagatgaacagcctgcgggccgaggacaccgccgtgtactattgtgtgcggcacggcaacttcggcaacagctatgtgtcttggtttgcctactggggccagggcaccctcgtgaccgtgtcatctgctagcacaaagggccctagcgtgttccctctggcccccagcagcaagagcacaagcggcggaacagccgccctgggctgcctcgtgaaggactacttccccgagcccgtgacagtgtcttggaacagcggagccctgacaagcggcgtgcacaccttccctgccgtgctgcagagcagcggcctgtactccctgagcagcgtggtcaccgtgcctagcagcagcctgggcacccagacctacatctgcaacgtgaaccacaagcccagcaacaccaaagtggacaagaaggtggagcccaagagctgtgatggcggaggagggtccggaggcggaggatccgaggtgcaattggttgaatctggtggtggtctggtaaaaccgggcggttccctgcgtctgagctgcgcggcttccggattcaccttctccaacgcgtggatgagctgggttcgccaggccccgggcaaaggcctcgagtgggttggtcgtatcaagtctaaaactgacggtggcaccacggattacgcggctccagttaaaggtcgttttaccatttcccgcgacgatagcaaaaacactctgtatctgcagatgaactctctgaaaactgaagacaccgcagtctactactgtactaccccgtgggaatggtcttggtacgattattggggccagggcacgctggttacggtgtctagcgctagtaccaagggccccagcgtgttccccctggcacccagcagcaagagcacatctggcggaacagccgctctgggctgtctggtgaaagactacttccccgagcccgtgaccgtgtcttggaactctggcgccctgaccagcggcgtgcacacctttccagccgtgctgcagagcagcggcctgtactccctgtcctccgtggtcaccgtgccctctagctccctgggaacacagacatatatctgtaatgtcaatcacaagccttccaacaccaaagtcgataagaaagtcgagcccaagagctgcgacaaaactcacacatgcccaccgtgcccagcacctgaagctgcagggggaccgtcagtcttcctcttccccccaaaacccaaggacaccctcatgatctcccggacccctgaggtcacatgcgtggtggtggacgtgagccacgaagaccctgaggtcaagttcaactggtacgtggacggcgtggaggtgcataatgccaagacaaagccgcgggaggagcagtacaacagcacgtaccgtgtggtcagcgtcctcaccgtcctgcaccaggactggctgaatggcaaggagtacaagtgcaaggtctccaacaaagccctcggcgcccccatcgagaaaaccatctccaaagccaaagggcagccccgagaaccacaggtgtacaccctgcccccatgccgggatgagctgaccaagaaccaggtcagcctgtggtgcctggtcaaaggcttctatcccagcgacatcgccgtggagtgggagagcaatgggcagccggagaacaactacaagaccacgcctcccgtgctggactccgacggctccttcttcctctacagcaagctcaccgtggacaagagcaggtggcagcaggggaacgtcttctcatgctccgtgatgcatgaggctctgcacaaccactacacgcagaagagcctctccctgtctccgggtaaa

SEQ ID NO: 193 - DNA, 1365 bp, synthetic construct
  misc_feature 1..1365: note = source = /note="Description of Artificial Sequence: Syntheticpolynucleotide"
  source 1..1365: mol_type = other DNA
gaggtgcagctgctggaatctggcggcggactggtgcagcctggcggatctctgagactgagctgtgccgccagcggcttcaccttcagcacctacgccatgaactgggtgcgccaggcccctggcaaaggcctggaatgggtgtcccggatcagaagcaagtacaacaactacgccacctactacgccgacagcgtgaagggccggttcaccatcagccgggacgacagcaagaacaccctgtacctgcagatgaacagcctgcgggccgaggacaccgccgtgtactattgtgtgcggcacggcaacttcggcaacagctatgtgtcttggtttgcctactggggccagggcaccctcgtgaccgtgtcatctgctagcaccaagggcccatcggtcttccccctggcaccctcctccaagagcacctctgggggcacagcggccctgggctgcctggtcaaggactacttccccgaaccggtgacggtgtcgtggaactcaggcgccctgaccagcggcgtgcacaccttcccggctgtcctacagtcctcaggactctactccctcagcagcgtggtgaccgtgccctccagcagcttgggcacccagacctacatctgcaacgtgaatcacaagcccagcaacaccaaggtggacaagaaagttgagcccaaatcttgtgacaaaactcacacatgcccaccgtgcccagcacctgaagctgcagggggaccgtcagtcttcctcttccccccaaaacccaaggacaccctcatgatctcccggacccctgaggtcacatgcgtggtggtggacgtgagccacgaagaccctgaggtcaagttcaactggtacgtggacggcgtggaggtgcataatgccaagacaaagccgcgggaggagcagtacaacagcacgtaccgtgtggtcagcgtcctcaccgtcctgcaccaggactggctgaatggcaaggagtacaagtgcaaggtctccaacaaagccctcggcgcccccatcgagaaaaccatctccaaagccaaagggcagccccgagaaccacaggtgtacaccctgcccccatgccgggatgagctgaccaagaaccaggtcagcctgtggtgcctggtcaaaggcttctatcccagcgacatcgccgtggagtgggagagcaatgggcagccggagaacaactacaagaccacgcctcccgtgctggactccgacggctccttcttcctctacagcaagctcaccgtggacaagagcaggtggcagcaggggaacgtcttctcatgctccgtgatgcatgaggctctgcacaaccactacacgcagaagagcctctccctgtctccgggtaaa

SEQ ID NO: 194 - DNA, 681 bp, synthetic construct
  misc_feature 1..681: note = source = /note="Description of Artificial Sequence: Syntheticpolynucleotide"
  source 1..681: mol_type = other DNA
gacaaaactcacacatgcccaccgtgcccagcacctgaactcctggggggaccgtcagtcttcctcttccccccaaaacccaaggacaccctcatgatctcccggacccctgaggtcacatgcgtggtggtggacgtgagccacgaagaccctgaggtcaagttcaactggtacgtggacggcgtggaggtgcataatgccaagacaaagccgcgggaggagcagtacaacagcacgtaccgtgtggtcagcgtcctcaccgtcctgcaccaggactggctgaatggcaaggagtacaagtgcaaggtctccaacaaagccctcccagcccccatcgagaaaaccatctccaaagccaaagggcagccccgagaaccacaggtgtgcaccctgcccccatcccgggatgagctgaccaagaaccaggtcagcctctcgtgcgcagtcaaaggcttctatcccagcgacatcgccgtggagtgggagagcaatgggcagccggagaacaactacaagaccacgcctcccgtgctggactccgacggctccttcttcctcgtgagcaagctcaccgtggacaagagcaggtggcagcaggggaacgtcttctcatgctccgtgatgcatgaggctctgcacaaccgcttcacgcagaagagcctctccctgtctccgggtaaa

SEQ ID NO: 195 - DNA, 2070 bp, synthetic construct
  misc_feature 1..2070: note = source = /note="Description of Artificial Sequence: Syntheticpolynucleotide"
  source 1..2070: mol_type = other DNA
caggtgcaattggttcaatctggtgctgaagtaaaaaaaccgggcgcttccgttaaagtgagctgcaaagcatccggatacaccttcacttcctattacatgcactgggttcgtcaagccccgggccagggtctggaatggatgggcatcattaacccaagcggtggccctacctcctacgcgcagaaattccagggtcgcgtcacgatgacccgtgacactagcacctctaccgtttatatggagctgtccagcctgcgttctgaagatactgcagtgtactactgtgcacgcggtgacttcgcttggctggactattggggtcaaggcaccctcgtaacggtttcttctgctagcacaaagggccccagcgtgttccctctggcccctagcagcaagagcacatctggcggaacagccgccctgggctgcctcgtgaaggactactttcccgagcctgtgaccgtgtcctggaactctggcgccctgacaagcggcgtgcacacctttccagccgtgctgcagagcagcggcctgtactctctgagcagcgtggtcaccgtgcctagcagcagcctgggcacccagacctacatctgcaacgtgaaccacaagcccagcaacaccaaagtggacaagaaggtggagcccaagagctgtgatggcggaggagggtccggaggcggaggatccgaggtgcagctgctggaatctggcggcggactggtgcagcctggcggatctctgagactgagctgtgccgccagcggcttcaccttcagcacctacgccatgaactgggtgcgccaggcccctggcaaaggcctggaatgggtgtcccggatcagaagcaagtacaacaactacgccacctactacgccgacagcgtgaagggccggttcaccatcagccgggacgacagcaagaacaccctgtacctgcagatgaacagcctgcgggccgaggacaccgccgtgtactattgtgtgcggcacggcaacttcggcaacagctatgtgtcttggtttgcctactggggccagggcaccctcgtgaccgtgtcaagcgctagtgtggccgctccctccgtgtttatctttcccccatccgatgaacagctgaaaagcggcaccgcctccgtcgtgtgtctgctgaacaatttttaccctagggaagctaaagtgcagtggaaagtggataacgcactgcagtccggcaactcccaggaatctgtgacagaacaggactccaaggacagcacctactccctgtcctccaccctgacactgtctaaggctgattatgagaaacacaaagtctacgcctgcgaagtcacccatcagggcctgagctcgcccgtcacaaagagcttcaacaggggagagtgtgacaagacccacacctgtcccccttgtcctgcccctgaagctgctggcggcccttctgtgttcctgttccccccaaagcccaaggacaccctgatgatcagccggacccccgaagtgacctgcgtggtggtggatgtgtcccacgaggaccctgaagtgaagttcaattggtacgtggacggcgtggaagtgcacaacgccaagacaaagccgcgggaggagcagtacaacagcacgtaccgtgtggtcagcgtcctcaccgtcctgcaccaggactggctgaatggcaaggagtacaagtgcaaggtctccaacaaagccctcggcgcccccatcgagaaaaccatctccaaagccaaagggcagccccgagaaccacaggtgtacaccctgcccccatgccgggatgagctgaccaagaaccaggtcagcctgtggtgcctggtcaaaggcttctatcccagcgacatcgccgtggagtgggagagcaatgggcagccggagaacaactacaagaccacgcctcccgtgctggactccgacggctccttcttcctctacagcaagctcaccgtggacaagagcaggtggcagcaggggaacgtcttctcatgctccgtgatgcatgaggctctgcacaaccactacacgcagaagagcctctccctgtctccgggtaaa

SEQ ID NO: 196 - DNA, 1341 bp, synthetic construct
  misc_feature 1..1341: note = source = /note="Description of Artificial Sequence: Syntheticpolynucleotide"
  source 1..1341: mol_type = other DNA
caggtgcaattggttcaatctggtgctgaagtaaaaaaaccgggcgcttccgttaaagtgagctgcaaagcatccggatacaccttcacttcctattacatgcactgggttcgtcaagccccgggccagggtctggaatggatgggcatcattaacccaagcggtggccctacctcctacgcgcagaaattccagggtcgcgtcacgatgacccgtgacactagcacctctaccgtttatatggagctgtccagcctgcgttctgaagatactgcagtgtactactgtgcacgcggtgacttcgcttggctggactattggggtcaaggcaccctcgtaacggtttcttctgctagcaccaagggcccctccgtgttccccctggcccccagcagcaagagcaccagcggcggcacagccgctctgggctgcctggtcaaggactacttccccgagcccgtgaccgtgtcctggaacagcggagccctgacctccggcgtgcacaccttccccgccgtgctgcagagttctggcctgtatagcctgagcagcgtggtcaccgtgccttctagcagcctgggcacccagacctacatctgcaacgtgaaccacaagcccagcaacaccaaggtggacaagaaggtggagcccaagagctgcgacaaaactcacacatgcccaccgtgcccagcacctgaagctgcagggggaccgtcagtcttcctcttccccccaaaacccaaggacaccctcatgatctcccggacccctgaggtcacatgcgtggtggtggacgtgagccacgaagaccctgaggtcaagttcaactggtacgtggacggcgtggaggtgcataatgccaagacaaagccgcgggaggagcagtacaacagcacgtaccgtgtggtcagcgtcctcaccgtcctgcaccaggactggctgaatggcaaggagtacaagtgcaaggtctccaacaaagccctcggcgcccccatcgagaaaaccatctccaaagccaaagggcagccccgagaaccacaggtgtgcaccctgcccccatcccgggatgagctgaccaagaaccaggtcagcctctcgtgcgcagtcaaaggcttctatcccagcgacatcgccgtggagtgggagagcaatgggcagccggagaacaactacaagaccacgcctcccgtgctggactccgacggctccttcttcctcgtgagcaagctcaccgtggacaagagcaggtggcagcaggggaacgtcttctcatgctccgtgatgcatgaggctctgcacaaccactacacgcagaagagcctctccctgtctccgggtaaa

SEQ ID NO: 197 - DNA, 657 bp, synthetic construct
  misc_feature 1..657: note = source = /note="Description of Artificial Sequence: Syntheticpolynucleotide"
  source 1..657: mol_type = other DNA
gatattgttatgactcaatctccactgtctctgccggtgactccaggcgaaccggcgagcatttcttgccgttccagccagtctctgctgcactccaacggctacaactatctcgattggtacctgcaaaaaccgggtcagagccctcagctgctgatctacctgggctctaaccgcgcttccggtgtaccggaccgtttcagcggctctggatccggcaccgatttcacgttgaaaatcagccgtgttgaagcagaagacgtgggcgtttattactgtatgcaggcaagcattatgaaccggacttttggtcaaggcaccaaggtcgaaattaaacgtacggtggctgcaccatctgtcttcatcttcccgccatctgatgagcagttgaaatctggaactgcctctgttgtgtgcctgctgaataacttctatcccagagaggccaaagtacagtggaaggtggataacgccctccaatcgggtaactcccaggagagtgtcacagagcaggacagcaaggacagcacctacagcctcagcagcaccctgacgctgagcaaagcagactacgagaaacacaaagtctacgcctgcgaagtcacccatcagggcctgagctcgcccgtcacaaagagcttcaacaggggagagtgt

SEQ ID NO: 198 - DNA, 642 bp, synthetic construct
  misc_feature 1..642: note = source = /note="Description of Artificial Sequence: Syntheticpolynucleotide"
  source 1..642: mol_type = other DNA
caggccgtcgtgacccaggaacccagcctgacagtgtctcctggcggcaccgtgaccctgacatgtggcagttctacaggcgccgtgaccaccagcaactacgccaactgggtgcaggaaaagcccggccaggccttcagaggactgatcggcggcaccaacaagagagcccctggcacccctgccagattcagcggatctctgctgggaggaaaggccgccctgacactgtctggcgcccagccagaagatgaggccgagtactactgcgccctgtggtacagcaacctgtgggtgttcggcggaggcaccaagctgacagtgctgagcagcgcttccaccaaaggcccttccgtgtttcctctggctcctagctccaagtccacctctggaggcaccgctgctctcggatgcctcgtgaaggattattttcctgagcctgtgacagtgtcctggaatagcggagcactgacctctggagtgcatactttccccgctgtgctgcagtcctctggactgtacagcctgagcagcgtggtgacagtgcccagcagcagcctgggcacccagacctacatctgcaacgtgaaccacaagcccagcaacaccaaggtggacaagaaggtggaacccaagtcttgt

SEQ ID NO: 199 - DNA, 1377 bp, synthetic construct
  misc_feature 1..1377: note = source = /note="Description of Artificial Sequence: Syntheticpolynucleotide"
  source 1..1377: mol_type = other DNA
gaggtgcagctgctggaatctggcggcggactggtgcagcctggcggatctctgagactgagctgtgccgccagcggcttcaccttcagcacctacgccatgaactgggtgcgccaggcccctggcaaaggcctggaatgggtgtcccggatcagaagcaagtacaacaactacgccacctactacgccgacagcgtgaagggccggttcaccatcagccgggacgacagcaagaacaccctgtacctgcagatgaacagcctgcgggccgaggacaccgccgtgtactattgtgtgcggcacggcaacttcggcaacagctatgtgtcttggtttgcctactggggccagggcaccctcgtgaccgtgtcatctgctagcgtggccgctccctccgtgtttatctttcccccatccgatgaacagctgaaaagcggcaccgcctccgtcgtgtgtctgctgaacaatttttaccctagggaagctaaagtgcagtggaaagtggataacgcactgcagtccggcaactcccaggaatctgtgacagaacaggactccaaggacagcacctactccctgtcctccaccctgacactgtctaaggctgattatgagaaacacaaagtctacgcctgcgaagtcacccatcagggcctgagctcgcccgtcacaaagagcttcaacaggggagagtgtgacaagacccacacctgtcccccttgtcctgcccctgaagctgctggcggcccttctgtgttcctgttccccccaaagcccaaggacaccctgatgatcagccggacccccgaagtgacctgcgtggtggtggatgtgtcccacgaggaccctgaagtgaagttcaattggtacgtggacggcgtggaagtgcacaacgccaagacaaagccgcgggaggagcagtacaacagcacgtaccgtgtggtcagcgtcctcaccgtcctgcaccaggactggctgaatggcaaggagtacaagtgcaaggtctccaacaaagccctcggcgcccccatcgagaaaaccatctccaaagccaaagggcagccccgagaaccacaggtgtacaccctgcccccatgccgggatgagctgaccaagaaccaggtcagcctgtggtgcctggtcaaaggcttctatcccagcgacatcgccgtggagtgggagagcaatgggcagccggagaacaactacaagaccacgcctcccgtgctggactccgacggctccttcttcctctacagcaagctcaccgtggacaagagcaggtggcagcaggggaacgtcttctcatgctccgtgatgcatgaggctctgcacaaccactacacgcagaagagcctctccctgtctccgggtaaa

SEQ ID NO: 200 - DNA, 2067 bp, synthetic construct
  misc_feature 1..2067: note = source = /note="Description of Artificial Sequence: Syntheticpolynucleotide"
  source 1..2067: mol_type = other DNA
gaggtgcaattggttgaatctggtggtggtctggtaaaaccgggcggttccctgcgtctgagctgcgcggcttccggattcaccttctccaacgcgtggatgagctgggttcgccaggccccgggcaaaggcctcgagtgggttggtcgtatcaagtctaaaactgacggtggcaccacggattacgcggctccagttaaaggtcgttttaccatttcccgcgacgatagcaaaaacactctgtatctgcagatgaactctctgaaaactgaagacaccgcagtctactactgtactaccccgtgggaatggtcttggtacgattattggggccagggcacgctggttacggtgtcttccgctagcacaaagggccctagcgtgttccctctggcccccagcagcaagagcacaagcggcggaacagccgccctgggctgcctcgtgaaggactacttccccgagcccgtgacagtgtcttggaacagcggagccctgacaagcggcgtgcacactttccctgccgtgctgcagagcagcggcctgtactccctgagcagcgtggtcaccgtgcctagcagcagcctgggcacccagacctacatctgcaacgtgaaccacaagcccagcaacaccaaagtggacaagaaggtggagcccaagagctgtgatggcggaggagggtccggaggcggaggatccgaggtgcagctgctggaatctggcggcggactggtgcagcctggcggatctctgagactgagctgtgccgccagcggcttcaccttcagcacctacgccatgaactgggtgcgccaggcccctggcaaaggcctggaatgggtgtcccggatcagaagcaagtacaacaactacgccacctactacgccgacagcgtgaagggccggttcaccatcagccgggacgacagcaagaacaccctgtacctgcagatgaacagcctgcgggccgaggacaccgccgtgtactattgtgtgcggcacggcaacttcggcgccagctatgtgtcttggtttgcctactggggccagggcaccctcgtgaccgtgtcaagcgctagtaccaagggccccagcgtgttccccctggcacccagcagcaagagcacatctggcggaacagccgctctgggctgtctggtgaaagactacttccccgagcccgtgaccgtgtcttggaactctggcgccctgaccagcggcgtgcacacctttccagccgtgctgcagagcagcggcctgtactccctgtcctccgtggtcaccgtgccctctagctccctgggaacacagacatatatctgtaatgtcaatcacaagccttccaacaccaaagtcgataagaaagtcgagcccaagagctgcgacaaaactcacacatgcccaccgtgcccagcacctgaagctgcagggggaccgtcagtcttcctcttccccccaaaacccaaggacaccctcatgatctcccggacccctgaggtcacatgcgtggtggtggacgtgagccacgaagaccctgaggtcaagttcaactggtacgtggacggcgtggaggtgcataatgccaagacaaagccgcgggaggagcagtacaacagcacgtaccgtgtggtcagcgtcctcaccgtcctgcaccaggactggctgaatggcaaggagtacaagtgcaaggtctccaacaaagccctcggcgcccccatcgagaaaaccatctccaaagccaaagggcagccccgagaaccacaggtgtacaccctgcccccatgccgggatgagctgaccaagaaccaggtcagcctgtggtgcctggtcaaaggcttctatcccagcgacatcgccgtggagtgggagagcaatgggcagccggagaacaactacaagaccacgcctcccgtgctggactccgacggctccttcttcctctacagcaagctcaccgtggacaagagcaggtggcagcaggggaacgtcttctcatgctccgtgatgcatgaggctctgcacaaccactacacgcagaagagcctctccctgtctccgggtaaa

SEQ ID NO: 201 - DNA, 2067 bp, synthetic construct
  misc_feature 1..2067: note = source = /note="Description of Artificial Sequence: Syntheticpolynucleotide"
  source 1..2067: mol_type = other DNA
gaggtgcaattggttgaatctggtggtggtctggtaaaaccgggcggttccctgcgtctgagctgcgcggcttccggattcaccttctccaacgcgtggatgagctgggttcgccaggccccgggcaaaggcctcgagtgggttggtcgtatcaagtctaaaactgacggtggcaccacggattacgcggctccagttaaaggtcgttttaccatttcccgcgacgatagcaaaaacactctgtatctgcagatgaactctctgaaaactgaagacaccgcagtctactactgtactaccccgtgggaatggtcttggtacgattattggggccagggcacgctggttacggtgtcttccgctagcacaaagggccctagcgtgttccctctggcccccagcagcaagagcacaagcggcggaacagccgccctgggctgcctcgtgaaggactacttccccgagcccgtgacagtgtcttggaacagcggagccctgacaagcggcgtgcacactttccctgccgtgctgcagagcagcggcctgtactccctgagcagcgtggtcaccgtgcctagcagcagcctgggcacccagacctacatctgcaacgtgaaccacaagcccagcaacaccaaagtggacaagaaggtggagcccaagagctgtgatggcggaggagggtccggaggcggaggatccgaggtgcagctgctggaatctggcggcggactggtgcagcctggcggatctctgagactgagctgtgccgccagcggcttcaccttcagcacctacgccatgaactgggtgcgccaggcccctggcaaaggcctggaatgggtgtcccggatcagaagcaagtacaacaactacgccacctactacgccgacagcgtgaagggccggttcaccatcagccgggacgacagcaagaacaccctgtacctgcagatgaacagcctgcgggccgaggacaccgccgtgtactattgtgtgcggcacggcaacttcggcaacgcctatgtgtcttggtttgcctactggggccagggcaccctcgtgaccgtgtcaagcgctagtaccaagggccccagcgtgttccccctggcacccagcagcaagagcacatctggcggaacagccgctctgggctgtctggtgaaagactacttccccgagcccgtgaccgtgtcttggaactctggcgccctgaccagcggcgtgcacacctttccagccgtgctgcagagcagcggcctgtactccctgtcctccgtggtcaccgtgccctctagctccctgggaacacagacatatatctgtaatgtcaatcacaagccttccaacaccaaagtcgataagaaagtcgagcccaagagctgcgacaaaactcacacatgcccaccgtgcccagcacctgaagctgcagggggaccgtcagtcttcctcttccccccaaaacccaaggacaccctcatgatctcccggacccctgaggtcacatgcgtggtggtggacgtgagccacgaagaccctgaggtcaagttcaactggtacgtggacggcgtggaggtgcataatgccaagacaaagccgcgggaggagcagtacaacagcacgtaccgtgtggtcagcgtcctcaccgtcctgcaccaggactggctgaatggcaaggagtacaagtgcaaggtctccaacaaagccctcggcgcccccatcgagaaaaccatctccaaagccaaagggcagccccgagaaccacaggtgtacaccctgcccccatgccgggatgagctgaccaagaaccaggtcagcctgtggtgcctggtcaaaggcttctatcccagcgacatcgccgtggagtgggagagcaatgggcagccggagaacaactacaagaccacgcctcccgtgctggactccgacggctccttcttcctctacagcaagctcaccgtggacaagagcaggtggcagcaggggaacgtcttctcatgctccgtgatgcatgaggctctgcacaaccactacacgcagaagagcctctccctgtctccgggtaaa

SEQ ID NO: 202 - DNA, 1323 bp, synthetic construct
  misc_feature 1..1323: note = source = /note="Description of Artificial Sequence: Syntheticpolynucleotide"
  source 1..1323: mol_type = other DNA
caggccgtcgtgacccaggaacccagcctgacagtgtctcctggcggcaccgtgaccctgacatgtggcagttctacaggcgccgtgaccaccagcaactacgccaactgggtgcaggaaaagcccggccaggccttcagaggactgatcggcggcaccaacaagagagcccctggcacccctgccagattcagcggatctctgctgggaggaaaggccgccctgacactgtctggcgcccagccagaagatgaggccgagtactactgcgccctgtggtacagcaacctgtgggtgttcggcggaggcaccaagctgacagtgctgagcagcgctagcaccaagggcccatcggtcttccccctggcaccctcctccaagagcacctctgggggcacagcggccctgggctgcctggtcaaggactacttccccgaaccggtgacggtgtcgtggaactcaggcgccctgaccagcggcgtgcacaccttcccggctgtcctacagtcctcaggactctactccctcagcagcgtggtgaccgtgccctccagcagcttgggcacccagacctacatctgcaacgtgaatcacaagcccagcaacaccaaggtggacaagaaagttgagcccaaatcttgtgacaaaactcacacatgcccaccgtgcccagcacctgaagctgcagggggaccgtcagtcttcctcttccccccaaaacccaaggacaccctcatgatctcccggacccctgaggtcacatgcgtggtggtggacgtgagccacgaagaccctgaggtcaagttcaactggtacgtggacggcgtggaggtgcataatgccaagacaaagccgcgggaggagcagtacaacagcacgtaccgtgtggtcagcgtcctcaccgtcctgcaccaggactggctgaatggcaaggagtacaagtgcaaggtctccaacaaagccctcggcgcccccatcgagaaaaccatctccaaagccaaagggcagccccgagaaccacaggtgtacaccctgcccccatcccgggatgagctgaccaagaaccaggtcagcctgacctgcctggtcaaaggcttctatcccagcgacatcgccgtggagtgggagagcaatgggcagccggagaacaactacaagaccacgcctcccgtgctggactccgacggctccttcttcctctacagcaagctcaccgtggacaagagcaggtggcagcaggggaacgtcttctcatgctccgtgatgcatgaggctctgcacaaccactacacgcagaagagcctctccctgtctccgggtaaa

SEQ ID NO: 203 - DNA, 681 bp, synthetic construct
  misc_feature 1..681: note = source = /note="Description of Artificial Sequence: Syntheticpolynucleotide"
  source 1..681: mol_type = other DNA
gaggtgcaattggttgaatctggtggtggtctggtaaaaccgggcggttccctgcgtctgagctgcgcggcttccggattcaccttctccaacgcgtggatgagctgggttcgccaggccccgggcaaaggcctcgagtgggttggtcgtatcaagtctaaaactgacggtggcaccacggattacgcggctccagttaaaggtcgttttaccatttcccgcgacgatagcaaaaacactctgtatctgcagatgaactctctgaaaactgaagacaccgcagtctactactgtactaccccgtgggaatggtcttggtacgattattggggccagggcacgctggttacggtgtcttccgctagcgtggccgctccctccgtgttcatcttcccaccttccgacgagcagctgaagtccggcaccgcttctgtcgtgtgcctgctgaacaacttctacccccgcgaggccaaggtgcagtggaaggtggacaacgccctgcagtccggcaacagccaggaatccgtgaccgagcaggactccaaggacagcacctactccctgtcctccaccctgaccctgtccaaggccgactacgagaagcacaaggtgtacgcctgcgaagtgacccaccagggcctgtctagccccgtgaccaagtctttcaaccggggcgagtgc

SEQ ID NO: 204 - DNA, 693 bp, synthetic construct
  misc_feature 1..693: note = source = /note="Description of Artificial Sequence: Syntheticpolynucleotide"
  source 1..693: mol_type = other DNA
gaagtgcagctgctggaatccggcggaggactggtgcagcctggcggatctctgagactgtcttgtgccgcctccggcttcaccttctccacctacgccatgaactgggtgcgacaggctcctggcaagggcctggaatgggtgtcccggatcagatccaagtacaacaactacgccacctactacgccgactccgtgaagggccggttcaccatctctcgggacgactccaagaacaccctgtacctgcagatgaactccctgcgggccgaggacaccgccgtgtactattgtgtgcggcacggcaacttcggcaactcctatgtgtcttggtttgcctactggggccagggcaccctcgtgaccgtgtcatctgctagccccaaggctgcccccagcgtgaccctgtttccccccagcagcgaggaactgcaggccaacaaggccaccctggtctgcctgatcagcgacttctacccaggcgccgtgaccgtggcctggaaggccgacagcagccccgtgaaggccggcgtggagaccaccacccccagcaagcagagcaacaacaagtacgccgccagcagctacctgagcctgacccccgagcagtggaagagccacaggtcctacagctgccaggtgacccacgagggcagcaccgtggagaaaaccgtggcccccaccgagtgcagc

SEQ ID NO: 205 - DNA, 327 bp, synthetic construct
  misc_feature 1..327: note = source = /note="Description of Artificial Sequence: Syntheticpolynucleotide"
  source 1..327: mol_type = other DNA
cagaccgtcgtgacccaggaacccagcctgacagtgtctcctggcggcaccgtgaccctgacatgtggcagttctacaggcgccgtgaccaccagcaactacgccaactgggtgcagcagaagccaggccaggctcccagaggactgatcggcggcaccaacgccagagcccctggcacccctgccagattcagcggatctctgctgggaggaaaggccgccctgacactgtctggcgtgcagcctgaagatgaggccgagtactactgcgccctgtggtacagcaacctgtgggtgttcggcggaggcaccaagctgacagtccta

SEQ ID NO: 206 - DNA, 327 bp, synthetic construct
  misc_feature 1..327: note = source = /note="Description of Artificial Sequence: Syntheticpolynucleotide"
  source 1..327: mol_type = other DNA
cagaccgtcgtgacccaggaacccagcctgacagtgtctcctggcggcaccgtgaccctgacatgtggcagttctacaggcgccgtgaccaccagcaactacgccaactgggtgcagcagaagccaggccaggctcccagaggactgatcggcggcaccaacaagagagcccctggcacccctgccagattcagcggatctctgctgggaggaaaggccgccctgacactgtctggcgtgcagcctgaagatgaggccgagtactactgcgccctgtggtacgccaacctgtgggtgttcggcggaggcaccaagctgacagtccta

SEQ ID NO: 207 - DNA, 366 bp, synthetic construct
  misc_feature 1..366: note = source = /note="Description of Artificial Sequence: Syntheticpolynucleotide"
  source 1..366: mol_type = other DNA
gaggtgcaattggtggaaagcggaggcggcctcgtgaagcctggcggatctctgagactgagctgtgccgccagcggcttcaccttcagcaacgcctggatgcactgggtgcgccaggcccctggaaaaggactcgagtgggtgggacggatcaagagcaagaccgatggcggcaccaccgactatgccgcccctgtgaagggccggttcaccatcagcagggacgacagcaagaacaccctgtacctgcagatgaacagcctgaaaaccgaggacaccgccgtgtactactgcaccaccccctgggagtggtcttggtacgactattggggccagggcaccctcgtgaccgtgtcctctgctagc

SEQ ID NO: 208 - DNA, 366 bp, synthetic construct
  misc_feature 1..366: note = source = /note="Description of Artificial Sequence: Syntheticpolynucleotide"
  source 1..366: mol_type = other DNA
gaggtgcaattggtggaaagcggaggcggcctcgtgaagcctggcggatctctgagactgagctgtgccgccagcggcttcaccttcagcaacgcctggatgagctgggtgcgccaggcccctggaaaaggactcgagtgggtgtcccggatcaagagcaagaccgatggcggcaccaccgactatgccgcccctgtgaagggccggttcaccatcagcagggacgacagcaagaacaccctgtacctgcagatgaacagcctgaaaaccgaggacaccgccgtgtactactgcaccaccccctgggagtggtcttggtacgactattggggccagggcaccctcgtgaccgtgtcctctgctagc

SEQ ID NO: 209 - DNA, 366 bp, synthetic construct
  misc_feature 1..366: note = source = /note="Description of Artificial Sequence: Syntheticpolynucleotide"
  source 1..366: mol_type = other DNA
gaggtgcaattggtggaaagcggaggcggcctcgtgaagcctggcggatctctgagactgagctgtgccgccagcggcttcaccttcagcaacgcctggatgagctgggtgcgccaggcccctggaaaaggactcgagtgggtgggatctatcaagagcaagaccgacggcggcaccaccgactatgccgcccctgtgaagggccggttcaccatcagcagggacgacagcaagaacaccctgtacctgcagatgaacagcctgaaaaccgaggacaccgccgtgtactactgcaccaccccctgggagtggtcttggtacgactattggggccagggcaccctcgtgaccgtgtcctctgctagc

SEQ ID NO: 210 - DNA, 366 bp, synthetic construct
  misc_feature 1..366: note = source = /note="Description of Artificial Sequence: Syntheticpolynucleotide"
  source 1..366: mol_type = other DNA
gaggtgcaattggtggaaagcggaggcggcctcgtgaagcctggcggatctctgagactgagctgtgccgccagcggcttcaccttcagcaacgcctggatgagctgggtgcgccaggcccctggaaaaggactcgagtgggtgggacggatcaagagcaagaccgatggcggcaccaccgactatgccgcccctgtgaagggccggttcaccatcagcagggacgacagcaagaacaccctgtacctgcagatgaacagcctgaaaaccgaggacaccgccgtgtactactgcaccaccccctacgagtggtcttggtacgactactggggccagggcaccctcgtgaccgtgtcatctgctagc

SEQ ID NO: 211 - DNA, 366 bp, synthetic construct
  misc_feature 1..366: note = source = /note="Description of Artificial Sequence: Syntheticpolynucleotide"
  source 1..366: mol_type = other DNA
gaggtgcaattggtggaaagcggaggcggcctcgtgaagcctggcggatctctgagactgagctgtgccgccagcggcttcaccttcagcaacgcctggatgagctgggtgcgccaggcccctggaaaaggactcgagtgggtgggacggatcaagagcaagaccgatggcggcaccaccgactatgccgcccctgtgaagggccggttcaccatcagcagggacgacagcaagaacaccctgtacctgcagatgaacagcctgaaaaccgaggacaccgccgtgtactactgcaccaccccctgggagtactcttggtacgactactggggccagggcaccctcgtgaccgtgtcatctgctagc

SEQ ID NO: 212 - DNA, 366 bp, synthetic construct
  misc_feature 1..366: note = source = /note="Description of Artificial Sequence: Syntheticpolynucleotide"
  source 1..366: mol_type = other DNA
caggtgcaattggttcaatctggtgctgaagtaaaaaaaccgggcgcttccgttaaagtgagctgcaaagcatccggatacaccttcacttcctattacatgcactgggttcgtcaagccccgggccagggtctggaatggatgggcatcattaacccaagcggtggctctacctcctacgcgcagaaattccagggtcgcgtcacgatgacccgtgacactagcacctctaccgtttatatggagctgtccagcctgcgttctgaagatactgcagtgtactactgtgcacgcaactacactatcgttgtttctccgttcgactattggggtcaaggcaccctcgtaacggtttcttctgctagc

SEQ ID NO: 213 - DNA, 366 bp, synthetic construct
  misc_feature 1..366: note = source = /note="Description of Artificial Sequence: Syntheticpolynucleotide"
  source 1..366: mol_type = other DNA
caggtgcaattggttcaatctggtgctgaagtaaaaaaaccgggcgcttccgttaaagtgagctgcaaagcatccggatacaccttcacttcctattacatgcactgggttcgtcaagccccgggccagggtctggaatggatgggcatcattaacccaagcggtggctctacctcctacgcgcagaaattccagggtcgcgtcacgatgacccgtgacactagcacctctaccgtttatatggagctgtccagcctgcgttctgaagatactgcagtgtactactgtgcacgcaactacttcatcggttctgttgctatggactattggggtcaaggcaccctcgtaacggtttcttctgctagc

SEQ ID NO: 214 - DNA, 357 bp, synthetic construct
  misc_feature 1..357: note = source = /note="Description of Artificial Sequence: Syntheticpolynucleotide"
  source 1..357: mol_type = other DNA
caggtgcaattggttcaatctggtgctgaagtaaaaaaaccgggcgcttccgttaaagtgagctgcaaagcatccggatacaccttcacttcctattacatgcactgggttcgtcaagccccgggccagggtctggaatggatgggcatcattaacccaagcggtggctctacctcctacgcgcagaaattccagggtcgcgtcacgatgacccgtgacactagcacctctaccgtttatatggagctgtccagcctgcgttctgaagatactgcagtgtactactgtgcacgcggtctgacttactctatggactattggggtcaaggcaccctcgtaacggtttcttctgctagc

SEQ ID NO: 215 - DNA, 342 bp, synthetic construct
  misc_feature 1..342: note = source = /note="Description of Artificial Sequence: Syntheticpolynucleotide"
  source 1..342: mol_type = other DNA
gatattgttatgactcaatctccactgtctctgccggtgactccaggcgaaccggcgagcatttcttgccgttccagccagtctctgctgcactccaacggctacaactatctcgattggtacctgcaaaaaccgggtcagagccctcagctgctgatctacctgggctctaaccgcgcttccggtgtaccggaccgtttcagcggctctggatccggcaccgatttcacgttgaaaatcagccgtgttgaagcagaagacgtgggcgtttattactgtatgcaggcactgcagattccaaacacttttggtcaaggcaccaaggtcgaaattaaacgtacg

SEQ ID NO: 216 - DNA, 354 bp, synthetic construct
  misc_feature 1..354: note = source = /note="Description of Artificial Sequence: Syntheticpolynucleotide"
  source 1..354: mol_type = other DNA
gaggtgcaattgttggagtctgggggaggcttggtacagcctggggggtccctgagactctcctgtgcagcctccggattcacctttagcagttatgccatgagctgggtccgccaggctccagggaaggggctggagtgggtctcagctattagtggtagtggtggtagcacatactacgcagactccgtgaagggccggttcaccatctccagagacaattccaagaacacgctgtatctgcagatgaacagcctgagagccgaggacacggccgtatattactgtgcgaaatacgcttacgctctggactactggggccaaggaaccctggtcaccgtctcgagtgctagc

SEQ ID NO: 217 - DNA, 327 bp, synthetic construct
  misc_feature 1..327: note = source = /note="Description of Artificial Sequence: Syntheticpolynucleotide"
  source 1..327: mol_type = other DNA
gaaatcgtgttaacgcagtctccaggcaccctgtctttgtctccaggggaaagagccaccctctcttgcagggccagtcagagtgttagcagcagctacttagcctggtaccagcagaaacctggccaggctcccaggctcctcatctatggagcatccagcagggccactggcatcccagacaggttcagtggcagtggatccgggacagacttcactctcaccatcagcagactggagcctgaagattttgcagtgtattactgtcagcagcatggcagcagcagcacgttcggccaggggaccaaagtggaaatcaaacgtacg

SEQ ID NO: 218 - DNA, 366 bp, synthetic construct
  misc_feature 1..366: note = source = /note="Description of Artificial Sequence: Syntheticpolynucleotide"
  source 1..366: mol_type = other DNA
caggtgcaattggttcaatctggtgctgaagtaaaaaaaccgggcgcttccgttaaagtgagctgcaaagcatccggatacaccttcacttcctattacatgcactgggttcgtcaagccccgggccagggtctggaatggatgggcatcattaacccaagcggtggctctacctcctacgcgcagaaattccagggtcgcgtcacgatgacccgtgacactagcacctctaccgtttatatggagctgtccagcctgcgttctgaagatactgcagtgtactactgtgcacgcggtgacttctctgctggtcgtctgatggactattggggtcaaggcaccctcgtaacggtttcttctgctagc

SEQ ID NO: 219 - DNA, 345 bp, synthetic construct
  misc_feature 1..345: note = source = /note="Description of Artificial Sequence: Syntheticpolynucleotide"
  source 1..345: mol_type = other DNA
gatattgttatgactcaatctccactgtctctgccggtgactccaggcgaaccggcgagcatttcttgccgttccagccagtctctgctgcactccaacggctacaactatctcgattggtacctgcaaaaaccgggtcagagccctcagctgctgatctacctgggctctaaccgcgcttccggtgtaccggaccgtttcagcggctctggatccggcaccgatttcacgttgaaaatcagccgtgttgaagcagaagacgtgggcgtttattactgtatgcaggcactgcagaccccaccaattacctttggtcaaggcaccaaggtcgaaattaaacgtacg

SEQ ID NO: 220 - DNA, 357 bp, synthetic construct
  misc_feature 1..357: note = source = /note="Description of Artificial Sequence: Syntheticpolynucleotide"
  source 1..357: mol_type = other DNA
caggtgcaattggttcaatctggtgctgaagtaaaaaaaccgggcgcttccgttaaagtgagctgcaaagcatccggatacaccttcacttcctattacatgcactgggttcgtcaagccccgggccagggtctggaatggatgggcatcattaacccaagcggtggctctacctcctacgcgcagaaattccagggtcgcgtcacgatgacccgtgacactagcacctctaccgtttatatggagctgtccagcctgcgttctgaagatactgcagtgtactactgtgcacgcggtgactacaacgctttcgactattggggtcacggcaccctcgtaacggtttcttctgctagc

SEQ ID NO: 221 - DNA, 339 bp, synthetic construct
  misc_feature 1..339: note = source = /note="Description of Artificial Sequence: Syntheticpolynucleotide"
  source 1..339: mol_type = other DNA
gatattgttatgactcaatctccactgtctctgccggtgactccaggcgaaccggcgagcatttcttgccgttccagccagtctctgctgcactccaacggctacaactatctcgattggtacctgcaaaaaccgggtcagagccctcagctgctgatctacctgggctctaaccgcgcttccggtgtaccggaccgtttcagcggctctggatccggcaccgatttcacgttgaaaatcagccgtgttgaagcagaagacgtgggcgtttattactgtatgcaggcatggcatagcccaacttttggtcaaggcaccaaggtcgaaattaaacgtacg

SEQ ID NO: 222 - DNA, 357 bp, synthetic construct
  misc_feature 1..357: note = source = /note="Description of Artificial Sequence: Syntheticpolynucleotide"
  source 1..357: mol_type = other DNA
caggtgcaattggttcaatctggtgctgaagtaaaaaaaccgggcgcttccgttaaagtgagctgcaaagcatccggatacaccttcacttcctattacatgcactgggttcgtcaagccccgggccagggtctggaatggatgggcatcattaacccaagcggtggctctacctcctacgcgcagaaattccagggtcgcgtcacgatgacccgtgacactagcacctctaccgtttatatggagctgtccagcctgcgttctgaagatactgcagtgtactactgtgcacgcggtgctacttacactatggactattggggtcaaggcaccctcgtaacggtttcttctgctagc

SEQ ID NO: 223 - DNA, 342 bp, synthetic construct
  misc_feature 1..342: note = source = /note="Description of Artificial Sequence: Syntheticpolynucleotide"
  source 1..342: mol_type = other DNA
gatattgttatgactcaatctccactgtctctgccggtgactccaggcgaaccggcgagcatttcttgccgttccagccagtctctgctgcactccaacggctacaactatctcgattggtacctgcaaaaaccgggtcagagccctcagctgctgatctacctgggctctaaccgcgcttccggtgtaccggaccgtttcagcggctctggatccggcaccgatttcacgttgaaaatcagccgtgttgaagcagaagacgtgggcgtttattactgtatgcaggcactgcagaccccaattacttttggtcaaggcaccaaggtcgaaattaaacgtacg

SEQ ID NO: 224 - DNA, 1344 bp, synthetic construct
  misc_feature 1..1344: note = source = /note="Description of Artificial Sequence: Syntheticpolynucleotide"
  source 1..1344: mol_type = other DNA
caggtgcagctgcagcagtctggcgccgagctcgtgaaacctggcgcctccgtgaagatcagctgcaaggccagcggctacagcttcaccggctacttcatgaactgggtcaagcagagccacggcaagagcctggaatggatcggcagaatccacccctacgacggcgacaccttctacaaccagaacttcaaggacaaggccaccctgaccgtggacaagagcagcaacaccgcccacatggaactgctgagcctgaccagcgaggacttcgccgtgtactactgcaccagatacgacggcagccgggccatggattattggggccagggcaccaccgtgacagtgtccagcgctagcaccaagggcccctccgtgttccccctggcccccagcagcaagagcaccagcggcggcacagccgctctgggctgcctggtcaaggactacttccccgagcccgtgaccgtgtcctggaacagcggagccctgacctccggcgtgcacaccttccccgccgtgctgcagagttctggcctgtatagcctgagcagcgtggtcaccgtgccttctagcagcctgggcacccagacctacatctgcaacgtgaaccacaagcccagcaacaccaaggtggacaagaaggtggagcccaagagctgcgacaaaactcacacatgcccaccgtgcccagcacctgaagctgcagggggaccgtcagtcttcctcttccccccaaaacccaaggacaccctcatgatctcccggacccctgaggtcacatgcgtggtggtggacgtgagccacgaagaccctgaggtcaagttcaactggtacgtggacggcgtggaggtgcataatgccaagacaaagccgcgggaggagcagtacaacagcacgtaccgtgtggtcagcgtcctcaccgtcctgcaccaggactggctgaatggcaaggagtacaagtgcaaggtctccaacaaagccctcggcgcccccatcgagaaaaccatctccaaagccaaagggcagccccgagaaccacaggtgtgcaccctgcccccatcccgggatgagctgaccaagaaccaggtcagcctctcgtgcgcagtcaaaggcttctatcccagcgacatcgccgtggagtgggagagcaatgggcagccggagaacaactacaagaccacgcctcccgtgctggactccgacggctccttcttcctcgtgagcaagctcaccgtggacaagagcaggtggcagcaggggaacgtcttctcatgctccgtgatgcatgaggctctgcacaaccactacacgcagaagagcctctccctgtctccgggtaaa

SEQ ID NO: 225 - DNA, 2073 bp, synthetic construct
  misc_feature 1..2073: note = source = /note="Description of Artificial Sequence: Syntheticpolynucleotide"
  source 1..2073: mol_type = other DNA
caggtgcagctgcagcagtctggcgccgagctcgtgaaacctggcgcctccgtgaagatcagctgcaaggccagcggctacagcttcaccggctacttcatgaactgggtcaagcagagccacggcaagagcctggaatggatcggcagaatccacccctacgacggcgacaccttctacaaccagaacttcaaggacaaggccaccctgaccgtggacaagagcagcaacaccgcccacatggaactgctgagcctgaccagcgaggacttcgccgtgtactactgcaccagatacgacggcagccgggccatggattattggggccagggcaccaccgtgacagtgtccagcgctagcacaaagggccccagcgtgttccctctggcccctagcagcaagagcacatctggcggaacagccgccctgggctgcctcgtgaaggactactttcccgagcctgtgaccgtgtcctggaactctggcgccctgacaagcggcgtgcacacctttccagccgtgctgcagagcagcggcctgtactctctgagcagcgtggtcaccgtgcctagcagcagcctgggcacccagacctacatctgcaacgtgaaccacaagcccagcaacaccaaagtggacaagaaggtggagcccaagagctgtgatggcggaggagggtccggaggcggaggatccgaagtgcagctggtggaaagcggcggaggcctggtgcagcctaagggctctctgaagctgagctgtgccgccagcggcttcaccttcaacacctacgccatgaactgggtgcgccaggcccctggcaaaggcctggaatgggtggcccggatcagaagcaagtacaacaattacgccacctactacgccgacagcgtgaaggaccggttcaccatcagccgggacgacagccagagcatcctgtacctgcagatgaacaacctgaaaaccgaggacaccgccatgtactactgcgtgcggcacggcaacttcggcaacagctatgtgtcttggtttgcctactggggccagggcaccctcgtgacagtgtctgctgctagcgtggccgctccctccgtgtttatctttcccccatccgatgaacagctgaaaagcggcaccgcctccgtcgtgtgtctgctgaacaatttttaccctagggaagctaaagtgcagtggaaagtggataacgcactgcagtccggcaactcccaggaatctgtgacagaacaggactccaaggacagcacctactccctgtcctccaccctgacactgtctaaggctgattatgagaaacacaaagtctacgcctgcgaagtcacccatcagggcctgagctcgcccgtcacaaagagcttcaacaggggagagtgtgacaagacccacacctgtcccccttgtcctgcccctgaagctgctggcggcccttctgtgttcctgttccccccaaagcccaaggacaccctgatgatcagccggacccccgaagtgacctgcgtggtggtggatgtgtcccacgaggaccctgaagtgaagttcaattggtacgtggacggcgtggaagtgcacaacgccaagacaaagccgcgggaggagcagtacaacagcacgtaccgtgtggtcagcgtcctcaccgtcctgcaccaggactggctgaatggcaaggagtacaagtgcaaggtctccaacaaagccctcggcgcccccatcgagaaaaccatctccaaagccaaagggcagccccgagaaccacaggtgtacaccctgcccccatgccgggatgagctgaccaagaaccaggtcagcctgtggtgcctggtcaaaggcttctatcccagcgacatcgccgtggagtgggagagcaatgggcagccggagaacaactacaagaccacgcctcccgtgctggactccgacggctccttcttcctctacagcaagctcaccgtggacaagagcaggtggcagcaggggaacgtcttctcatgctccgtgatgcatgaggctctgcacaaccactacacgcagaagagcctctccctgtctccgggtaaa

SEQ ID NO: 226 - DNA, 654 bp, synthetic construct
  misc_feature 1..654: note = source = /note="Description of Artificial Sequence: Syntheticpolynucleotide"
  source 1..654: mol_type = other DNA
gacatcgagctgacccagagccctgcctctctggccgtgtctctgggacagagagccatcatcagctgcaaggccagccagagcgtgtcctttgccggcacctctctgatgcactggtatcaccagaagcccggccagcagcccaagctgctgatctacagagccagcaacctggaagccggcgtgcccacaagattttccggcagcggcagcaagaccgacttcaccctgaacatccaccccgtggaagaagaggacgccgccacctactactgccagcagagcagagagtacccctacaccttcggcggaggcaccaagctggaaatcaagcgtacggtggctgcaccatctgtcttcatcttcccgccatctgatgagcagttgaaatctggaactgcctctgttgtgtgcctgctgaataacttctatcccagagaggccaaagtacagtggaaggtggataacgccctccaatcgggtaactcccaggagagtgtcacagagcaggacagcaaggacagcacctacagcctcagcagcaccctgacgctgagcaaagcagactacgagaaacacaaagtctacgcctgcgaagtcacccatcagggcctgagctcgcccgtcacaaagagcttcaacaggggagagtgt

SEQ ID NO: 227 - protein, 209 aa, Homo sapiens
RIAWARTELLNVCMNAKHHKEKPGPEDKLHEQCRPWRKNACCSTNTSQEAHKDVSYLYRFNWNHCGEMAPACKRHFIQDTCLYECSPNLGPWIQQVDQSWRKERVLNVPLCKEDCEQWWEDCRTSYTCKSNWHKGWNWTSGFNKCAVGAACQPFHFYFPTPTVLCNEIWTHSYKVSNYSRGSGRCIQMWFDPAQGNPNEEVARFYAAAM

SEQ ID NO: 228 - protein, 214 aa, Homo sapiens
TMCSAQDRTDLLNVCMDAKHHKTKPGPEDKLHDQCSPWKKNACCTASTSQELHKDTSRLYNFNWDHCGKMEPACKRHFIQDTCLYECSPNLGPWIQQVNQSWRKERFLDVPLCKEDCQRWWEDCHTSHTCKSNWHRGWDWTSGVNKCPAGALCRTFESYFPTPAALCEGLWSHSYKVSNYSRGSGRCIQMWFDSAQGNPNEEVARFYAAAMHVN

SEQ ID NO: 229 - protein, 220 aa, Homo sapiens
SARARTDLLNVCMNAKHHKTQPSPEDELYGQCSPWKKNACCTASTSQELHKDTSRLYNFNWDHCGKMEPTCKRHFIQDSCLYECSPNLGPWIRQVNQSWRKERILNVPLCKEDCERWWEDCRTSYTCKSNWHKGWNWTSGINECPAGALCSTFESYFPTPAALCEGLWSHSFKVSNYSRGSGRCIQMWFDSAQGNPNEEVAKFYAAAMNAGAPSRGIIDS

SEQ ID NO: 230 - protein, 208 aa, Mus musculus
TRARTELLNVCMDAKHHKEKPGPEDNLHDQCSPWKTNSCCSTNTSQEAHKDISYLYRFNWNHCGTMTSECKRHFIQDTCLYECSPNLGPWIQQVDQSWRKERILDVPLCKEDCQQWWEDCQSSFTCKSNWHKGWNWSSGHNECPVGASCHPFTFYFPTSAALCEEIWSHSYKLSNYSRGSGRCIQMWFDPAQGNPNEEVARFYAEAMS

SEQ ID NO: 231 - protein, 213 aa, Macaca fascicularis
EAQTRTARARTELLNVCMNAKHHKEKPGPEDKLHEQCRPWKKNACCSTNTSQEAHKDVSYLYRFNWNHCGEMAPACKRHFIQDTCLYECSPNLGPWIQQVDQSWRKERVLNVPLCKEDCERWWEDCRTSYCKSNWHKGWNWTSGFNKCPVGAACQPFHFYFPTPTVLCNEIWTYSYKVSNYSRGSGRCIQMWFDPAQGNPNEEVARFYAAAMS

SEQ ID NO: 232 - protein, 9 aa, synthetic construct
  REGION 1..9: note = source = /note="Description of Artificial Sequence: Syntheticpeptide"
PWEYSWYDY

SEQ ID NO: 233 - protein, 11 aa, synthetic construct
  REGION 1..11: note = source = /note="Description of Artificial Sequence: Syntheticpeptide"
NYTIVVSPFDY

SEQ ID NO: 234 - protein, 11 aa, synthetic construct
  REGION 1..11: note = source = /note="Description of Artificial Sequence: Syntheticpeptide"
NYFIGSVAMDY

SEQ ID NO: 235 - protein, 8 aa, synthetic construct
  REGION 1..8: note = source = /note="Description of Artificial Sequence: Syntheticpeptide"
GLTYSMDY

SEQ ID NO: 236 - protein, 9 aa, synthetic construct
  REGION 1..9: note = source = /note="Description of Artificial Sequence: Syntheticpeptide"
MQALQIPNT

SEQ ID NO: 237 - protein, 7 aa, synthetic construct
  REGION 1..7: note = source = /note="Description of Artificial Sequence: Syntheticpeptide"
YAYALDY

SEQ ID NO: 238 - protein, 8 aa, synthetic construct
  REGION 1..8: note = source = /note="Description of Artificial Sequence: Syntheticpeptide"
QQHGSSST

SEQ ID NO: 239 - protein, 11 aa, synthetic construct
  REGION 1..11: note = source = /note="Description of Artificial Sequence: Syntheticpeptide"
GDFSAGRLMDY

SEQ ID NO: 240 - protein, 10 aa, synthetic construct
  REGION 1..10: note = source = /note="Description of Artificial Sequence: Syntheticpeptide"
MQALQTPPIT

SEQ ID NO: 241 - protein, 8 aa, synthetic construct
  REGION 1..8: note = source = /note="Description of Artificial Sequence: Syntheticpeptide"
GDYNAFDY

SEQ ID NO: 242 - protein, 8 aa, synthetic construct
  REGION 1..8: note = source = /note="Description of Artificial Sequence: Syntheticpeptide"
MQAWHSPT

SEQ ID NO: 243 - protein, 8 aa, synthetic construct
  REGION 1..8: note = source = /note="Description of Artificial Sequence: Syntheticpeptide"
GATYTMDY

SEQ ID NO: 244 - protein, 9 aa, synthetic construct
  REGION 1..9: note = source = /note="Description of Artificial Sequence: Syntheticpeptide"
MQALQTPIT

SEQ ID NO: 245 - protein, 227 aa, synthetic construct
  REGION 1..227: note = source = /note="Description of Artificial Sequence: Syntheticpolypeptide"
DKTHTCPPCPAPELLGGPSVFLFPPKPKDTLMISRTPEVTCVVVDVSHEDPEVKFNWYVDGVEVHNAKTKPREEQYNSTYRVVSVLTVLHQDWLNGKEYKCKVSNKALPAPIEKTISKAKGQPREPQVYTLPPSRDELTKNQVSLTCLVKGFYPSDIAVEWESNGQPENNYKTTPPVLDSDGSFFLYSKLTVDKSRWQQGNVFSCSVMHEALHNHYTQKSLSLSPGK

SEQ ID NO: 246 - DNA, 2076 bp, synthetic construct
  misc_feature 1..2076: note = source = /note="Description of Artificial Sequence: Syntheticpolynucleotide"
  source 1..2076: mol_type = other DNA
caggtgcaattggttcaatctggtgctgaagtaaaaaaaccgggcgcttccgttaaagtgagctgcaaagcatccggatacaccttcacttcctattacatgcactgggttcgtcaagccccgggccagggtctggaatggatgggcatcattaacccaagcggtggctctacctcctacgcgcagaaattccagggtcgcgtcacgatgacccatgacactagcacctctaccgtttatatggagctgtccagcctgcgttctgaagatactgcagtgtactactgtgcacgctctttcttcactggtttccatctggactattggggtcaaggcaccctcgtaacggtttcttctgctagcacaaagggccccagcgtgttccctctggcccctagcagcaagagcacatctggcggaacagccgccctgggctgcctcgtgaaggactactttcccgagcctgtgaccgtgtcctggaactctggcgccctgacaagcggcgtgcacacctttccagccgtgctgcagagcagcggcctgtactctctgagcagcgtggtcaccgtgcctagcagcagcctgggcacccagacctacatctgcaacgtgaaccacaagcccagcaacaccaaagtggacaagaaggtggagcccaagagctgtgatggcggaggagggtccggaggcggaggatccgaggtgcagctgctggaatctggcggcggactggtgcagcctggcggatctctgagactgagctgtgccgccagcggcttcaccttcagcacctacgccatgaactgggtgcgccaggcccctggcaaaggcctggaatgggtgtcccggatcagaagcaagtacaacaactacgccacctactacgccgacagcgtgaagggccggttcaccatcagccgggacgacagcaagaacaccctgtacctgcagatgaacagcctgcgggccgaggacaccgccgtgtactattgtgtgcggcacggcaacttcggcaacagctatgtgtcttggtttgcctactggggccagggcaccctcgtgaccgtgtcaagcgctagtgtggccgctccctccgtgtttatctttcccccatccgatgaacagctgaaaagcggcaccgcctccgtcgtgtgtctgctgaacaatttttaccctagggaagctaaagtgcagtggaaagtggataacgcactgcagtccggcaactcccaggaatctgtgacagaacaggactccaaggacagcacctactccctgtcctccaccctgacactgtctaaggctgattatgagaaacacaaagtctacgcctgcgaagtcacccatcagggcctgagctcgcccgtcacaaagagcttcaacaggggagagtgtgacaagacccacacctgtcccccttgtcctgcccctgaagctgctggcggcccttctgtgttcctgttccccccaaagcccaaggacaccctgatgatcagccggacccccgaagtgacctgcgtggtggtggatgtgtcccacgaggaccctgaagtgaagttcaattggtacgtggacggcgtggaagtgcacaacgccaagacaaagccgcgggaggagcagtacaacagcacgtaccgtgtggtcagcgtcctcaccgtcctgcaccaggactggctgaatggcaaggagtacaagtgcaaggtctccaacaaagccctcggcgcccccatcgagaaaaccatctccaaagccaaagggcagccccgagaaccacaggtgtacaccctgcccccatgccgggatgagctgaccaagaaccaggtcagcctgtggtgcctggtcaaaggcttctatcccagcgacatcgccgtggagtgggagagcaatgggcagccggagaacaactacaagaccacgcctcccgtgctggactccgacggctccttcttcctctacagcaagctcaccgtggacaagagcaggtggcagcaggggaacgtcttctcatgctccgtgatgcatgaggctctgcacaaccactacacgcagaagagcctctccctgtctccgggtaaa

SEQ ID NO: 247 - DNA, 1347 bp, synthetic construct
  misc_feature 1..1347: note = source = /note="Description of Artificial Sequence: Syntheticpolynucleotide"
  source 1..1347: mol_type = other DNA
caggtgcaattggttcaatctggtgctgaagtaaaaaaaccgggcgcttccgttaaagtgagctgcaaagcatccggatacaccttcacttcctattacatgcactgggttcgtcaagccccgggccagggtctggaatggatgggcatcattaacccaagcggtggctctacctcctacgcgcagaaattccagggtcgcgtcacgatgacccatgacactagcacctctaccgtttatatggagctgtccagcctgcgttctgaagatactgcagtgtactactgtgcacgctctttcttcactggtttccatctggactattggggtcaaggcaccctcgtaacggtttcttctgctagcaccaagggcccctccgtgttccccctggcccccagcagcaagagcaccagcggcggcacagccgctctgggctgcctggtcaaggactacttccccgagcccgtgaccgtgtcctggaacagcggagccctgacctccggcgtgcacaccttccccgccgtgctgcagagttctggcctgtatagcctgagcagcgtggtcaccgtgccttctagcagcctgggcacccagacctacatctgcaacgtgaaccacaagcccagcaacaccaaggtggacaagaaggtggagcccaagagctgcgacaaaactcacacatgcccaccgtgcccagcacctgaagctgcagggggaccgtcagtcttcctcttccccccaaaacccaaggacaccctcatgatctcccggacccctgaggtcacatgcgtggtggtggacgtgagccacgaagaccctgaggtcaagttcaactggtacgtggacggcgtggaggtgcataatgccaagacaaagccgcgggaggagcagtacaacagcacgtaccgtgtggtcagcgtcctcaccgtcctgcaccaggactggctgaatggcaaggagtacaagtgcaaggtctccaacaaagccctcggcgcccccatcgagaaaaccatctccaaagccaaagggcagccccgagaaccacaggtgtgcaccctgcccccatcccgggatgagctgaccaagaaccaggtcagcctctcgtgcgcagtcaaaggcttctatcccagcgacatcgccgtggagtgggagagcaatgggcagccggagaacaactacaagaccacgcctcccgtgctggactccgacggctccttcttcctcgtgagcaagctcaccgtggacaagagcaggtggcagcaggggaacgtcttctcatgctccgtgatgcatgaggctctgcacaaccactacacgcagaagagcctctccctgtctccgggtaaa

SEQ ID NO: 248 - protein, 120 aa, synthetic construct
  REGION 1..120: note = source = /note="Description of Artificial Sequence: Syntheticpolypeptide"
EVQLVESGGGLVKPGGSLRLSCAASGFTFSNAWMSWVRQAPGKGLEWVGRIKSKTEGGTTDYAAPVKGRFTISRDDSKNTLYLQMNSLKTEDTAVYYCTTPWEWSWYDYWGQGTLVTVSS

SEQ ID NO: 249 - protein, 120 aa, synthetic construct
  REGION 1..120: note = source = /note="Description of Artificial Sequence: Syntheticpolypeptide"
EVQLVESGGGLVKPGGSLRLSCAASGFTFSNAWMSWVRQAPGKGLEWVGRIKSKTQGGTTDYAAPVKGRFTISRDDSKNTLYLQMNSLKTEDTAVYYCTTPWEWSWYDYWGQGTLVTVSS

SEQ ID NO: 250 - protein, 125 aa, synthetic construct
  REGION 1..125: note = source = /note="Description of Artificial Sequence: Syntheticpolypeptide"
EVQLLESGGGLVQPGGSLRLSCAASGFTFSTYAMNWVRQAPGKGLEWVSRIRSKYNNYATYYADSVKGRFTISRDDSKNTLYLQMNSLRAEDTAVYYCVRHGNFGASYVSWFAYWGQGTLVTVSS

SEQ ID NO: 251 - protein, 125 aa, synthetic construct
  REGION 1..125: note = source = /note="Description of Artificial Sequence: Syntheticpolypeptide"
EVQLLESGGGLVQPGGSLRLSCAASGFTFSTYAMNWVRQAPGKGLEWVSRIRSKYNNYATYYADSVKGRFTISRDDSKNTLYLQMNSLRAEDTAVYYCVRHGNFGNAYVSWFAYWGQGTLVTVSS

SEQ ID NO: 252 - protein, 689 aa, synthetic construct; identical to SEQ ID NO: 99
  REGION 1..689: note = source = /note="Description of Artificial Sequence: Syntheticpolypeptide"

SEQ ID NO: 253 - protein, 450 aa, synthetic construct; identical to SEQ ID NO: 90
  REGION 1..450: note = source = /note="Description of Artificial Sequence: Syntheticpolypeptide"

SEQ ID NO: 254 - protein, 215 aa, synthetic construct; identical to SEQ ID NO: 35
  REGION 1..215: note = source = /note="Description of Artificial Sequence: Syntheticpolypeptide"

SEQ ID NO: 255 - protein, 689 aa, synthetic construct; identical to SEQ ID NO: 100
  REGION 1..689: note = source = /note="Description of Artificial Sequence: Syntheticpolypeptide"

SEQ ID NO: 256 - protein, 690 aa, synthetic construct
  REGION 1..690: note = source = /note="Description of Artificial Sequence: Syntheticpolypeptide"
QVQLVQSGAEVKKPGASVKVSCKASGYTFTSYYMHWVRQAPGQGLEWMGIINPSGGPTSYAQKFQGRVTMTRDTSTSTVYMELSSLRSEDTAVYYCARGDFAWLDYWGQGTLVTVSSASTKGPSVFPLAPSSKSTSGGTAALGCLVKDYFPEPVTVSWNSGALTSGVHTFPAVLQSSGLYSLSSVVTVPSSSLGTQTYICNVNHKPSNTKVDKKVEPKSCDGGGGSGGGGSEVQLLESGGGLVQPGGSLRLSCAASGFTFSTYAMNWVRQAPGKGLEWVSRIRSKYNNYATYYADSVKGRFTISRDDSKNTLYLQMNSLRAEDTAVYYCVRHGNFGASYVSWFAYWGQGTLVTVSSASVAAPSVFIFPPSDEQLKSGTASVVCLLNNFYPREAKVQWKVDNALQSGNSQESVTEQDSKDSTYSLSSTLTLSKADYEKHKVYACEVTHQGLSSPVTKSFNRGECDKTHTCPPCPAPEAAGGPSVFLFPPKPKDTLMISRTPEVTCVVVDVSHEDPEVKFNWYVDGVEVHNAKTKPREEQYNSTYRVVSVLTVLHQDWLNGKEYKCKVSNKALGAPIEKTISKAKGQPREPQVYTLPPCRDELTKNQVSLWCLVKGFYPSDIAVEWESNGQPENNYKTTPPVLDSDGSFFLYSKLTVDKSRWQQGNVFSCSVMHEALHNHYTQKSLSLSPGK

SEQ ID NO: 257 - protein, 447 aa, synthetic construct; identical to SEQ ID NO: 95
  REGION 1..447: note = source = /note="Description of Artificial Sequence: Syntheticpolypeptide"

SEQ ID NO: 258 - protein, 219 aa, synthetic construct
  REGION 1..219: note = source = /note="Description of Artificial Sequence: Syntheticpolypeptide"
DIVMTQSPLSLPVTPGEPASISCRSSQSLLHSNGYNYLDWYLQKPGQSPQLLIYLGSNRASGVPDRFSGSGSGTDFTLKISRVEAEDVGVYYCMQASIMQRTFGQGTKVEIKRTVAAPSVFIFPPSDEQLKSGTASVVCLLNNFYPREAKVQWKVDNALQSGNSQESVTEQDSKDSTYSLSSTLTLSKADYEKHKVYACEVTHQGLSSPVTKSFNRGEC

SEQ ID NO: 259 - protein, 214 aa, synthetic construct; identical to SEQ ID NO: 86
  REGION 1..214: note = source = /note="Description of Artificial Sequence: Syntheticpolypeptide"

SEQ ID NO: 260 - protein, 690 aa, synthetic construct
  REGION 1..690: note = source = /note="Description of Artificial Sequence: Syntheticpolypeptide"
QVQLVQSGAEVKKPGASVKVSCKASGYTFTSYYMHWVRQAPGQGLEWMGIINPSGGPTSYAQKFQGRVTMTRDTSTSTVYMELSSLRSEDTAVYYCARGDFAWLDYWGQGTLVTVSSASTKGPSVFPLAPSSKSTSGGTAALGCLVKDYFPEPVTVSWNSGALTSGVHTFPAVLQSSGLYSLSSVVTVPSSSLGTQTYICNVNHKPSNTKVDKKVEPKSCDGGGGSGGGGSEVQLLESGGGLVQPGGSLRLSCAASGFTFSTYAMNWVRQAPGKGLEWVSRIRSKYNNYATYYADSVKGRFTISRDDSKNTLYLQMNSLRAEDTAVYYCVRHGNFGNAYVSWFAYWGQGTLVTVSSASVAAPSVFIFPPSDEQLKSGTASVVCLLNNFYPREAKVQWKVDNALQSGNSQESVTEQDSKDSTYSLSSTLTLSKADYEKHKVYACEVTHQGLSSPVTKSFNRGECDKTHTCPPCPAPEAAGGPSVFLFPPKPKDTLMISRTPEVTCVVVDVSHEDPEVKFNWYVDGVEVHNAKTKPREEQYNSTYRVVSVLTVLHQDWLNGKEYKCKVSNKALGAPIEKTISKAKGQPREPQVYTLPPCRDELTKNQVSLWCLVKGFYPSDIAVEWESNGQPENNYKTTPPVLDSDGSFFLYSKLTVDKSRWQQGNVFSCSVMHEALHNHYTQKSLSLSPGK

SEQ ID NO: 261 - DNA, 360 bp, synthetic construct
  misc_feature 1..360: note = source = /note="Description of Artificial Sequence: Syntheticpolynucleotide"
  source 1..360: mol_type = other DNA
gaggtgcaattggttgaatctggtggtggtctggtaaaaccgggcggttccctgcgtctgagctgcgcggcttccggattcaccttctccaacgcgtggatgagctgggttcgccaggccccgggcaaaggcctcgagtgggttggtcgtatcaagtctaaaactgagggtggcaccacggattacgcggctccagttaaaggtcgttttaccatttcccgcgacgatagcaaaaacactctgtatctgcagatgaactctctgaaaactgaagacaccgcagtctactactgtactaccccgtgggaatggtcttggtacgattattggggccagggcacgctggttacggtgtcttcc

SEQ ID NO: 262 - DNA, 360 bp, synthetic construct
  misc_feature 1..360: note = source = /note="Description of Artificial Sequence: Syntheticpolynucleotide"
  source 1..360: mol_type = other DNA
gaggtgcaattggttgaatctggtggtggtctggtaaaaccgggcggttccctgcgtctgagctgcgcggcttccggattcaccttctccaacgcgtggatgagctgggttcgccaggccccgggcaaaggcctcgagtgggttggtcgtatcaagtctaaaactcagggtggcaccacggattacgcggctccagttaaaggtcgttttaccatttcccgcgacgatagcaaaaacactctgtatctgcagatgaactctctgaaaactgaagacaccgcagtctactactgtactaccccgtgggaatggtcttggtacgattattggggccagggcacgctggttacggtgtcttcc

SEQ ID NO: 263 - DNA, 375 bp, synthetic construct
  misc_feature 1..375: note = source = /note="Description of Artificial Sequence: Syntheticpolynucleotide"
  source 1..375: mol_type = other DNA
gaggtgcagctgctggaatctggcggcggactggtgcagcctggcggatctctgagactgagctgtgccgccagcggcttcaccttcagcacctacgccatgaactgggtgcgccaggcccctggcaaaggcctggaatgggtgtcccggatcagaagcaagtacaacaactacgccacctactacgccgacagcgtgaagggccggttcaccatcagccgggacgacagcaagaacaccctgtacctgcagatgaacagcctgcgggccgaggacaccgccgtgtactattgtgtgcggcacggcaacttcggcgccagctatgtgtcttggtttgcctactggggccagggcaccctcgtgaccgtgtcaagc

SEQ ID NO: 264 - DNA, 375 bp, synthetic construct
  misc_feature 1..375: note = source = /note="Description of Artificial Sequence: Syntheticpolynucleotide"
  source 1..375: mol_type = other DNA
gaggtgcagctgctggaatctggcggcggactggtgcagcctggcggatctctgagactgagctgtgccgccagcggcttcaccttcagcacctacgccatgaactgggtgcgccaggcccctggcaaaggcctggaatgggtgtcccggatcagaagcaagtacaacaactacgccacctactacgccgacagcgtgaagggccggttcaccatcagccgggacgacagcaagaacaccctgtacctgcagatgaacagcctgcgggccgaggacaccgccgtgtactattgtgtgcggcacggcaacttcggcaacgcctatgtgtcttggtttgcctactggggccagggcaccctcgtgaccgtgtcaagc

SEQ ID NO: 265 - DNA, 2067 bp, synthetic construct; identical to SEQ ID NO: 200
  misc_feature 1..2067: note = source = /note="Description of Artificial Sequence: Syntheticpolynucleotide"
  source 1..2067: mol_type = other DNA

SEQ ID NO: 266 - DNA, 1350 bp, synthetic construct; identical to SEQ ID NO: 190
  misc_feature 1..1350: note = source = /note="Description of Artificial Sequence: Syntheticpolynucleotide"
  source 1..1350: mol_type = other DNA

SEQ ID NO: 267 - DNA, 645 bp, synthetic construct; identical to SEQ ID NO: 191
  misc_feature 1..645: note = source = /note="Description of Artificial Sequence: Syntheticpolynucleotide"
  source 1..645: mol_type = other DNA

SEQ ID NO: 268 - DNA, 2067 bp, synthetic construct; identical to SEQ ID NO: 201
  misc_feature 1..2067: note = source = /note="Description of Artificial Sequence: Syntheticpolynucleotide"
  source 1..2067: mol_type = other DNA

SEQ ID NO: 269 - DNA, 2070 bp, synthetic construct
  misc_feature 1..2070: note = source = /note="Description of Artificial Sequence: Syntheticpolynucleotide"
  source 1..2070: mol_type = other DNA
caggtgcaattggttcaatctggtgctgaagtaaaaaaaccgggcgcttccgttaaagtgagctgcaaagcatccggatacaccttcacttcctattacatgcactgggttcgtcaagccccgggccagggtctggaatggatgggcatcattaacccaagcggtggccctacctcctacgcgcagaaattccagggtcgcgtcacgatgacccgtgacactagcacctctaccgtttatatggagctgtccagcctgcgttctgaagatactgcagtgtactactgtgcacgcggtgacttcgcttggctggactattggggtcaaggcaccctcgtaacggtttcttctgctagcacaaagggccccagcgtgttccctctggcccctagcagcaagagcacatctggcggaacagccgccctgggctgcctcgtgaaggactactttcccgagcctgtgaccgtgtcctggaactctggcgccctgacaagcggcgtgcacacctttccagccgtgctgcagagcagcggcctgtactctctgagcagcgtggtcaccgtgcctagcagcagcctgggcacccagacctacatctgcaacgtgaaccacaagcccagcaacaccaaagtggacaagaaggtggagcccaagagctgtgatggcggaggagggtccggaggcggaggatccgaggtgcagctgctggaatctggcggcggactggtgcagcctggcggatctctgagactgagctgtgccgccagcggcttcaccttcagcacctacgccatgaactgggtgcgccaggcccctggcaaaggcctggaatgggtgtcccggatcagaagcaagtacaacaactacgccacctactacgccgacagcgtgaagggccggttcaccatcagccgggacgacagcaagaacaccctgtacctgcagatgaacagcctgcgggccgaggacaccgccgtgtactattgtgtgcggcacggcaacttcggcgccagctatgtgtcttggtttgcctactggggccagggcaccctcgtgaccgtgtcaagcgctagtgtggccgctccctccgtgtttatctttcccccatccgatgaacagctgaaaagcggcaccgcctccgtcgtgtgtctgctgaacaatttttaccctagggaagctaaagtgcagtggaaagtggataacgcactgcagtccggcaactcccaggaatctgtgacagaacaggactccaaggacagcacctactccctgtcctccaccctgacactgtctaaggctgattatgagaaacacaaagtctacgcctgcgaagtcacccatcagggcctgagctcgcccgtcacaaagagcttcaacaggggagagtgtgacaagacccacacctgtcccccttgtcctgcccctgaagctgctggcggcccttctgtgttcctgttccccccaaagcccaaggacaccctgatgatcagccggacccccgaagtgacctgcgtggtggtggatgtgtcccacgaggaccctgaagtgaagttcaattggtacgtggacggcgtggaagtgcacaacgccaagacaaagccgcgggaggagcagtacaacagcacgtaccgtgtggtcagcgtcctcaccgtcctgcaccaggactggctgaatggcaaggagtacaagtgcaaggtctccaacaaagccctcggcgcccccatcgagaaaaccatctccaaagccaaagggcagccccgagaaccacaggtgtacaccctgcccccatgccgggatgagctgaccaagaaccaggtcagcctgtggtgcctggtcaaaggcttctatcccagcgacatcgccgtggagtgggagagcaatgggcagccggagaacaactacaagaccacgcctcccgtgctggactccgacggctccttcttcctctacagcaagctcaccgtggacaagagcaggtggcagcaggggaacgtcttctcatgctccgtgatgcatgaggctctgcacaaccactacacgcagaagagcctctccctgtctccgggtaaa

SEQ ID NO: 270 - DNA, 1341 bp, synthetic construct; identical to SEQ ID NO: 196
  misc_feature 1..1341: note = source = /note="Description of Artificial Sequence: Syntheticpolynucleotide"
  source 1..1341: mol_type = other DNA

SEQ ID NO: 271 - DNA, 657 bp, synthetic construct
  misc_feature 1..657: note = source = /note="Description of Artificial Sequence: Syntheticpolynucleotide"
  source 1..657: mol_type = other DNA
gatattgttatgactcaatctccactgtctctgccggtgactccaggcgaaccggcgagcatttcttgccgttccagccagtctctgctgcactccaacggctacaactatctcgattggtacctgcaaaaaccgggtcagagccctcagctgctgatctacctgggctctaaccgcgcttccggtgtaccggaccgtttcagcggctctggatccggcaccgatttcacgttgaaaatcagccgtgttgaagcagaagacgtgggcgtttattactgtatgcaggcaagcattatgcagcggacttttggtcaaggcaccaaggtcgaaattaaacgtacggtggctgcaccatctgtcttcatcttcccgccatctgatgagcagttgaaatctggaactgcctctgttgtgtgcctgctgaataacttctatcccagagaggccaaagtacagtggaaggtggataacgccctccaatcgggtaactcccaggagagtgtcacagagcaggacagcaaggacagcacctacagcctcagcagcaccctgacgctgagcaaagcagactacgagaaacacaaagtctacgcctgcgaagtcacccatcagggcctgagctcgcccgtcacaaagagcttcaacaggggagagtgt

SEQ ID NO: 272 - DNA, 642 bp, synthetic construct; identical to SEQ ID NO: 198
  misc_feature 1..642: note = source = /note="Description of Artificial Sequence: Syntheticpolynucleotide"
  source 1..642: mol_type = other DNA

SEQ ID NO: 273 - DNA, 2070 bp, synthetic construct
  misc_feature 1..2070: note = source = /note="Description of Artificial Sequence: Syntheticpolynucleotide"
  source 1..2070: mol_type = other DNA
caggtgcaattggttcaatctggtgctgaagtaaaaaaaccgggcgcttccgttaaagtgagctgcaaagcatccggatacaccttcacttcctattacatgcactgggttcgtcaagccccgggccagggtctggaatggatgggcatcattaacccaagcggtggccctacctcctacgcgcagaaattccagggtcgcgtcacgatgacccgtgacactagcacctctaccgtttatatggagctgtccagcctgcgttctgaagatactgcagtgtactactgtgcacgcggtgacttcgcttggctggactattggggtcaaggcaccctcgtaacggtttcttctgctagcacaaagggccccagcgtgttccctctggcccctagcagcaagagcacatctggcggaacagccgccctgggctgcctcgtgaaggactactttcccgagcctgtgaccgtgtcctggaactctggcgccctgacaagcggcgtgcacacctttccagccgtgctgcagagcagcggcctgtactctctgagcagcgtggtcaccgtgcctagcagcagcctgggcacccagacctacatctgcaacgtgaaccacaagcccagcaacaccaaagtggacaagaaggtggagcccaagagctgtgatggcggaggagggtccggaggcggaggatccgaggtgcagctgctggaatctggcggcggactggtgcagcctggcggatctctgagactgagctgtgccgccagcggcttcaccttcagcacctacgccatgaactgggtgcgccaggcccctggcaaaggcctggaatgggtgtcccggatcagaagcaagtacaacaactacgccacctactacgccgacagcgtgaagggccggttcaccatcagccgggacgacagcaagaacaccctgtacctgcagatgaacagcctgcgggccgaggacaccgccgtgtactattgtgtgcggcacggcaacttcggcaacgcctatgtgtcttggtttgcctactggggccagggcaccctcgtgaccgtgtcaagcgctagtgtggccgctccctccgtgtttatctttcccccatccgatgaacagctgaaaagcggcaccgcctccgtcgtgtgtctgctgaacaatttttaccctagggaagctaaagtgcagtggaaagtggataacgcactgcagtccggcaactcccaggaatctgtgacagaacaggactccaaggacagcacctactccctgtcctccaccctgacactgtctaaggctgattatgagaaacacaaagtctacgcctgcgaagtcacccatcagggcctgagctcgcccgtcacaaagagcttcaacaggggagagtgtgacaagacccacacctgtcccccttgtcctgcccctgaagctgctggcggcccttctgtgttcctgttccccccaaagcccaaggacaccctgatgatcagccggacccccgaagtgacctgcgtggtggtggatgtgtcccacgaggaccctgaagtgaagttcaattggtacgtggacggcgtggaagtgcacaacgccaagacaaagccgcgggaggagcagtacaacagcacgtaccgtgtggtcagcgtcctcaccgtcctgcaccaggactggctgaatggcaaggagtacaagtgcaaggtctccaacaaagccctcggcgcccccatcgagaaaaccatctccaaagccaaagggcagccccgagaaccacaggtgtacaccctgcccccatgccgggatgagctgaccaagaaccaggtcagcctgtggtgcctggtcaaaggcttctatcccagcgacatcgccgtggagtgggagagcaatgggcagccggagaacaactacaagaccacgcctcccgtgctggactccgacggctccttcttcctctacagcaagctcaccgtggacaagagcaggtggcagcaggggaacgtcttctcatgctccgtgatgcatgaggctctgcacaaccactacacgcagaagagcctctccctgtctccgggtaaa

SEQ ID NO: 274 - protein, 440 aa, synthetic construct
  REGION 1..440: note = source = /note="Description of Artificial Sequence: Syntheticpolypeptide"
QVQLVESGGGVVQPGRSLRLDCKASGITFSNSGMHWVRQAPGKGLEWVAVIWYDGSKRYYADSVKGRFTISRDNSKNTLFLQMNSLRAEDTAVYYCATNDDYWGQGTLVTVSSASTKGPSVFPLAPCSRSTSESTAALGCLVKDYFPEPVTVSWNSGALTSGVHTFPAVLQSSGLYSLSSVVTVPSSSLGTKTYTCNVDHKPSNTKVDKRVESKYGPPCPPCPAPEFLGGPSVFLFPPKPKDTLMISRTPEVTCVVVDVSQEDPEVQFNWYVDGVEVHNAKTKPREEQFNSTYRVVSVLTVLHQDWLNGKEYKCKVSNKGLPSSIEKTISKAKGQPREPQVYTLPPSQEEMTKNQVSLTCLVKGFYPSDIAVEWESNGQPENNYKTTPPVLDSDGSFFLYSRLTVDKSRWQEGNVFSCSVMHEALHNHYTQKSLSLSLGK

SEQ ID NO: 275 - protein, 214 aa, synthetic construct
  REGION 1..214: note = source = /note="Description of Artificial Sequence: Syntheticpolypeptide"
EIVLTQSPATLSLSPGERATLSCRASQSVSSYLAWYQQKPGQAPRLLIYDASNRATGIPARFSGSGSGTDFTLTISSLEPEDFAVYYCQQSSNWPRTFGQGTKVEIKRTVAAPSVFIFPPSDEQLKSGTASVVCLLNNFYPREAKVQWKVDNALQSGNSQESVTEQDSKDSTYSLSSTLTLSKADYEKHKVYACEVTHQGLSSPVTKSFNRGEC

SEQ ID NO: 276 - protein, 447 aa, synthetic construct
  REGION 1..447: note = source = /note="Description of Artificial Sequence: Syntheticpolypeptide"
QVQLVQSGVEVKKPGASVKVSCKASGYTFTNYYMYWVRQAPGQGLEWMGGINPSNGGTNFNEKFKNRVTLTTDSSTTTAYMELKSLQFDDTAVYYCARRDYRFDMGFDYWGQGTTVTVSSASTKGPSVFPLAPCSRSTSESTAALGCLVKDYFPEPVTVSWNSGALTSGVHTFPAVLQSSGLYSLSSVVTVPSSSLGTKTYTCNVDHKPSNTKVDKRVESKYGPPCPPCPAPEFLGGPSVFLFPPKPKDTLMISRTPEVTCVVVDVSQEDPEVQFNWYVDGVEVHNAKTKPREEQFNSTYRVVSVLTVLHQDWLNGKEYKCKVSNKGLPSSIEKTISKAKGQPREPQVYTLPPSQEEMTKNQVSLTCLVKGFYPSDIAVEWESNGQPENNYKTTPPVLDSDGSFFLYSRLTVDKSRWQEGNVFSCSVMHEALHNHYTQKSLSLSLGK

SEQ ID NO: 277 - protein, 218 aa, synthetic construct
  REGION 1..218: note = source = /note="Description of Artificial Sequence: Syntheticpolypeptide"
EIVLTQSPATLSLSPGERATLSCRASKGVSTSGYSYLHWYQQKPGQAPRLLIYLASYLESGVPARFSGSGSGTDFTLTISSLEPEDFAVYYCQHSRDLPLTFGGGTKVEIKRTVAAPSVFIFPPSDEQLKSGTASVVCLLNNFYPREAKVQWKVDNALQSGNSQESVTEQDSKDSTYSLSSTLTLSKADYEKHKVYACEVTHQGLSSPVTKSFNRGEC

SEQ ID NO: 278 - protein, 447 aa, synthetic construct
  REGION 1..447: note = source = /note="Description of Artificial Sequence: Syntheticpolypeptide"
EVQLVESGGGLVQPGGSLRLSCAASGFTFSDSWIHWVRQAPGKGLEWVAWISPYGGSTYYADSVKGRFTISADTSKNTAYLQMNSLRAEDTAVYYCARRHWPGGFDYWGQGTLVTVSSASTKGPSVFPLAPSSKSTSGGTAALGCLVKDYFPEPVTVSWNSGALTSGVHTFPAVLQSSGLYSLSSVVTVPSSSLGTQTYICNVNHKPSNTKVDKKVEPKSCDKTHTCPPCPAPELLGGPSVFLFPPKPKDTLMISRTPEVTCVVVDVSHEDPEVKFNWYVDGVEVHNAKTKPREEQYASTYRVVSVLTVLHQDWLNGKEYKCKVSNKALPAPIEKTISKAKGQPREPQVYTLPPSREEMTKNQVSLTCLVKGFYPSDIAVEWESNGQPENNYKTTPPVLDSDGSFFLYSKLTVDKSRWQQGNVFSCSVMHEALHNHYTQKSLSLSPG

SEQ ID NO: 279 - protein, 214 aa, synthetic construct
  REGION 1..214: note = source = /note="Description of Artificial Sequence: Syntheticpolypeptide"
DIQMTQSPSSLSASVGDRVTITCRASQDVSTAVAWYQQKPGKAPKLLIYSASFLYSGVPSRFSGSGSGTDFTLTISSLQPEDFATYYCQQYLYHPATFGQGTKVEIKRTVAAPSVFIFPPSDEQLKSGTASVVCLLNNFYPREAKVQWKVDNALQSGNSQESVTEQDSKDSTYSLSSTLTLSKADYEKHKVYACEVTHQGLSSPVTKSFNRGEC

SEQ ID NO: 280 - protein, 118 aa, synthetic construct [sequence omitted]

SEQ ID NO: 281 - protein, 122 aa, synthetic construct
  REGION 1..122: note = source = /note="Description of Artificial Sequence: Syntheticpolypeptide"
EVQLVESGGGLVQPGGSLRLSCAASGFTFSDSWIHWVRQAPGKGLEWVAWISPYGGSTYYADSVKGRFTISADTSKNTAYLQMNSLRAEDTAVYYCARRHWPGGFDYWGQGTLVTVSSASTK

SEQ ID NO: 282 - protein, 108 aa, synthetic construct
  REGION 1..108: note = source = /note="Description of Artificial Sequence: Syntheticpolypeptide"
DIQMTQSPSSLSASVGDRVTITCRASQDVSTAVAWYQQKPGKAPKLLIYSASFLYSGVPSRFSGSGSGTDFTLTISSLQPEDFATYYCQQYLYHPATFGQGTKVEIKR

SEQ ID NO: 283 - protein, 10 aa, synthetic construct
  VARIANT 6: note = /replace="Gly"
  REGION 1..10: note = MISC_FEATURE - /note="Variant residues given in the sequence have nopreference with respect to those in the annotationsfor variant positions"
  REGION 1..10: note = source = /note="Description of Artificial Sequence: Syntheticpeptide"
GFTFSDSWIH

SEQ ID NO: 284 - protein, 18 aa, synthetic construct
  VARIANT 4: note = /replace="Leu"
  VARIANT 10: note = /replace="Ser"
  REGION 1..18: note = MISC_FEATURE - /note="Variant residues given in the sequence have nopreference with respect to those in the annotationsfor variant positions"
  REGION 1..18: note = source = /note="Description of Artificial Sequence: Syntheticpeptide"
AWISPYGGSTYYADSVKG

SEQ ID NO: 285 - protein, 9 aa, synthetic construct
  REGION 1..9: note = source = /note="Description of Artificial Sequence: Syntheticpeptide"
RHWPGGFDY

SEQ ID NO: 286 - protein, 11 aa, synthetic construct
  MOD_RES 5: note = /replace="Val"
  MOD_RES 6: note = /replace="Ile"
  MOD_RES 7: note = /replace="Asn"
  MOD_RES 9: note = /replace="Phe"
  MOD_RES 10: note = /replace="Leu"
  REGION 1..11: note = misc_feature - /note="Variant residues given in the sequence have nopreference with respect to those in the annotationsfor variant positions"
  REGION 1..11: note = source = /note="Description of Artificial Sequence: Syntheticpeptide"
RASQDVSTAVA

SEQ ID NO: 287 - protein, 7 aa, synthetic construct
  MOD_RES 4: note = /replace="Thr"
  MOD_RES 6: note = /replace="Ala"
  REGION 1..7: note = misc_feature - /note="Variant residues given in the sequence have nopreference with respect to those in the annotationsfor variant positions"
  REGION 1..7: note = source = /note="Description of Artificial Sequence: Syntheticpeptide"
SASFLYS

SEQ ID NO: 288 - protein, 9 aa, synthetic construct
  MOD_RES 3: note = /replace="Gly" or "Phe" or "Ser"
  MOD_RES 4: note = /replace="Tyr" or "Phe" or "Trp"
  MOD_RES 5: note = /replace="Asn" or "Ala" or "Thr" or "Gly" or "Phe" or "Ile"
  MOD_RES 6: note = /replace="Val" or "Pro" or "Thr" or "Ile"
  MOD_RES 8: note = /replace="Trp" or "Arg" or "Pro" or "Thr"
  REGION 1..9: note = misc_feature - /note="Variant residues given in the sequence have nopreference with respect to those in the annotationsfor variant positions"
  REGION 1..9: note = source = /note="Description of Artificial Sequence: Syntheticpeptide"
QQYLYHPAT

SEQ ID NO: 289 - protein, 10 aa, synthetic construct
  REGION 1..10: note = source = /note="Description of Artificial Sequence: Syntheticpeptide"
GFTFSDSWIH

SEQ ID NO: 290 - protein, 18 aa, synthetic construct
  REGION 1..18: note = source = /note="Description of Artificial Sequence: Syntheticpeptide"
AWISPYGGSTYYADSVKG

SEQ ID NO: 291 - protein, 9 aa, synthetic construct
  REGION 1..9: note = source = /note="Description of Artificial Sequence: Syntheticpeptide"
RHWPGGFDY

SEQ ID NO: 292 - protein, 11 aa, synthetic construct
  REGION 1..11: note = source = /note="Description of Artificial Sequence: Syntheticpeptide"
RASQDVSTAVA

SEQ ID NO: 293 - protein, 7 aa, synthetic construct
  REGION 1..7: note = source = /note="Description of Artificial Sequence: Syntheticpeptide"
SASFLYS

SEQ ID NO: 294 - protein, 9 aa, synthetic construct
  REGION 1..9: note = source = /note="Description of Artificial Sequence: Syntheticpeptide"
QQYLYHPAT

SEQ ID NO: 295 - protein, 25 aa, synthetic construct [sequence omitted]

SEQ ID NO: 296 - protein, 13 aa, synthetic construct
  REGION 1..13: note = source = /note="Description of Artificial Sequence: Syntheticpeptide"
WVRQAPGKGLEWV

SEQ ID NO: 297 - protein, 32 aa, synthetic construct
  REGION 1..32: note = source = /note="Description of Artificial Sequence: Syntheticpolypeptide"
RFTISADTSKNTAYLQMNSLRAEDTAVYYCAR

SEQ ID NO: 298 - protein, 11 aa, synthetic construct
  REGION 1..11: note = source = /note="Description of Artificial Sequence: Syntheticpeptide"
WGQGTLVTVSA

SEQ ID NO: 299 - protein, 11 aa, synthetic construct
  REGION 1..11: note = source = /note="Description of Artificial Sequence: Syntheticpeptide"
WGQGTLVTVSS

SEQ ID NO: 300 - protein, 23 aa, synthetic construct
  REGION 1..23: note = source = /note="Description of Artificial Sequence: Syntheticpeptide"
DIQMTQSPSSLSASVGDRVTITC

SEQ ID NO: 301 - protein, 15 aa, synthetic construct
  REGION 1..15: note = source = /note="Description of Artificial Sequence: Syntheticpeptide"
WYQQKPGKAPKLLIY

SEQ ID NO: 302 - protein, 32 aa, synthetic construct
  REGION 1..32: note = source = /note="Description of Artificial Sequence: Syntheticpolypeptide"
GVPSRFSGSGSGTDFTLTISSLQPEDFATYYC

SEQ ID NO: 303 - protein, 11 aa, synthetic construct
  REGION 1..11: note = source = /note="Description of Artificial Sequence: Syntheticpeptide"
FGQGTKVEIKR

SEQ ID NO: 304 - protein, 9 aa, Mus musculus
GFSLSTSGM

SEQ ID NO: 305 - skipped

SEQ ID NO: 306 - protein, 8 aa, Mus musculus
NGYLYALD

SEQ ID NO: 307 - protein, 6 aa, Mus musculus
SSSVNY

SEQ ID NO: 308 - skipped

SEQ ID NO: 309 - protein, 7 aa, Mus musculus
WSSYPWT

SEQ ID NO: 310 - protein, 120 aa, Mus musculus
QVTLKESGPGILQPSQTLRLTCSFSGFSLSTSGMSVGWIRQPSGKGLEWLAHIWLNDDVFFNPALKSRLTISKDTSNNQVFLQIASVVTADTATYYCVRANGYLYALDYWGQGTSVTVSS

SEQ ID NO: 311 - protein, 106 aa, Mus musculus
QIVLTQSPAIMSASPGQKVTITCSASSSVNYTQWYQQKLGSSPKLWIYDAFKLAPGVPARFSGSGTGTSYSLTISSMEAEDAASYFCHQWSSYPWTFGGGTKLEIK

SEQ ID NO: 312 - protein, 120 aa, Mus musculus
QVTLKESGPGILQPSQTLSLTCSFSGFSLSTSGMSVGWIRQPSGKGLEWLAHIWLNDDVFFNPALKRRLTISKDTSNNQVFLQIASVVTADTATYYCVRANGYLYALDYWGQGISVTVSS

SEQ ID NO: 313 - protein, 106 aa, Mus musculus; identical to SEQ ID NO: 311

SEQ ID NO: 314 - protein, 6 aa, Mus musculus
SSSVQY

SEQ ID NO: 315 - protein, 6 aa, Mus musculus
SSSVSY

SEQ ID NO: 316 - protein, 7 aa, Mus musculus
GYSFTSY

SEQ ID NO: 317 - skipped

SEQ ID NO: 318 - protein, 9 aa, Mus musculus
GYYAWYYFD

SEQ ID NO: 319 - protein, 7 aa, Mus musculus
SQSIGNN

SEQ ID NO: 320 - skipped

SEQ ID NO: 321 - protein, 6 aa, Mus musculus
SNSWPL

SEQ ID NO: 322 - protein, 120 aa, Mus musculus
QVQLQQSGPQLVRPGASVQISCKASGYSFTSYLLHWLKQRPGQGLEWIGMIDPSDSETRLNQKFKDKATLTVDKSSSTAYMQLSSPTSEDSAVYYCARDGYYAWYYFDCWGQGTTLTVSS

SEQ ID NO: 323 - protein, 107 aa, Mus musculus
DIVLTQSPATLSVTPGDRVSLSCRASQSIGNNLHWYQQKSHESPRLLIKYASHSISGIPSKFSGTGSGTDFTLSFNSVETEDFGMYFCQQSNSWPLTFGAGTKLELK

SEQ ID NO: 324 - protein, 5 aa, Mus musculus
GDSIA

SEQ ID NO: 325 - skipped

SEQ ID NO: 326 - protein, 4 aa, Mus musculus
DYFD

SEQ ID NO: 327 - protein, 7 aa, Mus musculus
RQDVRKN

SEQ ID NO: 328 - skipped

SEQ ID NO: 329 - protein, 6 aa, Mus musculus
YDNLPF

SEQ ID NO: 330 - protein, 114 aa, Mus musculus
EVQLQESGPSLVKPSQTLSLTCSVTGDSIASAYWNWIRKFPGNKLEYMGYINYSGSTYYNPSLKSRISITRDTSQNQYYLQLNSVTTEDTATYYCVTGDYFDYWGRGTTLTVSS

SEQ ID NO: 331 - protein, 107 aa, Mus musculus
DIQMTQSPSSLSAYLGGKVTITCKARQDVRKNIGWYQHKPGKGPRLLIWYTSTLQSGIPSRFSGSGSGRDYSFNINNLEPEDIATYYCLQYDNLPFTFGTGTKLEIR

SEQ ID NO: 332 - protein, 5 aa, Mus musculus
GYTFT

SEQ ID NO: 333 - skipped

SEQ ID NO: 334 - protein, 4 aa, Mus musculus
GYPA

SEQ ID NO: 335 - protein, 12 aa, Mus musculus
SRTILHSSGNTY

SEQ ID NO: 336 - skipped

SEQ ID NO: 337 - protein, 6 aa, Mus musculus
DSHVPF

SEQ ID NO: 338 - protein, 115 aa, Mus musculus
QIQLVQSGPELKKPGETVKISCKASGYTFTDYSMHWVKQAPGRGLKWMGYINTETYEPTFGADFKGRFAFSLDTSATTAYLQINSLKTEDTATFFCGGGGYPAYWGQGTVVIVSA

SEQ ID NO: 339 - protein, 112 aa, Mus musculus
DVLMTQTPLSLPVSLGDQASISCRSSRTILHSSGNTYLEWYLQKPGQSPKLLIYKVSNRFSGVPDRFSGSGSGTDFTLNISRVEAEDLGVYYCFQDSHVPFTFGTGTKLEIK

SEQ ID NO: 340 - protein, 7 aa, Mus musculus
GFNIKTT

SEQ ID NO: 341 - skipped

SEQ ID NO: 342 - protein, 8 aa, Mus musculus
FGYVAWFA

SEQ ID NO: 343 - protein, 7 aa, Mus musculus
SQSVDNY

SEQ ID NO: 344 - skipped

SEQ ID NO: 345 - protein, 6 aa, Mus musculus
HYSSPY

SEQ ID NO: 346 - protein, 119 aa, Mus musculus
EVQLQQSVAELVRPGASVKLSCTASGFNIKTTYMHWVKQRPEQGLEWIGRIDPADDNTKYAPKFQGKATITADTSSNTAYLQLSSLTSEDAAIYYCVRDFGYVAWFAYWGQGTLVTFSA

SEQ ID NO: 347 - protein, 107 aa, Mus musculus
NIVMTPTPKFLPVSSGDRVTMTCRASQSVDNYVAWYQQKPGQSPKLLIYYASNRYIGVPDRFTGSGSGTDFTFTISSVQVEDLAVYFCQQHYSSPYTFGSGTKLEIK

SEQ ID NO: 348 - protein, 7 aa, Mus musculus
GYPFSEY

SEQ ID NO: 349 - skipped

SEQ ID NO: 350 - protein, 4 aa, Mus musculus
GYPA

SEQ ID NO: 351 - protein, 12 aa, Mus musculus
SRSIVHSSGNTY

SEQ ID NO: 352 - skipped

SEQ ID NO: 353 - protein, 5 aa, Mus musculus
DSHVP

SEQ ID NO: 354 - protein, 115 aa, Mus musculus
QIQLVQSGPELKKPGETVKISCKASGYPFSEYSIHWVKQAPGKGLKWMVYVNTETGQPIVGDDFRGRFVLSLETSASTAYLQINNLKNEDTATYFCGGGGYPAYWGQGTLVTVSA

SEQ ID NO: 355 - protein, 112 aa, Mus musculus
DVLMTQTPLSLPVSLGDQASISCRSSRSIVHSSGNTYLEWYLQKPGQSPKLLIYKVSNRFSGVPDRFSGSGSGTDFTLNISRVEAEDLGVYYCFQDSHVPFTFGTGTKLEIK

SEQ ID NO: 356 - protein, 7 aa, Mus musculus
GFTFSSS

SEQ ID NO: 357 - skipped

SEQ ID NO: 358 - protein, 8 aa, Mus musculus
YPHYYAMD

SEQ ID NO: 359 - protein, 7 aa, Mus musculus
SENIFSN

SEQ ID NO: 360 - skipped

SEQ ID NO: 361 - protein, 6 aa, Mus musculus
FYKIPF

SEQ ID NO: 362 - protein, 121 aa, Mus musculus
QGQMHQSGAELVKPGSSVKLSCKTSGFTFSSSFISWLKQKPGQSLEWIAWIYAATGSTSYNQKFTNKAQLTVDTSSSAAYMQFSSLTTEDSAIYYCARHAGYPHYYAMDYWGQGTSVTVSS

SEQ ID NO: 363 - protein, 107 aa, Mus musculus
DIQMTQSPASLSASVGETVTITCRASENIFSNLAWYQQKQGKSPQLLVYSATNLGDGVPSRFSGSGSGTQFSLKINSLQPEDFGNYYCQHFYKIPFTFGTGTKLEIK

SEQ ID NO: 364 - protein, 7 aa, Mus musculus
GFNIKDY

SEQ ID NO: 365 - skipped

SEQ ID NO: 366 - protein, 8 aa, Mus musculus
HGYVGWFA

SEQ ID NO: 367 - protein, 8 aa, Mus musculus
ASENVDTY

SEQ ID NO: 368 - skipped

SEQ ID NO: 369 - protein, 6 aa, Mus musculus
SYSYPW

SEQ ID NO: 370 - protein, 119 aa, Mus musculus
EVQLQQSGAEPLKPGASVKLTCTTSGFNIKDYYIHWVKQRSDQGLEWIGRIDPEDGELIYAPKFQDKATITVDTSSNIAYLQLNSLTSEDTAVYYCSRDHGYVGWFAYWGQGTLVTVSA

SEQ ID NO: 371 - protein, 107 aa, Mus musculus
NVVMTQSPKSMIMSVGQRVTLNCKASENVDTYVSWYQQKPEQSPKLLIYGASNRYTGVPDRFTGSRSATDFTLTISSVQAEDLAVYYCGQSYSYPWTFGGGTKLEFR

SEQ ID NO: 372 - protein, 219 aa, synthetic construct
  REGION 1..219: note = source = /note="Description of Artificial Sequence: Syntheticpolypeptide"
PTGAEFLGDGGDVSFSTRGTQNWTVERLLQAHAQLEERGYVFVGYHGTFLEAAQSIVFGGVAARSQDLAAIWAGFYIAGDPALAYGYAQDQEPDAAGRIRNGALLRVYVPASSLPGFYRTSLTLAAPEAAGEVERLIGHPLPLALDAITGPEEEGGRLETILGWPLAERTVVIPSAIPTDPRNVGGDLDPSSIPDKEQAISALPDYASQPGKPPREDLK

SEQ ID NO: 373 - protein, 219 aa, synthetic construct
  REGION 1..219: note = source = /note="Description of Artificial Sequence: Syntheticpolypeptide"
PTGAEFLGDGGDVSFSTRGTQNWTVERLLQAHAQLEERGYVFVGYHGTALEAAQSIVFGGVRARSQDLRAIWRGFYIAGDPAHAYGYAQDQEPDARGRIANGALLRVYVPASSLPGFYRTSLTLAAPEAAGEVERLIGHPLPLRLDAITGPEEEGGREETILGWPLAERTVVIPSAIPTDPRNVGGDLDPSSIPDKEQAISALPDYASQPGKPPREDLK

SEQ ID NO: 374 - protein, 107 aa, Homo sapiens [sequence omitted]

SEQ ID NO: 375 - protein, 105 aa, Homo sapiens
QPKAAPSVTLFPPSSEELQANKATLVCLISDFYPGAVTVAWKADSSPVKAGVETTTPSKQSNNKYAASSYLSLTPEQWKSHRSYSCQVTHEGSTVEKTVAPTECS

SEQ ID NO: 376 - protein, 330 aa, Homo sapiens [sequence omitted]

SEQ ID NO: 377 - protein, 330 aa, Homo sapiens
ASTKGPSVFPLAPSSKSTSGGTAALGCLVKDYFPEPVTVSWNSGALTSGVHTFPAVLQSSGLYSLSSVVTVPSSSLGTQTYICNVNHKPSNTKVDKKVEPKSCDKTHTCPPCPAPEAAGGPSVFLFPPKPKDTLMISRTPEVTCVVVDVSHEDPEVKFNWYVDGVEVHNAKTKPREEQYNSTYRVVSVLTVLHQDWLNGKEYKCKVSNKALPAPIEKTISKAKGQPREPQVYTLPPSRDELTKNQVSLTCLVKGFYPSDIAVEWESNGQPENNYKTTPPVLDSDGSFFLYSKLTVDKSRWQQGNVFSCSVMHEALHNHYTQKSLSLSPGK

SEQ ID NO: 378 - protein, 330 aa, Homo sapiens
ASTKGPSVFPLAPSSKSTSGGTAALGCLVKDYFPEPVTVSWNSGALTSGVHTFPAVLQSSGLYSLSSVVTVPSSSLGTQTYICNVNHKPSNTKVDKKVEPKSCDKTHTCPPCPAPEAAGGPSVFLFPPKPKDTLMISRTPEVTCVVVDVSHEDPEVKFNWYVDGVEVHNAKTKPREEQYNSTYRVVSVLTVLHQDWLNGKEYKCKVSNKALGAPIEKTISKAKGQPREPQVYTLPPSRDELTKNQVSLTCLVKGFYPSDIAVEWESNGQPENNYKTTPPVLDSDGSFFLYSKLTVDKSRWQQGNVFSCSVMHEALHNHYTQKSLSLSPGK

SEQ ID NO: 379 - protein, 327 aa, Homo sapiens
ASTKGPSVFPLAPCSRSTSESTAALGCLVKDYFPEPVTVSWNSGALTSGVHTFPAVLQSSGLYSLSSVVTVPSSSLGTKTYTCNVDHKPSNTKVDKRVESKYGPPCPSCPAPEFLGGPSVFLFPPKPKDTLMISRTPEVTCVVVDVSQEDPEVQFNWYVDGVEVHNAKTKPREEQFNSTYRVVSVLTVLHQDWLNGKEYKCKVSNKGLPSSIEKTISKAKGQPREPQVYTLPPSQEEMTKNQVSLTCLVKGFYPSDIAVEWESNGQPENNYKTTPPVLDSDGSFFLYSRLTVDKSRWQEGNVFSCSVMHEALHNHYTQKSLSLSLGK

SEQ ID NO: 380 - protein, 280 aa, Homo sapiens
SEVEYRAEVGQNAYLPCFYTPAAPGNLVPVCWGKGACPVFECGNVVLRTDERDVNYWTSRYWLNGDFRKGDVSLTIENVTLADSGIYCCRIQIPGIMNDEKFNLKLVIKPAKVTPAPTRQRDFTAAFPRMLTTRGHGPAETQTLGSLPDINLTQISTLANELRDSRLANDLRDSGATIRIGIYIGAGICAGLALALIFGALIFKWYSHSKEKIQNLSLISLANLPPSGLANAVAEGIRSEENIYTIEENVYEVEEPNEYYCYVSSRQQPSQPLGCRFAMP

SEQ ID NO: 381 - protein, 181 aa, Homo sapiens
SEVEYRAEVGQNAYLPCFYTPAAPGNLVPVCWGKGACPVFECGNVVLRTDERDVNYWTSRYWLNGDFRKGDVSLTIENVTLADSGIYCCRIQIPGIMNDEKFNLKLVIKPAKVTPAPTRQRDFTAAFPRMLTTRGHGPAETQTLGSLPDINLTQISTLANELRDSRLANDLRDSGATIRIG

SEQ ID NO: 382 - protein, 118 aa, synthetic construct
  REGION 1..118: note = source = /note="Description of Artificial Sequence: Syntheticpolypeptide"
EVQLVESGGGLVQPGGSLRLSCAASGFTFSDSWIHWVRQAPGKGLEWVAWISPYGGSTYYADSVKGRFTISADTSKNTAYLQMNSLRAEDTAVYYCARRHWPGGFDYWGQGTLVTVSA

SEQ ID NO: 383 - protein, 108 aa, synthetic construct; identical to SEQ ID NO: 282
  REGION 1..108: note = source = /note="Description of Artificial Sequence: Syntheticpolypeptide"

SEQ ID NO: 384 - protein, 24 aa, synthetic construct
  VARIANT 13..24: note = /replace=" "
  REGION 1..24: note = MISC_FEATURE - /note="This sequence may encompass 3-6 "Gly Gly Gly Ser"repeating units"
  REGION 1..24: note = MISC_FEATURE - /note="Variant residues given in the sequence have nopreference with respect to those in the annotationsfor variant positions"
  REGION 1..24: note = source = /note="Description of Artificial Sequence: Syntheticpeptide"
GGGSGGGSGGGSGGGSGGGSGGGS

SEQ ID NO: 385 - protein, 25 aa, synthetic construct
  VARIANT 11..25: note = /replace=" "
  REGION 1..25: note = MISC_FEATURE - /note="This sequence may encompass 2-5 "Gly Gly Gly Gly Ser"repeating units"
  REGION 1..25: note = MISC_FEATURE - /note="Variant residues given in the sequence have nopreference with respect to those in the annotationsfor variant positions"
  REGION 1..25: note = source = /note="Description of Artificial Sequence: Syntheticpeptide"
GGGGSGGGGSGGGGSGGGGSGGGGS

SEQ ID NO: 386 - protein, 10 aa, synthetic construct
  REGION 1..10: note = source = /note="Description of Artificial Sequence: Syntheticpeptide"
GGGGSGGGGS

SEQ ID NO: 387 - protein, 50 aa, synthetic construct
  VARIANT 6..50: note = /replace=" "
  REGION 1..50: note = MISC_FEATURE - /note="This sequence may encompass 1-10 "Gly Gly Gly Gly Ser"repeating units"
  REGION 1..50: note = MISC_FEATURE - /note="Variant residues given in the sequence have nopreference with respect to those in the annotationsfor variant positions"
  REGION 1..50: note = source = /note="Description of Artificial Sequence: Syntheticpolypeptide"
GGGGSGGGGSGGGGSGGGGSGGGGSGGGGSGGGGSGGGGSGGGGSGGGGS

SEQ ID NO: 388 - protein, 50 aa, synthetic construct
  VARIANT 6..50: note = /replace=" "
  REGION 1..50: note = MISC_FEATURE - /note="This sequence may encompass 1-10 "Ser Gly Gly Gly Gly"repeating units"
  REGION 1..50: note = MISC_FEATURE - /note="Variant residues given in the sequence have nopreference with respect to those in the annotationsfor variant positions"
  REGION 1..50: note = source = /note="Description of Artificial Sequence: Syntheticpolypeptide"
SGGGGSGGGGSGGGGSGGGGSGGGGSGGGGSGGGGSGGGGSGGGGSGGGG

SEQ ID NO: 389 - protein, 54 aa, synthetic construct
  VARIANT 10..54: note = /replace=" "
  REGION 5..54: note = MISC_FEATURE - /note="This region may encompass 1-10 "Ser Gly Gly Gly Gly"repeating units"
  REGION 1..54: note = MISC_FEATURE - /note="Variant residues given in the sequence have nopreference with respect to those in the annotationsfor variant positions"
  REGION 1..54: note = source = /note="Description of Artificial Sequence: Syntheticpolypeptide"
GGGGSGGGGSGGGGSGGGGSGGGGSGGGGSGGGGSGGGGSGGGGSGGGGSGGGG

SEQ ID NO: 390 - protein, 15 aa, synthetic construct
  REGION 1..15: note = source = /note="Description of Artificial Sequence: Syntheticpeptide"
EPKSCGGGGSGGGGS

SEQ ID NO: 391 - protein, 16 aa, synthetic construct
  REGION 1..16: note = source = /note="Description of Artificial Sequence: Syntheticpeptide"
EPKSCDGGGGSGGGGS

SEQ ID NO: 392 - protein, 5 aa, synthetic construct
  REGION 1..5: note = source = /note="Description of Artificial Sequence: Synthetic5xHis tag"
HHHHH

SEQ ID NO: 393 - protein, 692 aa, synthetic construct
  REGION 1..692: note = source = /note="Description of Artificial Sequence: Syntheticpolypeptide"
QVQLVQSGAEVKKPGASVKVSCKASGYTFTSYYMHWVRQAPGQGLEWMGIINPSGGSTSYAQKFQGRVTMTHDTSTSTVYMELSSLRSEDTAVYYCARSFFTGFHLDYWGQGTLVTVSSASTKGPSVFPLAPSSKSTSGGTAALGCLVKDYFPEPVTVSWNSGALTSGVHTFPAVLQSSGLYSLSSVVTVPSSSLGTQTYICNVNHKPSNTKVDKKVEPKSCDGGGGSGGGGSEVQLLESGGGLVQPGGSLRLSCAASGFTFSTYAMNWVRQAPGKGLEWVSRIRSKYNNYATYYADSVKGRFTISRDDSKNTLYLQMNSLRAEDTAVYYCVRHGNFGNSYVSWFAYWGQGTLVTVSSASVAAPSVFIFPPSDEQLKSGTASVVCLLNNFYPREAKVQWKVDNALQSGNSQESVTEQDSKDSTYSLSSTLTLSKADYEKHKVYACEVTHQGLSSPVTKSFNRGECDKTHTCPPCPAPEAAGGPSVFLFPPKPKDTLMISRTPEVTCVVVDVSHEDPEVKFNWYVDGVEVHNAKTKPREEQYNSTYRVVSVLTVLHQDWLNGKEYKCKVSNKALGAPIEKTISKAKGQPREPQVYTLPPCRDELTKNQVSLWCLVKGFYPSDIAVEWESNGQPENNYKTTPPVLDSDGSFFLYSKLTVDKSRWQQGNVFSCSVMHEALHNHYTQKSLSLSPGK

SEQ ID NO: 394 - protein, 449 aa, synthetic construct
  REGION 1..449: note = source = /note="Description of Artificial Sequence: Syntheticpolypeptide"
QVQLVQSGAEVKKPGASVKVSCKASGYTFTSYYMHWVRQAPGQGLEWMGIINPSGGSTSYAQKFQGRVTMTHDTSTSTVYMELSSLRSEDTAVYYCARSFFTGFHLDYWGQGTLVTVSSASTKGPSVFPLAPSSKSTSGGTAALGCLVKDYFPEPVTVSWNSGALTSGVHTFPAVLQSSGLYSLSSVVTVPSSSLGTQTYICNVNHKPSNTKVDKKVEPKSCDKTHTCPPCPAPEAAGGPSVFLFPPKPKDTLMISRTPEVTCVVVDVSHEDPEVKFNWYVDGVEVHNAKTKPREEQYNSTYRVVSVLTVLHQDWLNGKEYKCKVSNKALGAPIEKTISKAKGQPREPQVCTLPPSRDELTKNQVSLSCAVKGFYPSDIAVEWESNGQPENNYKTTPPVLDSDGSFFLVSKLTVDKSRWQQGNVFSCSVMHEALHNHYTQKSLSLSPGK

SEQ ID NO: 395 - protein, 216 aa, synthetic construct
  MOD_RES 201: note = Any amino acid
  REGION 1..216: note = source = /note="Description of Artificial Sequence: Syntheticpolypeptide"
EIVLTQSPGTLSLSPGERATLSCRASQSVSSSYLAWYQQKPGQAPRLLIYGASSRATGIPDRFSGSGSGTDFTLTISRLEPEDFAVYYCQQYTNEHYYTFGQGTKVEIKRTVAAPSVFIFPPSDEQLKSGTASVVCLLNNFYPREAKVQWKVDNALQSGNSQESVTEQDSKDSTYSLSSTLTLSKADYEKHKVYACEVTHXGLSSPVTKSFNRGEC

SEQ ID NO: 396 - protein, 7 aa, synthetic construct
  REGION 1..7: note = source = /note="Description of Artificial Sequence: Syntheticpeptide"
GTNARAP

SEQ ID NO: 397 - protein, 9 aa, synthetic construct
  REGION 1..9: note = source = /note="Description of Artificial Sequence: Syntheticpeptide"
ALWYANLWV

SEQ ID NO: 398 - protein, 5 aa, synthetic construct
  REGION 1..5: note = source = /note="Description of Artificial Sequence: Syntheticpeptide"
NAWMH

SEQ ID NO: 399 - protein, 19 aa, synthetic construct
  REGION 1..19: note = source = /note="Description of Artificial Sequence: Syntheticpeptide"
SIKSKTDGGTTDYAAPVKG

SEQ ID NO: 400 - protein, 9 aa, synthetic construct
  REGION 1..9: note = source = /note="Description of Artificial Sequence: Syntheticpeptide"
PYEWSWYDY

SEQ ID NO: 401 - protein, 120 aa, synthetic construct
  REGION 1..120: note = source = /note="Description of Artificial Sequence: Syntheticpolypeptide"
EVQLVESGGGLVKPGGSLRLSCAASGFTFSNAWMSWVRQAPGKGLEWVGRIKSKTEGGTTDYAAPVKGRFTISRDDSKNTLYLQMNSLKTEDTAVYYCTTPYEWSWYDYWGQGTLVTVSS

SEQ ID NO: 402 - protein, 19 aa, synthetic construct
  REGION 1..19: note = source = /note="Description of Artificial Sequence: Syntheticpeptide"
RIKSKTEGGTTDYAAPVKG

SEQ ID NO: 403 - protein, 689 aa, synthetic construct
  REGION 1..689: note = source = /note="Description of Artificial Sequence: Syntheticpolypeptide"
EVQLVESGGGLVKPGGSLRLSCAASGFTFSNAWMSWVRQAPGKGLEWVGRIKSKTEGGTTDYAAPVKGRFTISRDDSKNTLYLQMNSLKTEDTAVYYCTTPYEWSWYDYWGQGTLVTVSSASTKGPSVFPLAPSSKSTSGGTAALGCLVKDYFPEPVTVSWNSGALTSGVHTFPAVLQSSGLYSLSSVVTVPSSSLGTQTYICNVNHKPSNTKVDKKVEPKSCDGGGGSGGGGSEVQLLESGGGLVQPGGSLRLSCAASGFTFSTYAMNWVRQAPGKGLEWVSRIRSKYNNYATYYADSVKGRFTISRDDSKNTLYLQMNSLRAEDTAVYYCVRHGNFGNSYVSWFAYWGQGTLVTVSSASTKGPSVFPLAPSSKSTSGGTAALGCLVKDYFPEPVTVSWNSGALTSGVHTFPAVLQSSGLYSLSSVVTVPSSSLGTQTYICNVNHKPSNTKVDKKVEPKSCDKTHTCPPCPAPEAAGGPSVFLFPPKPKDTLMISRTPEVTCVVVDVSHEDPEVKFNWYVDGVEVHNAKTKPREEQYNSTYRVVSVLTVLHQDWLNGKEYKCKVSNKALGAPIEKTISKAKGQPREPQVYTLPPCRDELTKNQVSLWCLVKGFYPSDIAVEWESNGQPENNYKTTPPVLDSDGSFFLYSKLTVDKSRWQQGNVFSCSVMHEALHNHYTQKSLSLSPGK

SEQ ID NO: 404 - protein, 450 aa, synthetic construct
  REGION 1..450: note = source = /note="Description of Artificial Sequence: Syntheticpolypeptide"
EVQLVESGGGLVKPGGSLRLSCAASGFTFSNAWMSWVRQAPGKGLEWVGRIKSKTEGGTTDYAAPVKGRFTISRDDSKNTLYLQMNSLKTEDTAVYYCTTPYEWSWYDYWGQGTLVTVSSASTKGPSVFPLAPSSKSTSGGTAALGCLVKDYFPEPVTVSWNSGALTSGVHTFPAVLQSSGLYSLSSVVTVPSSSLGTQTYICNVNHKPSNTKVDKKVEPKSCDKTHTCPPCPAPEAAGGPSVFLFPPKPKDTLMISRTPEVTCVVVDVSHEDPEVKFNWYVDGVEVHNAKTKPREEQYNSTYRVVSVLTVLHQDWLNGKEYKCKVSNKALGAPIEKTISKAKGQPREPQVCTLPPSRDELTKNQVSLSCAVKGFYPSDIAVEWESNGQPENNYKTTPPVLDSDGSFFLVSKLTVDKSRWQQGNVFSCSVMHEALHNRFTQKSLSLSPGK

SEQ ID NO: 405 - protein, 119 aa, synthetic construct
  REGION 1..119: note = source = /note="Description of Artificial Sequence: Syntheticpolypeptide"
EVQLLESGGGLVQPGGSLRLSCAASGFTFSSYAMSWVRQAPGKGLEWVSAISGSGGSTYYADSVKGRFTISRDNSKNTLYLQMNSLRAEDTAVYYCARGDYRYRYFDYWGQGTLVTVSS

SEQ ID NO: 406 - protein, 109 aa, synthetic construct
  REGION 1..109: note = source = /note="Description of Artificial Sequence: Syntheticpolypeptide"
SSELTQDPAVSVALGQTVRITCQGDSLRSYYASWYQQKPGQAPVLVIYGKNNRPSGIPDRFSGSSSGNTASLTITGAQAEDEADYYCNSRESPPTGLVVFGGGTKLTVL

SEQ ID NO: 407 - protein, 674 aa, synthetic construct
  REGION 1..674: note = source = /note="Description of Artificial Sequence: Syntheticpolypeptide"
EVQLLESGGGLVQPGGSLRLSCAASGFTFSSYAMSWVRQAPGKGLEWVSAISGSGGSTYYADSVKGRFTISRDNSKNTLYLQMNSLRAEDTAVYYCARGDYRYRYFDYWGQGTLVTVSSASTKGPSVFPLAPSSKSTSGGTAALGCLVEDYFPEPVTVSWNSGALTSGVHTFPAVLQSSGLYSLSSVVTVPSSSLGTQTYICNVNHKPSNTKVDEKVEPKSCDGGGGSGGGGSQAVVTQEPSLTVSPGGTVTLTCGSSTGAVTTSNYANWVQEKPGQAFRGLIGGTNKRAPGTPARFSGSLLGGKAALTLSGAQPEDEAEYYCALWYSNLWVFGGGTKLTVLSSASTKGPSVFPLAPSSKSTSGGTAALGCLVKDYFPEPVTVSWNSGALTSGVHTFPAVLQSSGLYSLSSVVTVPSSSLGTQTYICNVNHKPSNTKVDKKVEPKSCDKTHTCPPCPAPEAAGGPSVFLFPPKPKDTLMISRTPEVTCVVVDVSHEDPEVKFNWYVDGVEVHNAKTKPREEQYNSTYRVVSVLTVLHQDWLNGKEYKCKVSNKALGAPIEKTISKAKGQPREPQVYTLPPCRDELTKNQVSLWCLVKGFYPSDIAVEWESNGQPENNYKTTPPVLDSDGSFFLYSKLTVDKSRWQQGNVFSCSVMHEALHNHYTQKSLSLSPGK

SEQ ID NO: 408 - protein, 449 aa, synthetic construct
  REGION 1..449: note = source = /note="Description of Artificial Sequence: Syntheticpolypeptide"
EVQLLESGGGLVQPGGSLRLSCAASGFTFSSYAMSWVRQAPGKGLEWVSAISGSGGSTYYADSVKGRFTISRDNSKNTLYLQMNSLRAEDTAVYYCARGDYRYRYFDYWGQGTLVTVSSASTKGPSVFPLAPSSKSTSGGTAALGCLVEDYFPEPVTVSWNSGALTSGVHTFPAVLQSSGLYSLSSVVTVPSSSLGTQTYICNVNHKPSNTKVDEKVEPKSCDKTHTCPPCPAPEAAGGPSVFLFPPKPKDTLMISRTPEVTCVVVDVSHEDPEVKFNWYVDGVEVHNAKTKPREEQYNSTYRVVSVLTVLHQDWLNGKEYKCKVSNKALGAPIEKTISKAKGQPREPQVCTLPPSRDELTKNQVSLSCAVKGFYPSDIAVEWESNGQPENNYKTTPPVLDSDGSFFLVSKLTVDKSRWQQGNVFSCSVMHEALHNHYTQKSLSLSPGK

SEQ ID NO: 409 - protein, 215 aa, synthetic construct
  REGION 1..215: note = source = /note="Description of Artificial Sequence: Syntheticpolypeptide"
SSELTQDPAVSVALGQTVRITCQGDSLRSYYASWYQQKPGQAPVLVIYGKNNRPSGIPDRFSGSSSGNTASLTITGAQAEDEADYYCNSRESPPTGLVVFGGGTKLTVLGQPKAAPSVTLFPPSSKKLQANKATLVCLISDFYPGAVTVAWKADSSPVKAGVETTTPSKQSNNKYAASSYLSLTPEQWKSHRSYSCQVTHEGSTVEKTVAPTECS

SEQ ID NO: 410 - protein, 118 aa, synthetic construct
  REGION 1..118: note = source = /note="Description of Artificial Sequence: Syntheticpolypeptide"
QVQLVQSGAEVKKPGASVKVSCKASGYTFTSYYMHWVRQAPGQGLEWMGIINPSGGSTSYAQKFQGRVTMTRDTSTSTVYMELSSLRSEDTAVYYCARGDWSYYMDYWGQGTLVTVSS

SEQ ID NO: 411 - protein, 111 aa, synthetic construct
  REGION 1..111: note = source = /note="Description of Artificial Sequence: Syntheticpolypeptide"
DIVMTQSPLSLPVTPGEPASISCRSSQSLLHSNGYNYLDWYLQKPGQSPQLLIYLGSNRASGVPDRFSGSGSGTDFTLKISRVEAEDVGVYYCMQARQTPTFGQGTKVEIK

SEQ ID NO: 412 - protein, 673 aa, synthetic construct
  REGION 1..673: note = source = /note="Description of Artificial Sequence: Syntheticpolypeptide"
QVQLVQSGAEVKKPGASVKVSCKASGYTFTSYYMHWVRQAPGQGLEWMGIINPSGGSTSYAQKFQGRVTMTRDTSTSTVYMELSSLRSEDTAVYYCARGDWSYYMDYWGQGTLVTVSSASTKGPSVFPLAPSSKSTSGGTAALGCLVEDYFPEPVTVSWNSGALTSGVHTFPAVLQSSGLYSLSSVVTVPSSSLGTQTYICNVNHKPSNTKVDEKVEPKSCDGGGGSGGGGSQAVVTQEPSLTVSPGGTVTLTCGSSTGAVTTSNYANWVQEKPGQAFRGLIGGTNKRAPGTPARFSGSLLGGKAALTLSGAQPEDEAEYYCALWYSNLWVFGGGTKLTVLSSASTKGPSVFPLAPSSKSTSGGTAALGCLVKDYFPEPVTVSWNSGALTSGVHTFPAVLQSSGLYSLSSVVTVPSSSLGTQTYICNVNHKPSNTKVDKKVEPKSCDKTHTCPPCPAPEAAGGPSVFLFPPKPKDTLMISRTPEVTCVVVDVSHEDPEVKFNWYVDGVEVHNAKTKPREEQYNSTYRVVSVLTVLHQDWLNGKEYKCKVSNKALGAPIEKTISKAKGQPREPQVYTLPPCRDELTKNQVSLWCLVKGFYPSDIAVEWESNGQPENNYKTTPPVLDSDGSFFLYSKLTVDKSRWQQGNVFSCSVMHEALHNHYTQKSLSLSPGK

SEQ ID NO: 413 - protein, 448 aa, synthetic construct
  REGION 1..448: note = source = /note="Description of Artificial Sequence: Syntheticpolypeptide"
QVQLVQSGAEVKKPGASVKVSCKASGYTFTSYYMHWVRQAPGQGLEWMGIINPSGGSTSYAQKFQGRVTMTRDTSTSTVYMELSSLRSEDTAVYYCARGDWSYYMDYWGQGTLVTVSSASTKGPSVFPLAPSSKSTSGGTAALGCLVEDYFPEPVTVSWNSGALTSGVHTFPAVLQSSGLYSLSSVVTVPSSSLGTQTYICNVNHKPSNTKVDEKVEPKSCDKTHTCPPCPAPEAAGGPSVFLFPPKPKDTLMISRTPEVTCVVVDVSHEDPEVKFNWYVDGVEVHNAKTKPREEQYNSTYRVVSVLTVLHQDWLNGKEYKCKVSNKALGAPIEKTISKAKGQPREPQVCTLPPSRDELTKNQVSLSCAVKGFYPSDIAVEWESNGQPENNYKTTPPVLDSDGSFFLVSKLTVDKSRWQQGNVFSCSVMHEALHNHYTQKSLSLSPGK

SEQ ID NO: 414 - protein, 218 aa, synthetic construct
  REGION 1..218: note = source = /note="Description of Artificial Sequence: Syntheticpolypeptide"
DIVMTQSPLSLPVTPGEPASISCRSSQSLLHSNGYNYLDWYLQKPGQSPQLLIYLGSNRASGVPDRFSGSGSGTDFTLKISRVEAEDVGVYYCMQARQTPTFGQGTKVEIKRTVAAPSVFIFPPSDRKLKSGTASVVCLLNNFYPREAKVQWKVDNALQSGNSQESVTEQDSKDSTYSLSSTLTLSKADYEKHKVYACEVTHQGLSSPVTKSFNRGEC

SEQ ID NO: 415 - DNA, 360 bp, synthetic construct
  misc_feature 1..360: note = source = /note="Description of Artificial Sequence: Syntheticpolynucleotide"
  source 1..360: mol_type = other DNA
gaggtgcaattggtggaaagcggaggcggcctcgtgaagcctggcggatctctgagactgagctgtgccgccagcggcttcaccttcagcaacgcctggatgagctgggtgcgccaggcccctggaaaaggactcgagtgggtgggacggatcaagagcaagaccgagggcggcaccaccgactatgccgcccctgtgaagggccggttcaccatcagcagggacgacagcaagaacaccctgtacctgcagatgaacagcctgaaaaccgaggacaccgccgtgtactactgcaccaccccctacgagtggtcttggtacgactactggggccagggcaccctcgtgaccgtgtcatct

SEQ ID NO: 416 - DNA, 2067 bp, synthetic construct
  misc_feature 1..2067: note = source = /note="Description of Artificial Sequence: Syntheticpolynucleotide"
  source 1..2067: mol_type = other DNA
gaggtgcaattggtggaaagcggaggcggcctcgtgaagcctggcggatctctgagactgagctgtgccgccagcggcttcaccttcagcaacgcctggatgagctgggtgcgccaggcccctggaaaaggactcgagtgggtgggacggatcaagagcaagaccgagggcggcaccaccgactatgccgcccctgtgaagggccggttcaccatcagcagggacgacagcaagaacaccctgtacctgcagatgaacagcctgaaaaccgaggacaccgccgtgtactactgcaccaccccctacgagtggtcttggtacgactactggggccagggcaccctcgtgaccgtgtcatctgctagcacaaagggccctagcgtgttccctctggcccccagcagcaagagcacaagcggcggaacagccgccctgggctgcctcgtgaaggactacttccccgagcccgtgacagtgtcttggaacagcggagccctgacaagcggcgtgcacaccttccctgccgtgctgcagagcagcggcctgtactccctgagcagcgtggtcaccgtgcctagcagcagcctgggcacccagacctacatctgcaacgtgaaccacaagcccagcaacaccaaagtggacaagaaggtggagcccaagagctgtgatggcggaggagggtccggaggcggaggatccgaggtgcagctgctggaatctggcggcggactggtgcagcctggcggatctctgagactgagctgtgccgccagcggcttcaccttcagcacctacgccatgaactgggtgcgccaggcccctggcaaaggcctggaatgggtgtcccggatcagaagcaagtacaacaactacgccacctactacgccgacagcgtgaagggccggttcaccatcagccgggacgacagcaagaacaccctgtacctgcagatgaacagcctgcgggccgaggacaccgccgtgtactattgtgtgcggcacggcaacttcggcaacagctatgtgtcttggtttgcctactggggccagggcaccctcgtgaccgtgtcaagcgctagtaccaagggccccagcgtgttccccctggcacccagcagcaagagcacatctggcggaacagccgctctgggctgtctggtgaaagactacttccccgagcccgtgaccgtgtcttggaactctggcgccctgaccagcggcgtgcacacctttccagccgtgctgcagagcagcggcctgtactccctgtcctccgtggtcaccgtgccctctagctccctgggaacacagacatatatctgtaatgtcaatcacaagccttccaacaccaaagtcgataagaaagtcgagcccaagagctgcgacaaaactcacacatgcccaccgtgcccagcacctgaagctgcagggggaccgtcagtcttcctcttccccccaaaacccaaggacaccctcatgatctcccggacccctgaggtcacatgcgtggtggtggacgtgagccacgaagaccctgaggtcaagttcaactggtacgtggacggcgtggaggtgcataatgccaagacaaagccgcgggaggagcagtacaacagcacgtaccgtgtggtcagcgtcctcaccgtcctgcaccaggactggctgaatggcaaggagtacaagtgcaaggtctccaacaaagccctcggcgcccccatcgagaaaaccatctccaaagccaaagggcagccccgagaaccacaggtgtacaccctgcccccatgccgggatgagctgaccaagaaccaggtcagcctgtggtgcctggtcaaaggcttctatcccagcgacatcgccgtggagtgggagagcaatgggcagccggagaacaactacaagaccacgcctcccgtgctggactccgacggctccttcttcctctacagcaagctcaccgtggacaagagcaggtggcagcaggggaacgtcttctcatgctccgtgatgcatgaggctctgcacaaccactacacgcagaagagcctctccctgtctccgggtaaa

SEQ ID NO: 417 - DNA, 1350 bp, synthetic construct
  misc_feature 1..1350: note = source = /note="Description of Artificial Sequence: Syntheticpolynucleotide"
  source 1..1350: mol_type = other DNA
gaggtgcaattggtggaaagcggaggcggcctcgtgaagcctggcggatctctgagactgagctgtgccgccagcggcttcaccttcagcaacgcctggatgagctgggtgcgccaggcccctggaaaaggactcgagtgggtgggacggatcaagagcaagaccgagggcggcaccaccgactatgccgcccctgtgaagggccggttcaccatcagcagggacgacagcaagaacaccctgtacctgcagatgaacagcctgaaaaccgaggacaccgccgtgtactactgcaccaccccctacgagtggtcttggtacgactactggggccagggcaccctcgtgaccgtgtcatctgctagcaccaagggcccctccgtgttccccctggcccccagcagcaagagcaccagcggcggcacagccgctctgggctgcctggtcaaggactacttccccgagcccgtgaccgtgtcctggaacagcggagccctgacctccggcgtgcacaccttccccgccgtgctgcagagttctggcctgtatagcctgagcagcgtggtcaccgtgccttctagcagcctgggcacccagacctacatctgcaacgtgaaccacaagcccagcaacaccaaggtggacaagaaggtggagcccaagagctgcgacaaaactcacacatgcccaccgtgcccagcacctgaagctgcagggggaccgtcagtcttcctcttccccccaaaacccaaggacaccctcatgatctcccggacccctgaggtcacatgcgtggtggtggacgtgagccacgaagaccctgaggtcaagttcaactggtacgtggacggcgtggaggtgcataatgccaagacaaagccgcgggaggagcagtacaacagcacgtaccgtgtggtcagcgtcctcaccgtcctgcaccaggactggctgaatggcaaggagtacaagtgcaaggtctccaacaaagccctcggcgcccccatcgagaaaaccatctccaaagccaaagggcagccccgagaaccacaggtgtgcaccctgcccccatcccgggatgagctgaccaagaaccaggtcagcctctcgtgcgcagtcaaaggcttctatcccagcgacatcgccgtggagtgggagagcaatgggcagccggagaacaactacaagaccacgcctcccgtgctggactccgacggctccttcttcctcgtgagcaagctcaccgtggacaagagcaggtggcagcaggggaacgtcttctcatgctccgtgatgcatgaggctctgcacaaccgcttcacgcagaagagcctctccctgtctccgggtaaa

SEQ ID NO: 418 - DNA, 357 bp, synthetic construct
  misc_feature 1..357: note = source = /note="Description of Artificial Sequence: Syntheticpolynucleotide"
  source 1..357: mol_type = other DNA
gaggtgcaattgttggagtctgggggaggcttggtacagcctggggggtccctgagactctcctgtgcagcctccggattcacctttagcagttatgccatgagctgggtccgccaggctccagggaaggggctggagtgggtctcagctattagtggtagtggtggtagcacatactacgcagactccgtgaagggccggttcaccatctccagagacaattccaagaacacgctgtatctgcagatgaacagcctgagagccgaggacacggccgtatattactgtgcgcgtggtgactaccgttaccgttacttcgactactggggccaaggaaccctggtcaccgtctcgagt

SEQ ID NO: 419 - DNA, 327 bp, synthetic construct
  misc_feature 1..327: note = source = /note="Description of Artificial Sequence: Syntheticpolynucleotide"
  source 1..327: mol_type = other DNA
tcttctgaactgactcaagatccagctgttagcgtggctctgggtcagactgtacgtatcacctgccaaggcgattctctgcgctcctactacgcaagctggtaccagcagaaaccgggtcaggccccagttctggtgatttacggcaaaaacaaccgtccgtctgggatcccggaccgtttctccggcagctcttccggtaacacggcgagcctcaccatcactggcgctcaagcagaagacgaggccgactattactgtaactctcgggaaagcccaccaaccggcctggttgtcttcggtggcggtaccaagctgaccgtccta

SEQ ID NO: 420 - DNA, 2022 bp, synthetic construct
  misc_feature 1..2022: note = source = /note="Description of Artificial Sequence: Syntheticpolynucleotide"
  source 1..2022: mol_type = other DNA
gaggtgcaattgttggagtctgggggaggcttggtacagcctggggggtccctgagactctcctgtgcagcctccggattcacctttagcagttatgccatgagctgggtccgccaggctccagggaaggggctggagtgggtctcagctattagtggtagtggtggtagcacatactacgcagactccgtgaagggccggttcaccatctccagagacaattccaagaacacgctgtatctgcagatgaacagcctgagagccgaggacacggccgtatattactgtgcgcgtggtgactaccgttaccgttacttcgactactggggccaaggaaccctggtcaccgtctcgagtgctagcaccaagggcccctccgtgtttcctctggccccttccagcaagtccacctctggcggaactgccgctctgggctgcctggtggaagattacttccccgagcccgtgaccgtgtcctggaattctggcgctctgacctccggcgtgcacacctttccagctgtgctgcagtcctccggcctgtactccctgtcctccgtcgtgacagtgccctccagctctctgggcacccagacctacatctgcaacgtgaaccacaagccctccaacaccaaggtggacgagaaggtggaacccaagtcctgcgacggtggcggaggttccggaggcggaggatcccaggctgtcgtgacccaggaaccctccctgacagtgtctcctggcggcaccgtgaccctgacctgtggatcttctaccggcgctgtgaccacctccaactacgccaattgggtgcaggaaaagcccggccaggccttcagaggactgatcggcggcaccaacaagagagcccctggcacccctgccagattctccggttctctgctgggcggcaaggctgccctgactctgtctggtgctcagcctgaggacgaggccgagtactactgcgccctgtggtactccaacctgtgggtgttcggcggaggcaccaagctgaccgtgctgtccagcgcttccaccaagggacccagtgtgttccccctggcccccagctccaagtctacatccggtggcacagctgccctgggatgtctcgtgaaggactactttcctgagcctgtgacagtgtcttggaacagcggagccctgaccagcggagtgcacacattccctgcagtgctgcagagcagcggcctgtatagcctgagcagcgtcgtgaccgtgccttcctctagcctgggaacacagacatatatctgtaatgtgaatcataagcccagtaataccaaagtggataagaaagtggaacctaagagctgcgataagacccacacctgtcccccctgccctgctcctgaagctgctggtggccctagcgtgttcctgttccccccaaagcccaaggacaccctgatgatctcccggacccccgaagtgacctgcgtggtggtggatgtgtcccacgaggaccctgaagtgaagttcaattggtacgtggacggcgtggaagtgcacaacgccaagaccaagcctagagaggaacagtacaactccacctaccgggtggtgtccgtgctgacagtgctgcaccaggactggctgaacggcaaagagtacaagtgcaaggtgtccaacaaggccctgggcgctcccatcgaaaagaccatctccaaggccaagggccagccccgggaaccccaggtgtacaccctgcccccatgccgggatgagctgaccaagaaccaggtcagcctgtggtgcctggtcaaaggcttctatcccagcgacatcgccgtggagtgggagagcaatgggcagccggagaacaactacaagaccacgcctcccgtgctggactccgacggctccttcttcctctacagcaagctcaccgtggacaagagcaggtggcagcaggggaacgtcttctcatgctccgtgatgcatgaggctctgcacaaccactacacgcagaagagcctctccctgtctccgggtaaa

SEQ ID NO: 421 - DNA, 1347 bp, synthetic construct
  misc_feature 1..1347: note = source = /note="Description of Artificial Sequence: Syntheticpolynucleotide"
  source 1..1347: mol_type = other DNA
gaggtgcaattgttggagtctgggggaggcttggtacagcctggggggtccctgagactctcctgtgcagcctccggattcacctttagcagttatgccatgagctgggtccgccaggctccagggaaggggctggagtgggtctcagctattagtggtagtggtggtagcacatactacgcagactccgtgaagggccggttcaccatctccagagacaattccaagaacacgctgtatctgcagatgaacagcctgagagccgaggacacggccgtatattactgtgcgcgtggtgactaccgttaccgttacttcgactactggggccaaggaaccctggtcaccgtctcgagtgctagcaccaagggcccctccgtgttccccctggcccccagcagcaagagcaccagcggcggcacagccgctctgggctgcctggtcgaggactacttccccgagcccgtgaccgtgtcctggaacagcggagccctgacctccggcgtgcacaccttccccgccgtgctgcagagttctggcctgtatagcctgagcagcgtggtcaccgtgccttctagcagcctgggcacccagacctacatctgcaacgtgaaccacaagcccagcaacaccaaggtggacgagaaggtggagcccaagagctgcgacaaaactcacacatgcccaccgtgcccagcacctgaagctgcagggggaccgtcagtcttcctcttccccccaaaacccaaggacaccctcatgatctcccggacccctgaggtcacatgcgtggtggtggacgtgagccacgaagaccctgaggtcaagttcaactggtacgtggacggcgtggaggtgcataatgccaagacaaagccgcgggaggagcagtacaacagcacgtaccgtgtggtcagcgtcctcaccgtcctgcaccaggactggctgaatggcaaggagtacaagtgcaaggtctccaacaaagccctcggcgcccccatcgagaaaaccatctccaaagccaaagggcagccccgagaaccacaggtgtgcaccctgcccccatcccgggatgagctgaccaagaaccaggtcagcctctcgtgcgcagtcaaaggcttctatcccagcgacatcgccgtggagtgggagagcaatgggcagccggagaacaactacaagaccacgcctcccgtgctggactccgacggctccttcttcctcgtgagcaagctcaccgtggacaagagcaggtggcagcaggggaacgtcttctcatgctccgtgatgcatgaggctctgcacaaccactacacgcagaagagcctctccctgtctccgggtaaa

SEQ ID NO: 422 - DNA, 645 bp, synthetic construct
  misc_feature 1..645: note = source = /note="Description of Artificial Sequence: Syntheticpolynucleotide"
  source 1..645: mol_type = other DNA
tcttctgaactgactcaagatccagctgttagcgtggctctgggtcagactgtacgtatcacctgccaaggcgattctctgcgctcctactacgcaagctggtaccagcagaaaccgggtcaggccccagttctggtgatttacggcaaaaacaaccgtccgtctgggatcccggaccgtttctccggcagctcttccggtaacacggcgagcctcaccatcactggcgctcaagcagaagacgaggccgactattactgtaactctcgggaaagcccaccaaccggcctggttgtcttcggtggcggtaccaagctgaccgtcctaggtcaacccaaggctgcccccagcgtgaccctgttcccccccagcagcaagaaactgcaggccaacaaggccaccctggtctgcctgatcagcgacttctacccaggcgccgtgaccgtggcctggaaggccgacagcagccccgtgaaggccggcgtggagaccaccacccccagcaagcagagcaacaacaagtacgccgccagcagctacctgagcctgacccccgagcagtggaagagccacaggtcctacagctgccaggtgacccacgagggcagcaccgtggagaaaaccgtggcccccaccgagtgcagc

SEQ ID NO: 423 - DNA, 354 bp, synthetic construct
  misc_feature 1..354: note = source = /note="Description of Artificial Sequence: Syntheticpolynucleotide"
  source 1..354: mol_type = other DNA
caggtgcaattggttcaatctggtgctgaagtaaaaaaaccgggcgcttccgttaaagtgagctgcaaagcatccggatacaccttcacttcctattacatgcactgggttcgtcaagccccgggccagggtctggaatggatgggcatcattaacccaagcggtggctctacctcctacgcgcagaaattccagggtcgcgtcacgatgacccgtgacactagcacctctaccgtttatatggagctgtccagcctgcgttctgaagatactgcagtgtactactgtgcacgcggtgactggtcttactacatggactattggggtcaaggcaccctcgtaacggtttcttct

SEQ ID NO: 424 - DNA, 333 bp, synthetic construct
  misc_feature 1..333: note = source = /note="Description of Artificial Sequence: Syntheticpolynucleotide"
  source 1..333: mol_type = other DNA
gatattgttatgactcaatctccactgtctctgccggtgactccaggcgaaccggcgagcatttcttgccgttccagccagtctctgctgcactccaacggctacaactatctcgattggtacctgcaaaaaccgggtcagagccctcagctgctgatctacctgggctctaaccgcgcttccggtgtaccggaccgtttcagcggctctggatccggcaccgatttcacgttgaaaatcagccgtgttgaagcagaagacgtgggcgtttattactgtatgcaggcacggcagaccccaacttttggtcaaggcaccaaggtcgaaattaaa

SEQ ID NO: 425 - DNA, 2019 bp, synthetic construct
  misc_feature 1..2019: note = source = /note="Description of Artificial Sequence: Syntheticpolynucleotide"
  source 1..2019: mol_type = other DNA
caggtgcaattggttcaatctggtgctgaagtaaaaaaaccgggcgcttccgttaaagtgagctgcaaagcatccggatacaccttcacttcctattacatgcactgggttcgtcaagccccgggccagggtctggaatggatgggcatcattaacccaagcggtggctctacctcctacgcgcagaaattccagggtcgcgtcacgatgacccgtgacactagcacctctaccgtttatatggagctgtccagcctgcgttctgaagatactgcagtgtactactgtgcacgcggtgactggtcttactacatggactattggggtcaaggcaccctcgtaacggtttcttctgctagcaccaagggcccctccgtgtttcctctggccccttccagcaagtccacctctggcggaactgccgctctgggctgcctggtggaagattacttccccgagcccgtgaccgtgtcctggaattctggcgctctgacctccggcgtgcacacctttccagctgtgctgcagtcctccggcctgtactccctgtcctccgtcgtgacagtgccctccagctctctgggcacccagacctacatctgcaacgtgaaccacaagccctccaacaccaaggtggacgagaaggtggaacccaagtcctgcgacggtggcggaggttccggaggcggaggatcccaggctgtcgtgacccaggaaccctccctgacagtgtctcctggcggcaccgtgaccctgacctgtggatcttctaccggcgctgtgaccacctccaactacgccaattgggtgcaggaaaagcccggccaggccttcagaggactgatcggcggcaccaacaagagagcccctggcacccctgccagattctccggttctctgctgggcggcaaggctgccctgactctgtctggtgctcagcctgaggacgaggccgagtactactgcgccctgtggtactccaacctgtgggtgttcggcggaggcaccaagctgaccgtgctgtccagcgcttccaccaagggacccagtgtgttccccctggcccccagctccaagtctacatccggtggcacagctgccctgggatgtctcgtgaaggactactttcctgagcctgtgacagtgtcttggaacagcggagccctgaccagcggagtgcacacattccctgcagtgctgcagagcagcggcctgtatagcctgagcagcgtcgtgaccgtgccttcctctagcctgggaacacagacatatatctgtaatgtgaatcataagcccagtaataccaaagtggataagaaagtggaacctaagagctgcgataagacccacacctgtcccccctgccctgctcctgaagctgctggtggccctagcgtgttcctgttccccccaaagcccaaggacaccctgatgatctcccggacccccgaagtgacctgcgtggtggtggatgtgtcccacgaggaccctgaagtgaagttcaattggtacgtggacggcgtggaagtgcacaacgccaagaccaagcctagagaggaacagtacaactccacctaccgggtggtgtccgtgctgacagtgctgcaccaggactggctgaacggcaaagagtacaagtgcaaggtgtccaacaaggccctgggcgctcccatcgaaaagaccatctccaaggccaagggccagccccgggaaccccaggtgtacaccctgcccccatgccgggatgagctgaccaagaaccaggtcagcctgtggtgcctggtcaaaggcttctatcccagcgacatcgccgtggagtgggagagcaatgggcagccggagaacaactacaagaccacgcctcccgtgctggactccgacggctccttcttcctctacagcaagctcaccgtggacaagagcaggtggcagcaggggaacgtcttctcatgctccgtgatgcatgaggctctgcacaaccactacacgcagaagagcctctccctgtctccgggtaaa

SEQ ID NO: 426 - DNA, 1344 bp, synthetic construct
  misc_feature 1..1344: note = source = /note="Description of Artificial Sequence: Syntheticpolynucleotide"
  source 1..1344: mol_type = other DNA
caggtgcaattggttcaatctggtgctgaagtaaaaaaaccgggcgcttccgttaaagtgagctgcaaagcatccggatacaccttcacttcctattacatgcactgggttcgtcaagccccgggccagggtctggaatggatgggcatcattaacccaagcggtggctctacctcctacgcgcagaaattccagggtcgcgtcacgatgacccgtgacactagcacctctaccgtttatatggagctgtccagcctgcgttctgaagatactgcagtgtactactgtgcacgcggtgactggtcttactacatggactattggggtcaaggcaccctcgtaacggtttcttctgctagcaccaagggcccctccgtgttccccctggcccccagcagcaagagcaccagcggcggcacagccgctctgggctgcctggtcgaggactacttccccgagcccgtgaccgtgtcctggaacagcggagccctgacctccggcgtgcacaccttccccgccgtgctgcagagttctggcctgtatagcctgagcagcgtggtcaccgtgccttctagcagcctgggcacccagacctacatctgcaacgtgaaccacaagcccagcaacaccaaggtggacgagaaggtggagcccaagagctgcgacaaaactcacacatgcccaccgtgcccagcacctgaagctgcagggggaccgtcagtcttcctcttccccccaaaacccaaggacaccctcatgatctcccggacccctgaggtcacatgcgtggtggtggacgtgagccacgaagaccctgaggtcaagttcaactggtacgtggacggcgtggaggtgcataatgccaagacaaagccgcgggaggagcagtacaacagcacgtaccgtgtggtcagcgtcctcaccgtcctgcaccaggactggctgaatggcaaggagtacaagtgcaaggtctccaacaaagccctcggcgcccccatcgagaaaaccatctccaaagccaaagggcagccccgagaaccacaggtgtgcaccctgcccccatcccgggatgagctgaccaagaaccaggtcagcctctcgtgcgcagtcaaaggcttctatcccagcgacatcgccgtggagtgggagagcaatgggcagccggagaacaactacaagaccacgcctcccgtgctggactccgacggctccttcttcctcgtgagcaagctcaccgtggacaagagcaggtggcagcaggggaacgtcttctcatgctccgtgatgcatgaggctctgcacaaccactacacgcagaagagcctctccctgtctccgggtaaa

SEQ ID NO: 427 - DNA, 654 bp, synthetic construct
  misc_feature 1..654: note = source = /note="Description of Artificial Sequence: Syntheticpolynucleotide"
  source 1..654: mol_type = other DNA
gatattgttatgactcaatctccactgtctctgccggtgactccaggcgaaccggcgagcatttcttgccgttccagccagtctctgctgcactccaacggctacaactatctcgattggtacctgcaaaaaccgggtcagagccctcagctgctgatctacctgggctctaaccgcgcttccggtgtaccggaccgtttcagcggctctggatccggcaccgatttcacgttgaaaatcagccgtgttgaagcagaagacgtgggcgtttattactgtatgcaggcacggcagaccccaacttttggtcaaggcaccaaggtcgaaattaaacgtacggtggctgcaccatctgtcttcatcttcccgccatctgatcggaagttgaaatctggaactgcctctgttgtgtgcctgctgaataacttctatcccagagaggccaaagtacagtggaaggtggataacgccctccaatcgggtaactcccaggagagtgtcacagagcaggacagcaaggacagcacctacagcctcagcagcaccctgacgctgagcaaagcagactacgagaaacacaaagtctacgcctgcgaagtcacccatcagggcctgagctcgcccgtcacaaagagcttcaacaggggagagtgt

SEQ ID NO: 428 - protein, 104 aa, synthetic construct
  REGION 1..104: note = source = /note="Description of Artificial Sequence: Syntheticpolypeptide"
ASTKGPSVFPLAPSSKSTSGGTAALGCLVKDYFPEPVTVSWNSGALTSGVHTFPAVLQSSGLYSLSSVVTVPSSSLGTQTYICNVNHKPSNTKVDKKVEPKSCD

SEQ ID NO: 429 - protein, 27 aa, synthetic construct
  VARIANT 13..24: note = /replace=" "
  REGION 1..24: note = MISC_FEATURE - /note="This region may encompass 3-6 "Gly Gly Gly Ser"repeating units"
  VARIANT 25..27: note = /replace=" "
  REGION 1..27: note = MISC_FEATURE - /note="Variant residues given in the sequence have nopreference with respect to those in the annotationsfor variant positions"
  REGION 1..27: note = source = /note="Description of Artificial Sequence: Syntheticpeptide"
GGGSGGGSGGGSGGGSGGGSGGGSGGG

SEQ ID NO: 430 - protein, 28 aa, synthetic construct
  VARIANT 11..25: note = /replace=" "
  REGION 1..25: note = MISC_FEATURE - /note="This region may encompass 2-5 "Gly Gly Gly Gly Ser"repeating units"
  VARIANT 26..28: note = /replace=" "
  REGION 1..28: note = MISC_FEATURE - /note="Variant residues given in the sequence have nopreference with respect to those in the annotationsfor variant positions"
  REGION 1..28: note = source = /note="Description of Artificial Sequence: Syntheticpeptide"
GGGGSGGGGSGGGGSGGGGSGGGGSGGG